European Patent Application EP 4 549 452 A1, published May 7, 2025. Title: PHARMACEUTICAL COMPOSITION FOR RESISTING INFECTION WITH SARS-COV-2 OR MUTANT THEREOF AND COMBINED DRUG THEREOF. Applicant: WestVac Biopharma Co., Ltd. Application CN. The sequence listing filed with the application follows.

SEQUENCE LISTING (79 sequences)

SEQ ID NO: 1 - protein, 226 aa, synthetic construct
VQPTESIVRFPNITNLCPFGEVFNATRFASVYAWNRKRISNCVADYSVLYNSASFSTFKCYGVSPTKLNDLCFTNVYADSFVIRGDEVRQIAPGQTGKIADYNYKLPDDFTGCVIAWNSNNLDSKVGGNYNYLYRLFRKSNLKPFERDISTEIYQAGSTPCNGVEGFNCYFPLQSYGFQPTNGVGYQPYRVVVLSFELLHAPATVCGPKKSTNLVKNKCVNFNFNG

SEQ ID NO: 2 - protein, 492 aa, synthetic construct
MLLVNQSHQGFNKEHTSKMVSAIVLYVLLAAAAHSAFAADSIHIKDSDDLKNRLAEAGDKLVVIDFMATWCGPCKMIGPKLDEMANEMSDSIVVLKVDVDECEDIATEYNINSMPTFVFVKNSKKIEEFSGANVDKLRNTIIKLKLAGSGSGHMHHHHHHSSGDDDDKVQPTESIVRFPNITNLCPFGEVFNATRFASVYAWNRKRISNCVADYSVLYNSASFSTFKCYGVSPTKLNDLCFTNVYADSFVIRGDEVRQIAPGQTGNIADYNYKLPDDFTGCVIAWNSNNLDSKVGGNYNYRYRLFRKSNLKPFERDISTEIYQAGSTPCNGVKGFNCYFPLQSYGFQPTYGVGYQPYRVVVLSFELLHAPATVCGPKKSTNLVKNKSVNFNFNGLYENQKLIANQFNSAIGKIQDSLSSTASALGKLQDVVNQNAQALNTLVKQLKNHTSPDVDLGDISGINASVVNIQKEIDRLNEVAKNLNESLIDLQEL

SEQ ID NO: 3 - protein, 492 aa, synthetic construct
MLLVNQSHQGFNKEHTSKMVSAIVLYVLLAAAAHSAFAADSIHIKDSDDLKNRLAEAGDKLVVIDFMATWCGPCKMIGPKLDEMANEMSDSIVVLKVDVDECEDIATEYNINSMPTFVFVKNSKKIEEFSGANVDKLRNTIIKLKLAGSGSGHMHHHHHHSSGDDDDKVQPTESIVRFPNITNLCPFGEVFNATRFASVYAWNRKRISNCVADYSVLYNSASFSTFKCYGVSPTKLNDLCFTNVYADSFVIRGDEVRQIAPGQTGKIADYNYKLPDDFTGCVIAWNSNNLDSKVGGNYNYRYRLFRKSNLKPFERDISTEIYQAGSKPCNGVEGFNCYFPLQSYGFQPTNGVGYQPYRVVVLSFELLHAPATVCGPKKSTNLVKNKSVNFNFNGLYENQKLIANQFNSAIGKIQDSLSSTASALGKLQDVVNQNAQALNTLVKQLKNHTSPDVDLGDISGINASVVNIQKEIDRLNEVAKNLNESLIDLQEL

SEQ ID NO: 4 - protein, 492 aa, synthetic construct
MLLVNQSHQGFNKEHTSKMVSAIVLYVLLAAAAHSAFAADSIHIKDSDDLKNRLAEAGDKLVVIDFMATWCGPCKMIGPKLDEMANEMSDSIVVLKVDVDECEDIATEYNINSMPTFVFVKNSKKIEEFSGANVDKLRNTIIKLKLAGSGSGHMHHHHHHSSGDDDDKVQPTESIVRFPNITNLCPFDEVFNATRFASVYAWNRKRISNCVADYSVLYNLAPFFTFKCYGVSPTKLNDLCFTNVYADSFVIRGDEVRQIAPGQTGNIADYNYKLPDDFTGCVIAWNSNKLDSKVSGNYNYLYRLFRKSNLKPFERDISTEIYQAGNKPCNGVAGFNCYFPLRSYSFRPTYGVGHQPYRVVVLSFELLHAPATVCGPKKSTNLVKNKSVNFNFNGLYENQKLIANQFNSAIGKIQDSLSSTASALGKLQDVVNQNAQALNTLVKQLKNHTSPDVDLGDISGINASVVNIQKEIDRLNEVAKNLNESLIDLQEL

SEQ ID NO: 5 - protein, 492 aa, synthetic construct
MLLVNQSHQGFNKEHTSKMVSAIVLYVLLAAAAHSAFAADSIHIKDSDDLKNRLAEAGDKLVVIDFMATWCGPCKMIGPKLDEMANEMSDSIVVLKVDVDECEDIATEYNINSMPTFVFVKNSKKIEEFSGANVDKLRNTIIKLKLAGSGSGHMHHHHHHSSGDDDDKVQPTESIVRFPNITNLCPFDEVFNATRFASVYAWNRKRISNCVADYSVLYNFAPFFAFKCYGVSPTKLNDLCFTNVYADSFVIRGNEVSQIAPGQTGNIADYNYKLPDDFTGCVIAWNSNKLDSKVGGNYNYLYRLFRKSNLKPFERDISTEIYQAGNKPCNGVAGFNCYFPLRSYGFRPTYGVGHQPYRVVVLSFELLHAPATVCGPKKSTNLVKNKSVNFNFNGLYENQKLIANQFNSAIGKIQDSLSSTASALGKLQDVVNQNAQALNTLVKQLKNHTSPDVDLGDISGINASVVNIQKEIDRLNEVAKNLNESLIDLQEL

SEQ ID NO: 6 - protein, 492 aa, synthetic construct
MLLVNQSHQGFNKEHTSKMVSAIVLYVLLAAAAHSAFAADSIHIKDSDDLKNRLAEAGDKLVVIDFMATWCGPCKMIGPKLDEMANEMSDSIVVLKVDVDECEDIATEYNINSMPTFVFVKNSKKIEEFSGANVDKLRNTIIKLKLAGSGSGHMHHHHHHSSGDDDDKVQPTESIVRFPNITNLCPFDEVFNATRFASVYAWNRKRISNCVADYSVLYNFAPFFAFKCYGVSPTKLNDLCFTNVYADSFVIRGNEVSQIAPGQTGNIADYNYKLPDDFTGCVIAWNSNKLDSKVGGNYNYRYRLFRKSNLKPFERDISTEIYQAGNKPCNGVAGVNCYFPLQSYGFRPTYGVGHQPYRVVVLSFELLHAPATVCGPKKSTNLVKNKSVNFNFNGLYENQKLIANQFNSAIGKIQDSLSSTASALGKLQDVVNQNAQALNTLVKQLKNHTSPDVDLGDISGINASVVNIQKEIDRLNEVAKNLNESLIDLQEL

SEQ ID NO: 7 - protein, 492 aa, synthetic construct
MLLVNQSHQGFNKEHTSKMVSAIVLYVLLAAAAHSAFAADSIHIKDSDDLKNRLAEAGDKLVVIDFMATWCGPCKMIGPKLDEMANEMSDSIVVLKVDVDECEDIATEYNINSMPTFVFVKNSKKIEEFSGANVDKLRNTIIKLKLAGSGSGHMHHHHHHSSGDDDDKVQPTESIVRFPNITNLCPFDEVFNATRFASVYAWNRKRISNCVADYSVLYNFAPFFAFKCYGVSPTKLNDLCFTNVYADSFVIRGNEVSQIAPGQTGNIADYNYKLPDDFTGCVIAWNSNKLDSKVGGNYNYQYRLFRKSNLKPFERDISTEIYQAGNKPCNGVAGFNCYFPLRSYGFRPTYGVGHQPYRVVVLSFELLHAPATVCGPKKSTNLVKNKSVNFNFNGLYENQKLIANQFNSAIGKIQDSLSSTASALGKLQDVVNQNAQALNTLVKQLKNHTSPDVDLGDISGINASVVNIQKEIDRLNEVAKNLNESLIDLQEL

SEQ ID NO: 8 - protein, 492 aa, synthetic construct
MLLVNQSHQGFNKEHTSKMVSAIVLYVLLAAAAHSAFAADSIHIKDSDDLKNRLAEAGDKLVVIDFMATWCGPCKMIGPKLDEMANEMSDSIVVLKVDVDECEDIATEYNINSMPTFVFVKNSKKIEEFSGANVDKLRNTIIKLKLAGSGSGHMHHHHHHSSGDDDDKVQPTESIVRFPNITNLCPFDEVFNATTFASVYAWNRKRISNCVADYSVLYNFAPFFAFKCYGVSPTKLNDLCFTNVYADSFVIRGNEVSQIAPGQTGNIADYNYKLPDDFTGCVIAWNSNKLDSKVGGNYNYRYRLFRKSNLKPFERDISTEIYQAGNKPCNGVAGVNCYFPLQSYGFRPTYGVGHQPYRVVVLSFELLHAPATVCGPKKSTNLVKNKSVNFNFNGLYENQKLIANQFNSAIGKIQDSLSSTASALGKLQDVVNQNAQALNTLVKQLKNHTSPDVDLGDISGINASVVNIQKEIDRLNEVAKNLNESLIDLQEL

SEQ ID NO: 9 - protein, 492 aa, synthetic construct
MLLVNQSHQGFNKEHTSKMVSAIVLYVLLAAAAHSAFAADSIHIKDSDDLKNRLAEAGDKLVVIDFMATWCGPCKMIGPKLDEMANEMSDSIVVLKVDVDECEDIATEYNINSMPTFVFVKNSKKIEEFSGANVDKLRNTIIKLKLAGSGSGHMHHHHHHSSGDDDDKVQPTESIVRFPNITNLCPFDEVFNATRFASVYAWNRKRISNCVADYSVLYNFAPFFAFKCYGVSPTKLNDLCFTNVYADSFVIRGNEVSQIAPGQTGNIADYNYKLPDDFTGCVIAWNSNKLDSTVGGNYNYRYRLFRKSKLKPFERDISTEIYQAGNKPCNGVAGVNCYFPLQSYGFRPTYGVGHQPYRVVVLSFELLHAPATVCGPKKSTNLVKNKSVNFNFNGLYENQKLIANQFNSAIGKIQDSLSSTASALGKLQDVVNQNAQALNTLVKQLKNHTSPDVDLGDISGINASVVNIQKEIDRLNEVAKNLNESLIDLQEL

SEQ ID NO: 10 - DNA, 1479 bp, synthetic construct
  source 1..1479: mol_type = other DNA
atgctactagtaaatcagtcacaccaaggcttcaataaggaacacacaagcaagatggtgagcgctatcgtgctgtacgtcctgctggccgctgctgctcacagcgctttcgctgctgactccatccacatcaaggacagcgacgacctgaagaaccgtctggccgaggccggtgacaagctggtcgtcatcgacttcatggccacttggtgcggtccttgcaagatgatcggccctaagctggacgagatggctaacgagatgtccgacagcatcgtggtcctgaaggtggacgtcgacgagtgcgaggacatcgccaccgaatacaacatcaacagcatgcccaccttcgtgttcgtgaagaacagcaagaagatcgaggaattttccggcgctaacgtcgacaagctgcgtaacaccatcatcaagctgaagctggccggctccggctccggccacatgcatcaccaccaccaccattcctccggtgacgacgacgacaaggtgcagccaaccgaatctatcgtcagattcccaaacatcactaacctgtgccctttcggagaggtgttcaacgctaccaggttcgccagcgtctacgcttggaaccgcaagcgtatcagcaactgcgtcgccgactactctgtgctgtacaactccgctagcttctctactttcaagtgctacggcgtgtcacctaccaagctgaacgacctgtgcttcactaacgtctacgccgactccttcgtgatccgcggagacgaagtccgtcagatcgctcctggacagaccggaaatatcgctgactacaactacaagctgccagacgacttcactggctgcgtgatcgcttggaactcaaacaacctggactccaaggtcggtggcaactacaactaccggtacaggctgttcagaaagtcaaacctgaagcctttcgagcgcgacatctcaaccgaaatctaccaggctggttccactccctgcaacggtgtgaagggcttcaactgctacttccccctgcagtcctacggtttccagccaacctatggagtcggttaccagccttaccgtgtggtcgtgctgagcttcgaactgctccacgctcctgctactgtgtgcggtcccaagaagtctactaacctggtcaaaaacaaaagcgtcaacttcaacttcaacggtctgtacgagaaccagaagctgatcgctaaccagttcaacagcgccatcggcaagatccaggactcactgtcatccactgcctccgctctgggaaagctgcaggacgtcgtgaaccagaacgcccaggctctgaacaccctggtcaagcagctgaagaaccacacctctcctgacgtcgacctgggcgacatcagcggaatcaacgcttctgtcgtgaacatccagaaggagatcgaccgcctgaacgaagtggccaagaacctgaacgaatccctgattgacctccaagaactctaa

SEQ ID NO: 11 - DNA, 1479 bp, synthetic construct
  source 1..1479: mol_type = other DNA
atgctactagtaaatcagtcacaccaaggcttcaataaggaacacacaagcaagatggtgagcgctatcgtgctgtacgtcctgctggccgctgctgctcacagcgctttcgctgctgactccatccacatcaaggacagcgacgacctgaagaaccgtctggccgaggccggtgacaagctggtcgtcatcgacttcatggccacttggtgcggtccttgcaagatgatcggccctaagctggacgagatggctaacgagatgtccgacagcatcgtggtcctgaaggtggacgtcgacgagtgcgaggacatcgccaccgaatacaacatcaacagcatgcccaccttcgtgttcgtgaagaacagcaagaagatcgaggaattttccggcgctaacgtcgacaagctgcgtaacaccatcatcaagctgaagctggccggctccggctccggccacatgcatcaccaccaccaccattcctccggtgacgacgacgacaaggtgcagccaaccgaatctatcgtcagattcccaaacatcactaacctgtgccctttcggagaggtgttcaacgctaccaggttcgccagcgtctacgcttggaaccgcaagcgtatcagcaactgcgtcgccgactactctgtgctgtacaactccgctagcttctctactttcaagtgctacggcgtgtcacctaccaagctgaacgacctgtgcttcactaacgtctacgccgactccttcgtgatccgcggagacgaagtccgtcagatcgctcctggacagaccggaaagatcgctgactacaactacaagctgccagacgacttcactggctgcgtgatcgcttggaactcaaacaacctggactccaaggtcggtggcaactacaactaccggtacaggctgttcagaaagtcaaacctgaagcctttcgagcgcgacatctcaaccgaaatctaccaggctggttccaagccctgcaacggtgtggagggcttcaactgctacttccccctgcagtcctacggtttccagccaaccaacggagtcggttaccagccttaccgtgtggtcgtgctgagcttcgaactgctccacgctcctgctactgtgtgcggtcccaagaagtctactaacctggtcaaaaacaaaagcgtcaacttcaacttcaacggtctgtacgagaaccagaagctgatcgctaaccagttcaacagcgccatcggcaagatccaggactcactgtcatccactgcctccgctctgggaaagctgcaggacgtcgtgaaccagaacgcccaggctctgaacaccctggtcaagcagctgaagaaccacacctctcctgacgtcgacctgggcgacatcagcggaatcaacgcttctgtcgtgaacatccagaaggagatcgaccgcctgaacgaagtggccaagaacctgaacgaatccctgattgacctccaagaactctaa

SEQ ID NO: 12 - DNA, 1479 bp, synthetic construct
  source 1..1479: mol_type = other DNA
atgctactagtaaatcagtcacaccaaggcttcaataaggaacacacaagcaagatggtgagcgctatcgtgctgtacgtcctgctggccgctgctgctcacagcgctttcgctgctgactccatccacatcaaggacagcgacgacctgaagaaccgtctggccgaggccggtgacaagctggtcgtcatcgacttcatggccacttggtgcggtccttgcaagatgatcggccctaagctggacgagatggctaacgagatgtccgacagcatcgtggtcctgaaggtggacgtcgacgagtgcgaggacatcgccaccgaatacaacatcaacagcatgcccaccttcgtgttcgtgaagaacagcaagaagatcgaggaattttccggcgctaacgtcgacaagctgcgtaacaccatcatcaagctgaagctggccggctccggctccggccacatgcatcaccaccaccaccattcctccggtgacgacgacgacaaggtgcagccaaccgaatctatcgtcagattcccaaacatcactaacctgtgccctttcgatgaggtgttcaacgctaccaggttcgccagcgtctacgcttggaaccgcaagcgtatcagcaactgcgtcgccgactactctgtgctgtacaacctcgctcctttcttcactttcaagtgctacggcgtgtcacctaccaagctgaacgacctgtgcttcactaacgtctacgccgactccttcgtgatccgcggagacgaagtccgtcagatcgctcctggacagaccggaaatatcgctgactacaactacaagctgccagacgacttcactggctgcgtgatcgcttggaactcaaacaagctggactccaaggtcagtggcaactacaactacctgtacaggctgttcagaaagtcaaacctgaagcctttcgagcgcgacatctcaaccgaaatctaccaggctggtaataagccctgcaacggtgtggctggcttcaactgctacttccccctgagatcctactctttccgaccaacctacggagtcggtcatcagccttaccgtgtggtcgtgctgagcttcgaactgctccacgctcctgctactgtgtgcggtcccaagaagtctactaacctggtcaaaaacaaaagcgtcaacttcaacttcaacggtctgtacgagaaccagaagctgatcgctaaccagttcaacagcgccatcggcaagatccaggactcactgtcatccactgcctccgctctgggaaagctgcaggacgtcgtgaaccagaacgcccaggctctgaacaccctggtcaagcagctgaagaaccacacctctcctgacgtcgacctgggcgacatcagcggaatcaacgcttctgtcgtgaacatccagaaggagatcgaccgcctgaacgaagtggccaagaacctgaacgaatccctgattgacctccaagaactctaa

SEQ ID NO: 13 - DNA, 1479 bp, synthetic construct
  source 1..1479: mol_type = other DNA
atgctgctggtgaaccagagccaccagggtttcaacaaggaacacactagcaagatggtgtctgctatcgtcctctacgtgctgctcgccgccgctgctcactcagctttcgccgctgactctatccacatcaaggactccgacgacctcaagaaccgtttggccgaagccggcgacaagctggtcgttatcgacttcatggctacctggtgtggcccttgcaagatgatcggacctaagctggacgaaatggctaacgagatgagcgacagcatcgtcgttctgaaggtggacgtcgacgaatgtgaggacatcgccactgagtacaacatcaacagcatgcctaccttcgttttcgtgaagaactctaagaagatcgaggagttctctggtgccaacgtggacaagctccgtaacaccatcatcaagctcaagctggccggcagcggtagcggtcacatgcaccaccaccaccaccattcaagcggcgacgacgacgacaaggtgcagccaaccgaatcaatcgtccgcttcccaaacatcactaacctgtgcccattcgacgaggtgttcaacgccacccgtttcgcctctgtctacgcttggaaccgcaagcgcatctccaactgtgtcgccgactacagcgtgctgtacaacttcgctcctttcttcgcattcaagtgttacggagtgtcccctaccaagctcaacgatttgtgcttcacaaacgtgtacgctgacagcttcgtgatccgtggtaacgaggtttctcaaatcgcccctggtcagacaggtaacatcgctgactacaactacaagctcccagacgacttcactggctgtgttatcgcttggaactcaaacaagctggactctaaggtgggtggtaactacaactacctctaccgtctgttccgcaagagcaacctcaagccattcgaacgtgacatcagcacagagatctaccaagccggtaacaagccctgcaacggcgttgccggattcaactgctacttccccctccgttcctacggattccgcccaacctacggcgtgggtcaccagccataccgcgtggttgtgctgagcttcgaactgctgcacgcccccgctaccgtgtgtggccctaagaagagcactaacctcgttaagaacaagtccgtgaacttcaacttcaacggtctctacgaaaaccagaagctgatcgctaaccagttcaactccgccatcggcaagatccaggactccctgtcctccacagcttccgctctgggcaagctgcaggacgttgtgaaccaaaacgctcaggccctgaacacactggtgaagcaactgaagaaccacaccagccccgacgttgacctgggtgacatcagcggtatcaacgctagcgtggtgaacatccagaaggagatcgacaggctgaacgaagtggctaagaacttgaacgagagcctcatcgacctgcaggaactgtaa

SEQ ID NO: 14 - DNA, 1479 bp, synthetic construct
  source 1..1479: mol_type = other DNA
atgctgctggtgaaccagagccaccagggtttcaacaaggaacacactagcaagatggtgtctgctatcgtcctctacgtgctgctcgccgccgctgctcactcagctttcgccgctgactctatccacatcaaggactccgacgacctcaagaaccgtttggccgaagccggcgacaagctggtcgttatcgacttcatggctacctggtgtggcccttgcaagatgatcggacctaagctggacgaaatggctaacgagatgagcgacagcatcgtcgttctgaaggtggacgtcgacgaatgtgaggacatcgccactgagtacaacatcaacagcatgcctaccttcgttttcgtgaagaactctaagaagatcgaggagttctctggtgccaacgtggacaagctccgtaacaccatcatcaagctcaagctggccggcagcggtagcggtcacatgcaccaccaccaccaccattcaagcggcgacgacgacgacaaggtgcagccaaccgaatcaatcgtccgcttcccaaacatcactaacctgtgcccattcgacgaggtgttcaacgccacccgtttcgcctctgtctacgcttggaaccgcaagcgcatctccaactgtgtcgccgactacagcgtgctgtacaacttcgctcctttcttcgcattcaagtgttacggagtgtcccctaccaagctcaacgatttgtgcttcacaaacgtgtacgctgacagcttcgtgatccgtggtaacgaggtttctcaaatcgcccctggtcagacaggtaacatcgctgactacaactacaagctcccagacgacttcactggctgtgttatcgcttggaactcaaacaagctggactctaaggtgggtggtaactacaactaccggtaccgtctgttccgcaagagcaacctcaagccattcgaacgtgacatcagcacagagatctaccaagccggtaacaagccctgcaacggcgttgccggagtcaactgctacttccccctccagtcctacggattccgcccaacctacggcgtgggtcaccagccataccgcgtggttgtgctgagcttcgaactgctgcacgcccccgctaccgtgtgtggccctaagaagagcactaacctcgttaagaacaagtccgtgaacttcaacttcaacggtctctacgaaaaccagaagctgatcgctaaccagttcaactccgccatcggcaagatccaggactccctgtcctccacagcttccgctctgggcaagctgcaggacgttgtgaaccaaaacgctcaggccctgaacacactggtgaagcaactgaagaaccacaccagccccgacgttgacctgggtgacatcagcggtatcaacgctagcgtggtgaacatccagaaggagatcgacaggctgaacgaagtggctaagaacttgaacgagagcctcatcgacctgcaggaactgtaa

SEQ ID NO: 15 - DNA, 1479 bp, synthetic construct
  source 1..1479: mol_type = other DNA
atgctgctggtgaaccagagccaccagggtttcaacaaggaacacactagcaagatggtgtctgctatcgtcctctacgtgctgctcgccgccgctgctcactcagctttcgccgctgactctatccacatcaaggactccgacgacctcaagaaccgtttggccgaagccggcgacaagctggtcgttatcgacttcatggctacctggtgtggcccttgcaagatgatcggacctaagctggacgaaatggctaacgagatgagcgacagcatcgtcgttctgaaggtggacgtcgacgaatgtgaggacatcgccactgagtacaacatcaacagcatgcctaccttcgttttcgtgaagaactctaagaagatcgaggagttctctggtgccaacgtggacaagctccgtaacaccatcatcaagctcaagctggccggcagcggtagcggtcacatgcaccaccaccaccaccattcaagcggcgacgacgacgacaaggtgcagccaaccgaatcaatcgtccgcttcccaaacatcactaacctgtgcccattcgacgaggtgttcaacgccacccgtttcgcctctgtctacgcttggaaccgcaagcgcatctccaactgtgtcgccgactacagcgtgctgtacaacttcgctcctttcttcgcattcaagtgttacggagtgtcccctaccaagctcaacgatttgtgcttcacaaacgtgtacgctgacagcttcgtgatccgtggtaacgaggtttctcaaatcgcccctggtcagacaggtaacatcgctgactacaactacaagctcccagacgacttcactggctgtgttatcgcttggaactcaaacaagctggactctaaggtgggtggtaactacaactaccagtaccgtctgttccgcaagagcaacctcaagccattcgaacgtgacatcagcacagagatctaccaagccggtaacaagccctgcaacggcgttgccggattcaactgctacttccccctccgttcctacggattccgcccaacctacggcgtgggtcaccagccataccgcgtggttgtgctgagcttcgaactgctgcacgcccccgctaccgtgtgtggccctaagaagagcactaacctcgttaagaacaagtccgtgaacttcaacttcaacggtctctacgaaaaccagaagctgatcgctaaccagttcaactccgccatcggcaagatccaggactccctgtcctccacagcttccgctctgggcaagctgcaggacgttgtgaaccaaaacgctcaggccctgaacacactggtgaagcaactgaagaaccacaccagccccgacgttgacctgggtgacatcagcggtatcaacgctagcgtggtgaacatccagaaggagatcgacaggctgaacgaagtggctaagaacttgaacgagagcctcatcgacctgcaggaactgtaa

SEQ ID NO: 16 - DNA, 1479 bp, synthetic construct; identical to SEQ ID NO: 14
  source 1..1479: mol_type = other DNA

SEQ ID NO: 17 - DNA, 1479 bp, synthetic construct
  source 1..1479: mol_type = other DNA
atgctgctggtgaaccagagccaccagggtttcaacaaggaacacactagcaagatggtgtctgctatcgtcctctacgtgctgctcgccgccgctgctcactcagctttcgccgctgactctatccacatcaaggactccgacgacctcaagaaccgtttggccgaagccggcgacaagctggtcgttatcgacttcatggctacctggtgtggcccttgcaagatgatcggacctaagctggacgaaatggctaacgagatgagcgacagcatcgtcgttctgaaggtggacgtcgacgaatgtgaggacatcgccactgagtacaacatcaacagcatgcctaccttcgttttcgtgaagaactctaagaagatcgaggagttctctggtgccaacgtggacaagctccgtaacaccatcatcaagctcaagctggccggcagcggtagcggtcacatgcaccaccaccaccaccattcaagcggcgacgacgacgacaaggtgcagccaaccgaatcaatcgtccgcttcccaaacatcactaacctgtgcccattcgacgaggtgttcaacgccacccgtttcgcctctgtctacgcttggaaccgcaagcgcatctccaactgtgtcgccgactacagcgtgctgtacaacttcgctcctttcttcgcattcaagtgttacggagtgtcccctaccaagctcaacgatttgtgcttcacaaacgtgtacgctgacagcttcgtgatccgtggtaacgaggtttctcaaatcgcccctggtcagacaggtaacatcgctgactacaactacaagctcccagacgacttcactggctgtgttatcgcttggaactcaaacaagctggactctacggtgggtggtaactacaactaccggtaccgtctgttccgcaagagcaagctcaagccattcgaacgtgacatcagcacagagatctaccaagccggtaacaagccctgcaacggcgttgccggagtcaactgctacttccccctccagtcctacggattccgcccaacctacggcgtgggtcaccagccataccgcgtggttgtgctgagcttcgaactgctgcacgcccccgctaccgtgtgtggccctaagaagagcactaacctcgttaagaacaagtccgtgaacttcaacttcaacggtctctacgaaaaccagaagctgatcgctaaccagttcaactccgccatcggcaagatccaggactccctgtcctccacagcttccgctctgggcaagctgcaggacgttgtgaaccaaaacgctcaggccctgaacacactggtgaagcaactgaagaaccacaccagccccgacgttgacctgggtgacatcagcggtatcaacgctagcgtggtgaacatccagaaggagatcgacaggctgaacgaagtggctaagaacttgaacgagagcctcatcgacctgcaggaactgtaa

SEQ ID NO: 18 - protein, 801 aa, synthetic construct
MDAMKRGLCCVLLLCGAVFVSPVQPTESIVRFPNITNLCPFDEVFNATRFASVYAWNRKRISNCVADYSVLYNLAPFFTFKCYGVSPTKLNDLCFTNVYADSFVIRGDEVRQIAPGQTGNIADYNYKLPDDFTGCVIAWNSNKLDSKVSGNYNYLYRLFRKSNLKPFERDISTEIYQAGNKPCNGVAGFNCYFPLRSYSFRPTYGVGHQPYRVVVLSFELLHAPATVCGPKKSTNLVKNKSVNFNFNGLYENQKLIANQFNSAIGKIQDSLSSTASALGKLQDVVNQNAQALNTLVKQLVQPTESIVRFPNITNLCPFGEVFNATRFASVYAWNRKRISNCVADYSVLYNSASFSTFKCYGVSPTKLNDLCFTNVYADSFVIRGDEVRQIAPGQTGKIADYNYKLPDDFTGCVIAWNSNNLDSKVGGNYNYRYRLFRKSNLKPFERDISTEIYQAGSKPCNGVEGFNCYFPLQSYGFQPTNGVGYQPYRVVVLSFELLHAPATVCGPKKSTNLVKNKSVNFNFNGKNHTSPDVDLGDISGINASVVNIQKEIDRLNEVAKNLNESLIDLQELGKYVQPTESIVRFPNITNLCPFGEVFNATRFASVYAWNRKRISNCVADYSVLYNSASFSTFKCYGVSPTKLNDLCFTNVYADSFVIRGDEVRQIAPGQTGNIADYNYKLPDDFTGCVIAWNSNNLDSKVGGNYNYLYRLFRKSNLKPFERDISTEIYQAGSTPCNGVKGFNCYFPLQSYGFQPTYGVGYQPYRVVVLSFELLHAPATVCGPKKSTNLVKNKSVNFNFNG

SEQ ID NO: 19 - DNA, 2406 bp, synthetic construct
  source 1..2406: mol_type = other DNA
atggacgccatgaagagaggcctgtgctgcgtgctgctcctgtgcggcgccgtgttcgtgagccccgtgcaacccaccgaaagcattgtgcggtttcccaatatcaccaacctctgtcctttcgacgaggtgttcaacgccacaagatttgctagcgtgtacgcctggaaccggaagagaatctccaattgtgtcgccgactatagcgtcctctataacctggcccccttcttcacattcaagtgctacggcgtgtcccccacaaagctgaacgacctgtgctttaccaatgtgtacgccgacagcttcgtcatcagaggggacgaggtccggcagatcgctcctgggcagaccggcaatatcgccgactacaactataagctccctgacgacttcaccgggtgcgtcattgcttggaactccaacaagctggattccaaagtgagcgggaactacaactatctctacagactgttcagaaagagcaacctgaaacctttcgaaagagacatctccacagagatctaccaagccggcaacaagccctgcaacggcgtggccggctttaattgttacttccccctcagaagctacagcttcagacccacctacggcgtgggccatcagccctatagagtcgtggtgctgtccttcgaactgctgcacgcccccgccaccgtgtgtggccccaagaaaagcacaaatctggtcaagaataagagcgtcaattttaatttcaacggcctgtacgagaatcagaagctgatcgccaatcagttcaacagcgccatcggcaagatccaagacagcctgagcagcaccgctagcgccctgggcaagctgcaagacgtggtgaatcagaacgcccaagccctgaacaccctggtgaagcagctggtgcagcccaccgaatccattgtcagattccccaacatcaccaacctgtgcccctttggcgaagtgtttaacgccacccggttcgctagcgtgtatgcctggaaccggaagagaattagcaactgcgtggccgattacagcgtgctctataacagcgctagcttcagcacctttaagtgctatggcgtgagccctaccaagctgaatgacctctgcttcaccaacgtgtatgctgatagcttcgtgatcagaggcgacgaagtgagacagatcgcccctgggcagaccggcaagattgccgactacaattataagctgcctgatgatttcaccggctgcgtgatcgcctggaacagcaacaacctggattccaaggtcgggggcaattacaattacagatacagactcttcagaaagtccaacctgaagcccttcgagagagacatcagcaccgagatctatcaagccgggagcaagccctgtaacggcgtggagggcttcaattgctactttcccctgcagtcctatgggtttcagcccaccaacggggtgggctatcagccctatagagtcgtcgtcctcagcttcgaactgctgcacgctcctgctacagtgtgcgggcccaagaagagcaccaatctcgtcaagaataaaagcgtcaacttcaacttcaacggcaagaaccacacaagccccgacgtggacctgggcgacatcagcggcatcaacgctagcgtggtgaacattcagaaggagatcgacagactgaacgaggtggccaagaacctgaacgagagcctgatcgacctgcaagagctgggcaagtacgtgcagcccaccgagagcatcgtgagattccccaatatcacaaatctctgcccttttggcgaggtgtttaacgctacaagattcgctagcgtctacgcctggaacagaaaacggatcagcaattgtgtggccgactatagcgtgctgtacaattccgctagcttcagcacattcaaatgctacggggtgtcccccaccaagctgaacgatctctgcttcaccaacgtctacgccgacagcttcgtgattagaggcgacgaggtcagacaaatcgcccctgggcagaccggcaacatcgctgactataattacaagctgcctgacgatttcaccgggtgtgtgatcgcctggaactccaacaatctggactccaaggtggggggcaactataactacctgtacagactctttagaaagagcaatctcaagcccttcgaacgggatattagcaccgaaatttaccaagccggctccacaccctgtaacggcgtgaaggggttcaactgctatttccccctgcagagctacggctttcagcccacctacggcgtggggtatcagccttaccgggtggtcgtgctcagcttcgagctgctgcatgctcctgccaccgtctgtgggcctaagaagagcaccaacctggtgaagaacaaatccgtgaacttcaactttaacggctga

SEQ ID NO: 20 - protein, 801 aa, synthetic construct
MDAMKRGLCCVLLLCGAVFVSPVQPTESIVRFPNITNLCPFDEVFNATRFASVYAWNRKRISNCVADYSVLYNFAPFFAFKCYGVSPTKLNDLCFTNVYADSFVIRGNEVSQIAPGQTGNIADYNYKLPDDFTGCVIAWNSNKLDSKVGGNYNYRYRLFRKSNLKPFERDISTEIYQAGNKPCNGVAGVNCYFPLQSYGFRPTYGVGHQPYRVVVLSFELLHAPATVCGPKKSTNLVKNKSVNFNFNGLYENQKLIANQFNSAIGKIQDSLSSTASALGKLQDVVNQNAQALNTLVKQLVQPTESIVRFPNITNLCPFGEVFNATRFASVYAWNRKRISNCVADYSVLYNSASFSTFKCYGVSPTKLNDLCFTNVYADSFVIRGDEVRQIAPGQTGKIADYNYKLPDDFTGCVIAWNSNNLDSKVGGNYNYRYRLFRKSNLKPFERDISTEIYQAGSKPCNGVEGFNCYFPLQSYGFQPTNGVGYQPYRVVVLSFELLHAPATVCGPKKSTNLVKNKSVNFNFNGKNHTSPDVDLGDISGINASVVNIQKEIDRLNEVAKNLNESLIDLQELGKYVQPTESIVRFPNITNLCPFGEVFNATRFASVYAWNRKRISNCVADYSVLYNSASFSTFKCYGVSPTKLNDLCFTNVYADSFVIRGDEVRQIAPGQTGKIADYNYKLPDDFTGCVIAWNSNNLDSKVGGNYNYLYRLFRKSNLKPFERDISTEIYQAGSTPCNGVEGFNCYFPLQSYGFQPTNGVGYQPYRVVVLSFELLHAPATVCGPKKSTNLVKNKSVNFNFNG

SEQ ID NO: 21 - DNA, 2406 bp, synthetic construct
  source 1..2406: mol_type = other DNA
atggacgccatgaagagaggcctgtgctgcgtgctgctcctgtgcggcgccgtgttcgtgagccccgtgcaacccaccgagagcattgtgagattccccaatatcaccaacctctgccccttcgacgaagtgtttaacgccacaagattcgctagcgtctacgcttggaatagaaagcggatcagcaactgcgtcgctgattactccgtgctgtacaacttcgcccccttcttcgctttcaagtgttacggggtgagccctaccaagctgaacgacctctgtttcaccaatgtgtacgccgatagcttcgtgatccggggcaacgaagtgagccaaatcgcccccggccaaaccggcaatatcgctgactacaactacaagctccctgatgacttcaccggctgtgtgatcgcttggaacagcaacaagctggacagcaaagtgggcgggaattataactacagataccggctcttccggaagagcaacctcaagccttttgagcgggacatctccaccgaaatctaccaagccggcaataaaccctgcaatggcgtggccggcgtgaactgctacttccctctgcaaagctacggctttagacccacctacggcgtgggccatcagccctacagagtggtcgtgctcagctttgagctgctccacgctcctgctacagtctgcggccctaaaaagagcacaaacctcgtcaagaacaaaagcgtgaacttcaactttaacggcctgtatgagaatcagaagctgatcgccaatcagttcaacagcgccatcggcaagatccaagacagcctgagcagcaccgctagcgccctgggcaagctgcaagacgtggtgaatcagaacgcccaagccctgaacaccctggtgaagcagctggtgcagcctaccgagtccatcgtgcggttccccaacatcacaaacctgtgtccctttggggaagtctttaacgccacccggttcgctagcgtgtatgcctggaatagaaagagaattagcaattgcgtggctgactatagcgtgctgtacaacagcgcctccttctccacatttaagtgctacggcgtgagccccacaaagctgaatgatctctgcttcaccaacgtgtacgccgacagcttcgtcattagaggcgatgaagtgagacagatcgctcctgggcagaccggcaaaattgctgactacaactataagctgcccgacgatttcaccggctgcgtgattgcctggaacagcaataacctggacagcaaggtcggcggcaactataactacagatacagactgttccggaagtccaacctgaagcccttcgagagagacatctccaccgagatctatcaagccggcagcaagccctgcaacggcgtggagggctttaactgctatttccccctgcagagctacggctttcagcctacaaacggcgtggggtatcagccctacagagtcgtggtcctgagctttgaactgctccatgctcccgctaccgtgtgtggccccaagaagagcaccaacctcgtgaaaaacaagtccgtgaatttcaacttcaacgggaagaaccacacaagccccgacgtggacctgggcgacatcagcggcatcaacgctagcgtggtgaacattcagaaggagatcgacagactgaacgaggtggccaagaacctgaacgagagcctgatcgacctgcaagagctgggcaagtacgtgcagcccacagagagcatcgtgcggttccccaacatcaccaatctgtgtcccttcggcgaggtcttcaatgccacccggttcgctagcgtgtatgcttggaacagaaaacggatcagcaattgcgtggccgactacagcgtgctgtataatagcgctagcttcagcaccttcaaatgttatggcgtctcccccaccaagctgaatgacctgtgtttcacaaacgtgtatgccgactccttcgtgatcagaggcgacgaggtcagacagattgcccctgggcagaccggcaagatcgccgactacaactacaaactgcccgatgacttcaccggctgcgtgatcgcctggaattccaacaatctggactccaaagtgggcgggaactacaactacctgtaccggctgtttagaaaaagcaacctgaaacctttcgagcgggatattagcacagaaatctatcaagccgggagcaccccctgcaatggggtggagggcttcaattgctacttccccctgcaatcctatgggtttcagcccaccaacggcgtgggctaccaaccctatagagtggtggtcctcagctttgagctgctgcacgcccccgccaccgtgtgcgggcccaaaaagagcaccaacctggtcaagaacaagtccgtcaactttaactttaacggctga

SEQ ID NO: 22 - protein, 867 aa, synthetic construct
MDAMKRGLCCVLLLCGAVFVSPVQPTESIVRFPNITNLCPFDEVFNATRFASVYAWNRKRISNCVADYSVLYNFAPFFAFKCYGVSPTKLNDLCFTNVYADSFVIRGNEVSQIAPGQTGNIADYNYKLPDDFTGCVIAWNSNKLDSKVGGNYNYRYRLFRKSNLKPFERDISTEIYQAGNKPCNGVAGVNCYFPLQSYGFRPTYGVGHQPYRVVVLSFELLHAPATVCGPKKSTNLVKNKSVNFNFNGTQNVLYENQKLIANQFNSAIGKIQDSLSSTASALGKLQDVVNQNAQALNTLVKQLSSNFGAISSVLNDILSRLDKVEVQPTESIVRFPNITNLCPFGEVFNATRFASVYAWNRKRISNCVADYSVLYNSASFSTFKCYGVSPTKLNDLCFTNVYADSFVIRGDEVRQIAPGQTGKIADYNYKLPDDFTGCVIAWNSNNLDSKVGGNYNYRYRLFRKSNLKPFERDISTEIYQAGSKPCNGVEGFNCYFPLQSYGFQPTNGVGYQPYRVVVLSFELLHAPATVCGPKKSTNLVKNKSVNFNFNGVYDPLQPELDSFKEELDKYFKNHTSPDVDLGDISGINASVVNIQKEIDRLNEVAKNLNESLIDLQELGKYGKYEQYIKWPWYIWLGFIAGVQPTESIVRFPNITNLCPFGEVFNATRFASVYAWNRKRISNCVADYSVLYNSASFSTFKCYGVSPTKLNDLCFTNVYADSFVIRGDEVRQIAPGQTGKIADYNYKLPDDFTGCVIAWNSNNLDSKVGGNYNYLYRLFRKSNLKPFERDISTEIYQAGSTPCNGVEGFNCYFPLQSYGFQPTNGVGYQPYRVVVLSFELLHAPATVCGPKKSTNLVKNKSVNFNFNG

SEQ ID NO: 23 - DNA, 2604 bp, synthetic construct
  source 1..2604: mol_type = other DNA
atggacgccatgaagagaggcctgtgctgcgtgctgctcctgtgcggcgccgtgttcgtgagccccgtgcaacctaccgagagcattgtccggttccccaatattaccaacctctgccccttcgacgaggtctttaacgctacaagattcgcctccgtgtacgcctggaaccggaagagaatcagcaattgcgtcgccgactactccgtgctctacaactttgcccccttcttcgctttcaagtgctacggcgtgagccccacaaagctcaacgacctgtgcttcaccaacgtgtacgccgacagctttgtcatcagaggcaacgaggtgagccaaattgcccctggccaaaccggcaacatcgccgattacaactacaagctccccgacgacttcaccggctgtgtgattgcttggaacagcaataagctcgacagcaaggtggggggcaactacaattaccggtaccggctgttccggaagtccaatctgaagcctttcgagagagacatcagcaccgagatctaccaagccgggaacaaaccctgcaatggcgtggccggcgtgaactgctacttccctctgcagagctacgggtttcggcccacctacggcgtgggccaccaaccctacagagtggtggtcctgagcttcgagctgctgcacgcccctgctacagtgtgtggccccaagaaaagcaccaatctcgtgaagaacaagagcgtcaacttcaattttaacggcacacagaacgtgctgtacgagaatcagaagctgatcgccaatcagttcaacagcgccatcggcaagatccaagacagcctgagcagcaccgctagcgccctgggcaagctgcaagacgtggtgaatcagaacgcccaagccctgaacaccctggtgaagcagctgagcagcaacttcggcgccatcagcagcgtgctgaacgacatcctgagcagactggacaaggtggaggtgcagcctacagagtccatcgtcagattccccaacatcaccaacctgtgccccttcggcgaggtgtttaatgccacacggttcgctagcgtgtacgcctggaatcggaagcggatctccaactgcgtcgctgactattccgtgctctataactccgctagcttcagcacatttaagtgctatggggtgtcccccaccaagctgaatgacctgtgcttcacaaacgtctacgccgactcctttgtcatccggggcgacgaagtccggcagatcgcccctgggcagaccggcaaaatcgctgactacaactacaaactgcccgatgacttcaccggctgtgtgatcgcctggaactccaacaatctggactccaaggtcggcggcaattacaattacagatacagactgttcagaaaatccaacctgaaacccttcgagcgggacatttccacagagatctatcaagccggcagcaaaccttgcaacggcgtggaggggttcaactgctattttcccctgcagagctacgggtttcagcccaccaacggcgtcggctaccaaccctatcgggtggtcgtgctgagcttcgaactcctgcacgctcccgccacagtctgcgggcctaaaaagagcaccaacctggtgaagaataaatccgtcaatttcaacttcaacggcgtgtacgaccccctgcagcccgagctggacagcttcaaggaggagctggacaagtacttcaagaaccacacaagccccgacgtggacctgggcgacatcagcggcatcaacgctagcgtggtgaacattcagaaggagatcgacagactgaacgaggtggccaagaacctgaacgagagcctgatcgacctgcaagagctgggcaagtacggcaagtacgagcagtacatcaagtggccctggtacatctggctgggcttcatcgccggcgtgcagcccaccgagagcatcgtccggtttcccaacattaccaacctgtgtcccttcggcgaggtcttcaatgccacacggttcgctagcgtctatgcctggaaccggaagagaattagcaactgcgtggccgactatagcgtcctgtacaacagcgctagcttctccaccttcaagtgttatggcgtgtcccccaccaagctgaatgacctctgttttaccaatgtctatgccgacagcttcgtgatcagaggcgatgaagtgagacagatcgcccctgggcagaccgggaagatcgccgactacaactataagctccccgatgacttcaccggctgcgtcattgcttggaactccaataatctggacagcaaggtggggggcaattataactacctgtatcggctgttcagaaagagcaacctgaagccttttgagagagatatcagcaccgaaatttatcaagccgggagcaccccctgcaacggggtggaaggcttcaactgttacttccccctgcagagctacggctttcagcctaccaacggggtggggtatcagccttatagagtcgtggtcctgtccttcgagctgctgcacgcccccgccacagtgtgcgggcccaagaagagcaccaatctggtgaaaaacaaaagcgtcaacttcaatttcaacggctga

SEQ ID NO: 24 - DNA, 3822 bp, synthetic construct
  source 1..3822: mol_type = other DNA
atgttcgtgttcctggtgctgctgcccctggtgagcagccagtgtgtgaacctgacaacaaggacccagctgcctcccgcctacaccaacagcttcacaaggggcgtgtactaccctgacaaggtgttcaggagcagcgtgctgcactccacacaggacctgttcctgcccttcttctccaacgtgacatggttccacgccatccacgtgtccggcaccaacggcacaaagagattcgacaaccccgtgctgcctttcaacgacggcgtgtacttcgcctccacagagaagtccaacatcatcaggggctggatcttcggcacaacactggacagcaagacacagagcctgctgatcgtgaacaacgccacaaacgtggtcattaaggtgtgtgagttccagttctgcaacgaccccttcctgggcgtgtactatcacaagaacaacaagagctggatggagagcgagttcagggtgtactccagcgccaacaactgtacattcgagtacgtgtcccagcctttcctgatggacctggagggcaagcagggcaacttcaagaacctgagggagttcgtgttcaagaacatcgacggctacttcaagatctactccaagcacacccccatcaacctggtgagagacctgcctcagggcttctccgccctggagcctctggtggacctgcccatcggcatcaacatcacaagattccagacactgctggccctgcacagaagctacctgacccccggcgattccagcagcggctggaccgctggcgccgctgcttactacgtgggctacctgcagcccaggacattcctgctgaagtacaacgagaacggcacaatcaccgatgccgtggattgcgccctggatcctctgagcgagaccaagtgtacactgaagtccttcacagtggagaagggcatctaccagacctccaacttcagagtgcagcccacagagagcatcgtgagattccctaacatcacaaacctgtgccctttcggcgaggtgttcaacgccacaaggttcgccagcgtgtacgcctggaacagaaagaggatcagcaactgcgtggccgattacagcgtgctgtacaactccgcctccttctccacattcaagtgctacggcgtgtcccccaccaagctgaacgatctgtgtttcaccaacgtgtacgccgactccttcgtgatcagaggcgacgaggtgaggcagatcgcccccggacagaccggcaagatcgccgattacaactacaagctgcccgatgacttcaccggctgtgtgatcgcctggaactccaacaacctggattccaaggtgggcggcaactacaactacctgtacagactgttcagaaagtccaacctgaagcccttcgagagagatatctccaccgagatctaccaggccggctccacaccttgtaacggcgtggagggcttcaactgctacttccccctgcagagctacggcttccagcctaccaacggcgtgggctaccagccttacagagtggtggtgctgtccttcgagctgctgcacgcccccgccacagtgtgtggcccaaagaagtccaccaacctggtgaagaacaagtgtgtgaacttcaacttcaacggcctgaccggcacaggcgtgctgaccgagagcaacaagaagttcctgcctttccagcagttcggcagagacatcgccgataccacagacgccgtgagagaccctcagaccctggagatcctggatatcaccccttgcagcttcggcggcgtgtccgtgatcacccctggcacaaacaccagcaaccaggtggccgtgctgtaccaggacgtgaactgtacagaggtgcccgtggccatccacgccgaccagctgacccccacatggagagtgtactccaccggctccaacgtgttccagacaagggccggctgcctgatcggcgccgagcatgtgaacaacagctacgagtgtgacatccctatcggcgccggcatctgcgccagctaccagacccagaccaacagccccaggagggccagatccgtggccagccagagcatcatcgcctacaccatgtccctgggcgccgagaacagcgtggcctactccaacaacagcatcgccatccccaccaacttcacaatctccgtgaccaccgagatcctgcccgtgagcatgaccaagacatccgtggattgtaccatgtacatctgcggcgacagcacagagtgctccaacctgctgctgcagtacggctccttctgtacccagctgaacagggccctgacaggcatcgccgtggagcaggacaagaacacccaggaggtgttcgcccaggtgaagcagatctacaagacacctcccatcaaggacttcggcggcttcaacttctcccagatcctgcccgacccttccaagccctccaagagatccttcatcgaggacctgctgttcaacaaggtgaccctggccgatgccggcttcatcaagcagtacggcgactgcctgggcgacatcgccgccagagacctgatctgcgcccagaagttcaacggcctcaccgtgctgccccctctgctgaccgatgagatgatcgcccagtacaccagcgccctgctggccggaacaatcaccagcggctggacattcggcgccggcgctgctctgcagatccctttcgccatgcagatggcctacaggttcaacggcatcggcgtgacccagaacgtgctgtacgagaaccagaagctgatcgccaaccagttcaacagcgccatcggcaagatccaggattccctgagcagcacagccagcgccctgggcaagctgcaggatgtggtgaaccagaacgcccaggccctgaacacactggtgaagcagctgagcagcaacttcggcgccatcagcagcgtgctcaacgacatcctgagcagactggataaggtggaggccgaggtgcagatcgatagactgatcaccggcaggctgcagtccctgcagacatacgtgacccagcagctgatcagagccgccgagatcagggccagcgccaacctggccgccaccaagatgtccgagtgtgtgctgggccagagcaagagggtggacttctgtggcaagggctaccacctgatgtccttccctcagtccgccccccacggcgtggtgttcctgcacgtgacatacgtgcctgcccaggagaagaacttcacaacagcccctgccatctgtcacgacggcaaggcccacttccccagggagggcgtgttcgtgagcaacggcacccactggttcgtgacccagaggaacttctacgagcctcagatcatcacaaccgataacacattcgtgagcggcaactgtgatgtggtcattggcatcgtgaacaataccgtgtacgatcccctgcagcctgagctggactccttcaaggaggagctggataagtacttcaagaaccacacctcccccgacgtggatctgggcgacattagcggcatcaacgcctccgtggtgaacatccagaaggagatcgacaggctgaacgaggtggccaagaacctgaacgagtccctgatcgatctgcaggagctgggcaagtacgagcagtacatcaagtggccctggtacatctggctgggcttcatcgccggcctgatcgccatcgtgatggtgacaatcatgctgtgttgcatgacatcctgttgttcctgtctgaagggctgttgtagctgtggctcctgttgcaagttcgacgaggatgactccgagcccgtgctgaagggcgtgaagctgcactacacctga

SEQ ID NO: 25 - protein, 1273 aa, synthetic construct
MFVFLVLLPLVSSQCVNLTTRTQLPPAYTNSFTRGVYYPDKVFRSSVLHSTQDLFLPFFSNVTWFHAIHVSGTNGTKRFDNPVLPFNDGVYFASTEKSNIIRGWIFGTTLDSKTQSLLIVNNATNVVIKVCEFQFCNDPFLGVYYHKNNKSWMESEFRVYSSANNCTFEYVSQPFLMDLEGKQGNFKNLREFVFKNIDGYFKIYSKHTPINLVRDLPQGFSALEPLVDLPIGINITRFQTLLALHRSYLTPGDSSSGWTAGAAAYYVGYLQPRTFLLKYNENGTITDAVDCALDPLSETKCTLKSFTVEKGIYQTSNFRVQPTESIVRFPNITNLCPFGEVFNATRFASVYAWNRKRISNCVADYSVLYNSASFSTFKCYGVSPTKLNDLCFTNVYADSFVIRGDEVRQIAPGQTGKIADYNYKLPDDFTGCVIAWNSNNLDSKVGGNYNYLYRLFRKSNLKPFERDISTEIYQAGSTPCNGVEGFNCYFPLQSYGFQPTNGVGYQPYRVVVLSFELLHAPATVCGPKKSTNLVKNKCVNFNFNGLTGTGVLTESNKKFLPFQQFGRDIADTTDAVRDPQTLEILDITPCSFGGVSVITPGTNTSNQVAVLYQDVNCTEVPVAIHADQLTPTWRVYSTGSNVFQTRAGCLIGAEHVNNSYECDIPIGAGICASYQTQTNSPRRARSVASQSIIAYTMSLGAENSVAYSNNSIAIPTNFTISVTTEILPVSMTKTSVDCTMYICGDSTECSNLLLQYGSFCTQLNRALTGIAVEQDKNTQEVFAQVKQIYKTPPIKDFGGFNFSQILPDPSKPSKRSFIEDLLFNKVTLADAGFIKQYGDCLGDIAARDLICAQKFNGLTVLPPLLTDEMIAQYTSALLAGTITSGWTFGAGAALQIPFAMQMAYRFNGIGVTQNVLYENQKLIANQFNSAIGKIQDSLSSTASALGKLQDVVNQNAQALNTLVKQLSSNFGAISSVLNDILSRLDKVEAEVQIDRLITGRLQSLQTYVTQQLIRAAEIRASANLAATKMSECVLGQSKRVDFCGKGYHLMSFPQSAPHGVVFLHVTYVPAQEKNFTTAPAICHDGKAHFPREGVFVSNGTHWFVTQRNFYEPQIITTDNTFVSGNCDVVIGIVNNTVYDPLQPELDSFKEELDKYFKNHTSPDVDLGDISGINASVVNIQKEIDRLNEVAKNLNESLIDLQELGKYEQYIKWPWYIWLGFIAGLIAIVMVTIMLCCMTSCCSCLKGCCSCGSCCKFDEDDSEPVLKGVKLHYT

SEQ ID NO: 26 - DNA, 3813 bp, synthetic construct
  source 1..3813: mol_type = other DNA
atgttcgtgttcctggtgctgctgcccctggtgagcagccaatgcgtgaacctgaccacaagaacacagctgccccccgcctacaccaacagcttcacaagaggcgtgtattatcccgacaaggtgttcagaagcagcgtgctgcacagcacccaagacctgtttctgccttttttcagcaacgtgacctggttccacgccatccacgtgagcggcaccaacggcaccaagagattcgccaaccccgtgctgcccttcaacgacggcgtgtacttcgctagcaccgagaagagcaacatcatcagaggctggatcttcggcaccaccctggatagcaagacacagagcctgctgatcgtgaacaacgccaccaacgtggtgatcaaggtgtgcgagtttcagttctgcaacgaccccttcctgggcgtgtattaccacaagaacaacaagagctggatggagagcgagttcagagtctacagcagcgccaacaactgcaccttcgagtacgtgagccaacccttcctgatggacctggagggcaagcaaggcaatttcaagaacctgagagagttcgtgttcaagaacatcgacggctacttcaagatctacagcaagcacacccccatcaacctggtgagaggcctgccccaaggcttcagcgccctggagcccctggtggacctgcccatcggcatcaacatcacaagatttcagacactgcaccggtcctatctcacccctggcgacagcagcagcgggtggaccgctggcgccgccgcttactacgtgggctacctgcagcctagaaccttcctgctgaagtacaacgagaacggcaccattaccgacgccgtggactgcgccctggaccccctgagcgagaccaagtgcaccctgaagagcttcaccgtggagaagggcatctatcagacaagcaacttcagagtgcagcccaccgagagcatcgtgagattccccaacatcaccaacctgtgccccttcggcgaggtgttcaacgccacaagattcgctagcgtgtacgcctggaaccggaaaagaatcagcaactgcgtggccgactacagcgtgctgtacaacagcgctagcttcagcaccttcaagtgctacggcgtgagccccaccaagctgaacgacctgtgcttcaccaacgtgtacgccgacagcttcgtgatcagaggcgacgaggtgagacagatcgcccccgggcagaccggcaacatcgccgactacaactacaagctgcccgacgacttcaccggctgcgtgatcgcctggaacagcaataacctggacagcaaggtgggcggcaactacaactacctgtacagactgttcagaaagagcaacctgaagcccttcgagagagacatcagcaccgagatctaccaagccggcagcaccccctgcaacggcgtgaagggcttcaactgctacttccccctgcagagctacggctttcagcccacctacggcgtgggctatcagccctacagagtggtcgtgctgagcttcgagctgctgcacgcccctgccaccgtgtgtggccccaagaagagcaccaacctggtgaagaacaagtgcgtgaacttcaacttcaacgggctgaccgggaccggcgtgctgaccgagagcaacaagaagtttctgccctttcaacagttcggcagagacatcgccgacaccaccgacgccgtccgggaccctcagaccctggagatcctggacatcaccccctgctccttcggcggcgtgagcgtgatcacccccggcaccaacacaagcaaccaagtggccgtgctgtaccaaggcgtgaactgcaccgaggtgcccgtggccatccacgccgatcagctgacccccacctggagagtgtacagcaccggcagcaacgtgtttcagacaagagccggctgcctgatcggcgccgagcacgtgaacaacagctacgagtgcgacatccccatcggcgccggcatctgcgctagctatcagacacagaccaacagccctagaagagctagaagcgtggctagccaaagcatcatcgcctacaccatgagcctgggcgtggagaacagcgtggcctacagcaacaacagcatcgccatccccaccaacttcaccatcagcgtgaccaccgaaatcctgcccgtgagcatgaccaagacaagcgtggactgcaccatgtacatctgcggcgacagcaccgagtgcagcaacctgctcctgcagtacggcagcttctgcacacagctgaacagagccctgaccggcatcgccgtggagcaagacaagaacacccaagaggtgttcgcccaagtgaagcagatctacaagaccccccccatcaaggacttcggcggcttcaacttcagccaaattctgcccgaccctagcaagcctagcaagagaagcttcatcgaggacctgctgttcaacaaggtgaccctggccgacgccggcttcatcaagcagtacggcgactgcctgggcgatatcgctgctagagacctgatctgcgctcagaagttcaacggcctgaccgtgctcccccccctgctgaccgacgagatgatcgctcagtacacaagcgctctgctcgccgggaccatcacatccgggtggacattcggggccggcgctgccctgcagatccccttcgccatgcagatggcctacagattcaacggcatcggcgtgacacagaacgtgctgtacgagaatcagaagctgatcgccaatcagttcaacagcgccatcggcaagatccaagacagcctgagcagcaccgctagcgccctgggcaagctgcaagacgtggtgaatcagaacgcccaagccctgaacaccctggtgaagcagctgagcagcaacttcggcgccatcagctccgtgctgaacgacatcctgagcagactggacccccccgaggccgaggtgcagattgacagactgatcaccggcagactgcagagcctgcagacctacgtgacacagcagctgatcagagccgccgagatcagagctagcgccaacctggccgccaccaagatgagcgagtgcgtgctggggcagagcaagagagtggacttctgcggcaagggctaccacctgatgagcttccctcagagcgccccccacggcgtggtgttcctgcacgtgacctacgtgcccgcccaagagaagaacttcaccaccgcccccgccatctgccacgacggcaaggcccacttccctagagagggcgtgttcgtgagcaacggcacccactggttcgtgacacagagaaacttctacgagcctcagatcatcaccaccgacaacaccttcgtgagcggcaactgcgacgtggtgatcggcattgtgaacaataccgtgtacgaccccctgcagcccgagctggacagcttcaaggaggagctggacaagtacttcaagaaccacacaagccccgacgtggacctgggcgacattagcggcatcaacgctagcgtggtgaacattcagaaggagatcgacagactgaacgaggtggccaagaacctgaacgagagcctgatcgacctgcaagagctgggcaagtacgagcagtacatcaagtggccctggtacatctggctgggcttcatcgccggcctgatcgccatcgtgatggtgaccatcatgctgtgctgcatgacaagctgttgcagctgcctgaagggctgctgcagctgcgggagctgctgcaagttcgacgaggacgacagcgagcccgtgctgaagggcgtgaagctgcactacacctga

SEQ ID NO: 27 - protein, 1270 aa, synthetic construct
MFVFLVLLPLVSSQCVNLTTRTQLPPAYTNSFTRGVYYPDKVFRSSVLHSTQDLFLPFFSNVTWFHAIHVSGTNGTKRFANPVLPFNDGVYFASTEKSNIIRGWIFGTTLDSKTQSLLIVNNATNVVIKVCEFQFCNDPFLGVYYHKNNKSWMESEFRVYSSANNCTFEYVSQPFLMDLEGKQGNFKNLREFVFKNIDGYFKIYSKHTPINLVRGLPQGFSALEPLVDLPIGINITRFQTLHRSYLTPGDSSSGWTAGAAAYYVGYLQPRTFLLKYNENGTITDAVDCALDPLSETKCTLKSFTVEKGIYQTSNFRVQPTESIVRFPNITNLCPFGEVFNATRFASVYAWNRKRISNCVADYSVLYNSASFSTFKCYGVSPTKLNDLCFTNVYADSFVIRGDEVRQIAPGQTGNIADYNYKLPDDFTGCVIAWNSNNLDSKVGGNYNYLYRLFRKSNLKPFERDISTEIYQAGSTPCNGVKGFNCYFPLQSYGFQPTYGVGYQPYRVVVLSFELLHAPATVCGPKKSTNLVKNKCVNFNFNGLTGTGVLTESNKKFLPFQQFGRDIADTTDAVRDPQTLEILDITPCSFGGVSVITPGTNTSNQVAVLYQGVNCTEVPVAIHADQLTPTWRVYSTGSNVFQTRAGCLIGAEHVNNSYECDIPIGAGICASYQTQTNSPRRARSVASQSIIAYTMSLGVENSVAYSNNSIAIPTNFTISVTTEILPVSMTKTSVDCTMYICGDSTECSNLLLQYGSFCTQLNRALTGIAVEQDKNTQEVFAQVKQIYKTPPIKDFGGFNFSQILPDPSKPSKRSFIEDLLFNKVTLADAGFIKQYGDCLGDIAARDLICAQKFNGLTVLPPLLTDEMIAQYTSALLAGTITSGWTFGAGAALQIPFAMQMAYRFNGIGVTQNVLYENQKLIANQFNSAIGKIQDSLSSTASALGKLQDVVNQNAQALNTLVKQLSSNFGAISSVLNDILSRLDPPEAEVQIDRLITGRLQSLQTYVTQQLIRAAEIRASANLAATKMSECVLGQSKRVDFCGKGYHLMSFPQSAPHGVVFLHVTYVPAQEKNFTTAPAICHDGKAHFPREGVFVSNGTHWFVTQRNFYEPQIITTDNTFVSGNCDVVIGIVNNTVYDPLQPELDSFKEELDKYFKNHTSPDVDLGDISGINASVVNIQKEIDRLNEVAKNLNESLIDLQELGKYEQYIKWPWYIWLGFIAGLIAIVMVTIMLCCMTSCCSCLKGCCSCGSCCKFDEDDSEPVLKGVKLHYT

SEQ ID NO: 28 - DNA, 3816 bp, synthetic construct
  source 1..3816: mol_type = other DNA
atgttcgtgttcctggtgctgctgcccctggtgagcagccaatgcgtgaacctgagaacaagaacacagctgccccccgcctacaccaacagcttcacaagaggggtctactaccccgacaaggtgttcagaagcagcgtgctgcacagcacccaagacctgttcctgcccttcttctccaacgtgacctggttccacgccatccacgtgagcggcaccaacggcaccaagagattcgacaaccccgtgctgcccttcaacgacggcgtgtacttcgctagcaccgagaagagcaacatcatcagaggctggatcttcggcaccaccctggacagcaagacacagagcctgctgattgtgaacaacgctaccaacgtggtgatcaaggtgtgcgagtttcagttctgcaacgaccccttcctgggggtgtactaccacaaaaacaacaagagctggatggagagcggcgtgtacagcagcgccaacaactgcaccttcgagtacgtgagccaacccttcctgatggacctggagggcaagcaaggcaacttcaagaacctcagagagttcgtgttcaagaacatcgacggctacttcaagatctacagcaagcacacccccatcaacctggtgagagacctgccccaaggcttcagcgccctggagcccctggtggacctgcccatcggcatcaacatcacaagatttcagaccctgctggccctgcacagaagctacctgacacccggcgacagcagcagcgggtggacagccggcgctgccgcttactacgtgggctacctgcagcctagaaccttcctgctgaagtacaacgagaacggcaccattaccgacgccgtcgactgcgccctggaccccctgagcgagaccaagtgcaccctgaagagcttcaccgtggagaagggcatctatcagacaagcaacttcagagtgcagcccaccgagagcatcgtgagattccccaacatcaccaacctgtgccccttcggcgaggtgttcaacgccacaagattcgctagcgtgtacgcctggaacagaaagagaatcagcaactgcgtggccgactacagcgtgctgtacaacagcgctagcttcagcaccttcaaatgctacggggtcagccccaccaagctgaacgacctgtgcttcaccaacgtgtacgccgacagcttcgtgatcagaggcgacgaggtgagacagatcgcccccgggcagaccggcaagatcgccgactacaactacaagctgcccgacgacttcaccggctgcgtgatcgcctggaactccaacaacctggatagcaaggtgggcggcaactacaactatagatacagactgttcagaaagagcaacctgaagcccttcgagagagacatcagcaccgagatctaccaagccggcagcaagccctgcaacggcgtggagggcttcaactgctacttccccctgcagagctacggctttcagcccaccaacggcgtgggctatcagccctacagagtggtcgtgctgagcttcgagctgctgcacgcccctgccaccgtgtgcggccccaagaagagcaccaacctggtgaagaacaagtgcgtgaacttcaacttcaacggcctgaccggcaccggcgtgctgaccgagagcaacaagaagttcctcccttttcagcagttcggcagagacatcgccgacaccaccgatgccgtgagagaccctcagaccctggagatcctggacatcaccccctgcagctttggcggcgtgagcgtgatcacccccggcaccaacacaagcaaccaagtggccgtgctgtaccaaggcgtgaactgcaccgaggtgcccgtggccatccacgccgatcagctgacccccacctggagagtgtacagcaccggcagcaacgtgtttcagacaagagccggctgcctgatcggcgccgagcacgtgaacaacagctacgagtgcgacatccccatcggcgccggcatctgcgctagctatcagacacagaccaacagcagacggagagctagaagcgtggctagccaaagcatcatcgcctacaccatgagcctgggcgccgagaacagcgtggcctacagcaacaacagcatcgccatccccaccaacttcaccatcagcgtgaccaccgagatcctgcccgtctccatgaccaagacaagcgtggactgcaccatgtacatctgcggcgacagcaccgagtgcagcaacctgctcctgcagtacggcagcttctgcacacagctgaacagagccctgaccggcatcgccgtggagcaagacaagaacacccaagaggtgttcgcccaagtgaagcagatctacaagaccccccccatcaaggacttcggcggcttcaacttcagccaaatcctgcccgaccctagcaagcctagcaagagaagcttcatcgaggacctgctgttcaacaaggtgaccctggccgacgccggcttcatcaagcagtacggcgactgcctgggcgacatcgccgctagagacctgatctgcgctcagaagttcaatggcctgaccgtcctgccccccctgctgaccgacgagatgatcgctcagtacacaagcgccctgctggccggcacaattacaagcggctggacattcggcgctggcgccgccctgcaaatccccttcgccatgcagatggcctacagattcaacggcatcggcgtgacacagaacgtgctgtacgagaatcagaagctgatcgccaatcagttcaacagcgccatcggcaagatccaagacagcctgagcagcaccgctagcgccctgggcaagctgcagaacgtggtgaatcagaacgcccaagccctgaacaccctggtgaagcagctgagcagcaacttcggcgccatcagctccgtgctgaacgatatcctgagcagactggacccccccgaggccgaggtgcagatcgaccggctgatcaccggcagactgcagagcctgcagacctacgtgacacagcagctgatcagagccgccgagatcagagctagcgccaacctggccgccaccaagatgagcgagtgcgtgctggggcagagcaagagagtggacttctgcggcaagggctaccacctgatgagcttccctcagagcgccccccacggcgtggtgttcctgcacgtgacctacgtgcccgcccaagagaagaacttcaccaccgcccccgccatctgccacgacggcaaggcccacttccctagagagggcgtgttcgtgagcaacggcacccactggttcgtgacacagagaaacttctacgagcctcagatcatcaccaccgacaacaccttcgtgagcggcaactgcgacgtggtgatcggcattgtgaacaatacagtctacgaccctctgcagcccgagctggacagcttcaaggaggagctggacaagtacttcaagaatcacacaagccccgacgtggacctgggggacatcagcggcatcaacgctagcgtggtgaacattcagaaggagatcgacagactgaacgaggtggccaagaacctgaacgagagcctgatcgacctgcaagagctgggcaagtacgagcagtacatcaagtggccctggtacatctggctgggcttcatcgccggcctgatcgccatcgtgatggtgaccatcatgctgtgctgcatgacaagctgctgcagctgcctgaagggctgctgctcctgcggcagctgctgcaagttcgacgaggacgacagcgagcccgtgctgaagggcgtgaagctgcactacacctga

SEQ ID NO: 29 - protein, 1271 aa, synthetic construct
MFVFLVLLPLVSSQCVNLRTRTQLPPAYTNSFTRGVYYPDKVFRSSVLHSTQDLFLPFFSNVTWFHAIHVSGTNGTKRFDNPVLPFNDGVYFASTEKSNIIRGWIFGTTLDSKTQSLLIVNNATNVVIKVCEFQFCNDPFLGVYYHKNNKSWMESGVYSSANNCTFEYVSQPFLMDLEGKQGNFKNLREFVFKNIDGYFKIYSKHTPINLVRDLPQGFSALEPLVDLPIGINITRFQTLLALHRSYLTPGDSSSGWTAGAAAYYVGYLQPRTFLLKYNENGTITDAVDCALDPLSETKCTLKSFTVEKGIYQTSNFRVQPTESIVRFPNITNLCPFGEVFNATRFASVYAWNRKRISNCVADYSVLYNSASFSTFKCYGVSPTKLNDLCFTNVYADSFVIRGDEVRQIAPGQTGKIADYNYKLPDDFTGCVIAWNSNNLDSKVGGNYNYRYRLFRKSNLKPFERDISTEIYQAGSKPCNGVEGFNCYFPLQSYGFQPTNGVGYQPYRVVVLSFELLHAPATVCGPKKSTNLVKNKCVNFNFNGLTGTGVLTESNKKFLPFQQFGRDIADTTDAVRDPQTLEILDITPCSFGGVSVITPGTNTSNQVAVLYQGVNCTEVPVAIHADQLTPTWRVYSTGSNVFQTRAGCLIGAEHVNNSYECDIPIGAGICASYQTQTNSRRRARSVASQSIIAYTMSLGAENSVAYSNNSIAIPTNFTISVTTEILPVSMTKTSVDCTMYICGDSTECSNLLLQYGSFCTQLNRALTGIAVEQDKNTQEVFAQVKQIYKTPPIKDFGGFNFSQILPDPSKPSKRSFIEDLLFNKVTLADAGFIKQYGDCLGDIAARDLICAQKFNGLTVLPPLLTDEMIAQYTSALLAGTITSGWTFGAGAALQIPFAMQMAYRFNGIGVTQNVLYENQKLIANQFNSAIGKIQDSLSSTASALGKLQNVVNQNAQALNTLVKQLSSNFGAISSVLNDILSRLDPPEAEVQIDRLITGRLQSLQTYVTQQLIRAAEIRASANLAATKMSECVLGQSKRVDFCGKGYHLMSFPQSAPHGVVFLHVTYVPAQEKNFTTAPAICHDGKAHFPREGVFVSNGTHWFVTQRNFYEPQIITTDNTFVSGNCDVVIGIVNNTVYDPLQPELDSFKEELDKYFKNHTSPDVDLGDISGINASVVNIQKEIDRLNEVAKNLNESLIDLQELGKYEQYIKWPWYIWLGFIAGLIAIVMVTIMLCCMTSCCSCLKGCCSCGSCCKFDEDDSEPVLKGVKLHYT

SEQ ID NO: 30 - DNA, 3813 bp, synthetic construct
  source 1..3813: mol_type = other DNA
atgttcgtgttcctggtgctgctgcccctggtgagcagccaatgcgtgaacctgaccacaagaacacagctgccccccgcctacaccaacagcttcacaagaggcgtgtattatcccgacaaggtgttcagaagcagcgtgctgcacagcacccaagacctgtttctgcccttcttcagcaacgtgacctggttccacgccatccacgtgagcggcaccaacggcaccaagagattcgccaaccccgtgctgcccttcaacgacggcgtgtacttcgctagcaccgagaagagcaacatcatcagaggctggatcttcggcaccaccctggatagcaagacacagagcctgctgatcgtgaacaacgccaccaacgtggtgatcaaggtgtgcgagtttcagttctgcaacgaccccttcctgggcgtgtattaccacaagaacaacaagagctggatggagagcgagttcagagtctacagcagcgccaacaactgcaccttcgagtacgtgagccaacccttcctgatggacctggagggcaagcaaggcaatttcaagaacctgagagagttcgtgttcaagaacatcgacggctacttcaagatctacagcaagcacacccccatcaacctggtgagaggcctgccccaaggcttcagcgccctggagcccctggtggacctgcccatcggcatcaacatcacaagatttcagaccctgcaccggagctatctgacccctggcgactcctcctccgggtggaccgctggcgccgccgcttactacgtgggctacctgcagcctagaaccttcctgctgaagtacaacgagaacggcaccattacagacgccgtggattgcgccctggaccccctgagcgagaccaagtgcaccctgaagagcttcaccgtggagaagggcatctatcagacaagcaacttcagagtgcagcccaccgagagcatcgtgagattccccaacatcaccaacctgtgccccttcggcgaggtgttcaacgccacaagattcgctagcgtgtacgcctggaacagaaaaagaatcagcaactgcgtggccgactacagcgtgctgtacaacagcgctagcttcagcaccttcaagtgctacggcgtgagccccaccaagctgaacgacctgtgcttcaccaacgtgtacgccgacagcttcgtgatcagaggcgacgaggtgagacagatcgcccccgggcagaccggcaacatcgccgactacaactataagctccccgacgacttcaccggctgcgtgatcgcttggaactccaacaacctggacagcaaggtgggcggcaactacaactacagatatagactgttcagaaagagcaacctgaagcccttcgagagagacatcagcaccgagatctaccaagccggcagcaagccctgcaacggcgtgaagggcttcaactgctacttccccctgcagagctacggctttcagcccacctacggcgtgggctatcagccctacagagtggtcgtgctgagcttcgagctgctgcacgcccccgccaccgtctgcggccccaagaagagcaccaacctggtgaagaacaagtgcgtgaacttcaacttcaacgggctgaccggcaccggcgtgctgaccgagagcaacaagaagttcctgccctttcagcagttcggcagagacatcgccgacaccaccgacgccgtgagagaccctcagaccctggagatcctggacatcacaccctgcagcttcggcggcgtgagcgtgatcacccccggcaccaacacaagcaaccaagtggccgtgctgtaccaaggcgtgaactgcaccgaggtgcccgtggccatccacgccgatcagctgacccccacctggagagtctatagcaccggcagcaacgtgtttcagacaagagccggctgcctgatcggcgccgagcacgtgaacaacagctacgagtgcgacatccccatcggcgccggcatctgcgctagctatcagacacagaccaacagccctagaagagctagaagcgtggctagccaaagcatcatcgcctacaccatgagcctgggcgtggagaacagcgtggcctacagcaacaacagcatcgccatccccaccaacttcaccatcagcgtgaccaccgagatcctccctgtgagcatgaccaagacaagcgtggactgcaccatgtacatctgcggcgacagcaccgagtgcagcaacctgctcctgcagtacggcagcttctgcacacagctgaacagagccctgaccggcatcgccgtggagcaagacaagaacacccaagaggtgttcgcccaagtgaagcagatctacaagaccccccccatcaaggacttcggcggcttcaacttcagccaaatcctgcccgaccctagcaagcctagcaagagaagcttcatcgaggacctgctgttcaacaaggtgaccctggccgacgccggcttcatcaagcagtacggcgactgcctgggcgacatcgccgctagagacctgatctgcgctcagaagttcaacggcctgaccgtgctgccccccctgctgaccgacgagatgatcgctcaatacacaagcgccctcctggccgggacaatcacatccggctggaccttcggcgccggggctgccctgcagatccccttcgccatgcagatggcctacagattcaacggcatcggcgtgacacagaacgtgctgtacgagaatcagaagctgatcgccaatcagttcaacagcgccatcggcaagatccaagacagcctgagcagcaccgctagcgccctgggcaagctgcaagacgtggtgaatcagaacgcccaagccctgaacaccctggtgaagcagctgagcagcaacttcggcgccatcagcagcgtgctgaacgacatcctgagcagactggacccccccgaggccgaggtgcagatcgatagactgatcaccggcagactgcagagcctgcagacctacgtgacacagcagctgatcagagccgccgagatcagagctagcgccaacctggccgccaccaagatgagcgagtgcgtgctggggcagagcaagagagtggacttctgcggcaagggctaccacctgatgagcttccctcagagcgccccccacggcgtggtgttcctgcacgtgacctacgtgcccgcccaagagaagaacttcaccaccgctcccgccatctgccacgacggcaaggcccacttccctagagagggcgtgttcgtgagcaacggcacccactggttcgtgacacagagaaacttctacgagcctcagatcatcaccaccgacaacaccttcgtgagcggcaactgcgacgtggtgatcggcatcgtgaacaataccgtctacgaccccctgcaacccgagctggacagcttcaaggaggagctggacaagtacttcaagaaccacacaagccccgacgtggacctgggcgatatcagcggcatcaacgctagcgtggtgaacattcagaaggaaatcgatcggctgaatgaggtggccaagaacctgaacgagagcctgatcgacctgcaagagctgggcaagtacgagcagtacatcaagtggccctggtacatctggctgggcttcatcgccggcctgatcgccatcgtgatggtgaccatcatgctgtgctgcatgacaagctgctgcagctgcctgaagggctgctgtagctgtggcagctgctgcaagttcgacgaggacgacagcgagcccgtgctgaagggcgtgaagctgcactacacctga

SEQ ID NO: 31 - protein, 1270 aa, synthetic construct
MFVFLVLLPLVSSQCVNLTTRTQLPPAYTNSFTRGVYYPDKVFRSSVLHSTQDLFLPFFSNVTWFHAIHVSGTNGTKRFANPVLPFNDGVYFASTEKSNIIRGWIFGTTLDSKTQSLLIVNNATNVVIKVCEFQFCNDPFLGVYYHKNNKSWMESEFRVYSSANNCTFEYVSQPFLMDLEGKQGNFKNLREFVFKNIDGYFKIYSKHTPINLVRGLPQGFSALEPLVDLPIGINITRFQTLHRSYLTPGDSSSGWTAGAAAYYVGYLQPRTFLLKYNENGTITDAVDCALDPLSETKCTLKSFTVEKGIYQTSNFRVQPTESIVRFPNITNLCPFGEVFNATRFASVYAWNRKRISNCVADYSVLYNSASFSTFKCYGVSPTKLNDLCFTNVYADSFVIRGDEVRQIAPGQTGNIADYNYKLPDDFTGCVIAWNSNNLDSKVGGNYNYRYRLFRKSNLKPFERDISTEIYQAGSKPCNGVKGFNCYFPLQSYGFQPTYGVGYQPYRVVVLSFELLHAPATVCGPKKSTNLVKNKCVNFNFNGLTGTGVLTESNKKFLPFQQFGRDIADTTDAVRDPQTLEILDITPCSFGGVSVITPGTNTSNQVAVLYQGVNCTEVPVAIHADQLTPTWRVYSTGSNVFQTRAGCLIGAEHVNNSYECDIPIGAGICASYQTQTNSPRRARSVASQSIIAYTMSLGVENSVAYSNNSIAIPTNFTISVTTEILPVSMTKTSVDCTMYICGDSTECSNLLLQYGSFCTQLNRALTGIAVEQDKNTQEVFAQVKQIYKTPPIKDFGGFNFSQILPDPSKPSKRSFIEDLLFNKVTLADAGFIKQYGDCLGDIAARDLICAQKFNGLTVLPPLLTDEMIAQYTSALLAGTITSGWTFGAGAALQIPFAMQMAYRFNGIGVTQNVLYENQKLIANQFNSAIGKIQDSLSSTASALGKLQDVVNQNAQALNTLVKQLSSNFGAISSVLNDILSRLDPPEAEVQIDRLITGRLQSLQTYVTQQLIRAAEIRASANLAATKMSECVLGQSKRVDFCGKGYHLMSFPQSAPHGVVFLHVTYVPAQEKNFTTAPAICHDGKAHFPREGVFVSNGTHWFVTQRNFYEPQIITTDNTFVSGNCDVVIGIVNNTVYDPLQPELDSFKEELDKYFKNHTSPDVDLGDISGINASVVNIQKEIDRLNEVAKNLNESLIDLQELGKYEQYIKWPWYIWLGFIAGLIAIVMVTIMLCCMTSCCSCLKGCCSCGSCCKFDEDDSEPVLKGVKLHYT

SEQ ID NO: 32 - DNA, 3813 bp, synthetic construct
  source 1..3813: mol_type = other DNA
atgttcgtgttcctggtgctgctgcccctggtgagcagccaatgcgtgaacctgaccacaagaacacagctgccccccgcctacaccaacagcttcacaagaggcgtgtactaccccgacaaggtgttcagaagcagcgtcctccacagcacccaagacctgttcctgcccttcttcagcaacgtgacctggttccacgtgatcagcggcaccaacggcaccaagagattcgacaaccccgtgctgcccttcaacgacggcgtgtacttcgctagcatcgagaagagcaacatcatcagaggctggatcttcggcaccaccctggacagcaagacacagagcctgctgatcgtcaacaacgccaccaacgtggtgatcaaggtgtgcgagtttcagttctgcaacgaccccttcctggaccacaagaacaacaagagctggatggagagcgagttcagagtgtatagcagcgctaacaactgcaccttcgagtacgtgagccaacccttcctgatggacctggagggcaagcaaggcaacttcaaaaacctgagagagttcgtgttcaagaacatcgacggctacttcaagatctacagcaagcacacccccatcatcgtgagagagcccgaggacctgccccaaggcttcagcgccctggagcccctggtggacctgcccatcggcatcaacatcacaagatttcagaccctgctggccctgcacagatcctatctgacccctggggacagcagcagcggctggaccgctggcgctgccgcctactacgtgggctacctgcagcctagaaccttcctgctgaagtacaacgagaacggcacaatcaccgatgccgtcgactgcgccctggaccccctgagcgagaccaagtgcaccctgaagagcttcaccgtggagaagggcatctatcagacaagcaacttcagagtgcagcccaccgagagcatcgtgagattccccaacatcaccaacctgtgccccttcgacgaggtgttcaacgccacaagattcgctagcgtgtacgcctggaatagaaagagaatcagcaactgcgtggccgactacagcgtgctgtacaacctggcccccttcttcaccttcaaatgctacggcgtgagccccaccaagctgaacgacctgtgcttcaccaacgtgtacgccgacagcttcgtgatcagaggcgacgaggtgagacagatcgcccccgggcagaccggcaacatcgccgactacaactacaagctgcccgacgacttcaccggctgcgtgatcgcctggaacagcaacaagctcgacagcaaggtgagcggcaactacaactacctgtacagactgttcagaaagagcaacctgaagcccttcgagagagacatcagcaccgagatctaccaagccggcaacaagccctgcaacggcgtggccggcttcaactgctacttccccctgagaagctacagcttcagacccacctacggcgtgggccatcagccctacagagtggtcgtgctgagcttcgagctgctgcacgcccccgccaccgtgtgcggccccaagaagagcaccaacctggtgaagaacaagtgcgtgaacttcaacttcaacggcctgaagggcaccggcgtgctgaccgagagcaacaagaagtttctgccctttcagcagttcggcagagacatcgccgacaccaccgacgccgtgagagaccctcagaccctggagatcctggacatcaccccctgctccttcggcggcgtgagcgtgatcacccccggcaccaacacaagcaaccaagtggccgtgctgtaccaaggcgtgaactgcaccgaggtgcccgtggccatccacgccgatcagctgacccccacctggagagtgtacagcaccggcagcaacgtgtttcagacaagagccggctgcctgatcggcgccgagtacgtgaacaacagctacgagtgcgacatccccatcggcgccggcatctgcgctagctatcagacacagaccaagagccacagaagagctagaagcgtggctagccaaagcatcatcgcctacaccatgagcctgggcgccgagaacagcgtggcctacagcaacaacagcatcgccatccccaccaacttcaccatcagcgtgaccaccgaaattctgcccgtgagcatgaccaagacaagcgtggactgcaccatgtacatctgcggcgacagcaccgagtgcagcaacctgctcctgcagtacggcagcttctgcacacagctgaagagagccctgaccggcatcgccgtggagcaagacaagaacacccaagaggtgttcgcccaagtgaagcagatctacaagaccccccccatcaagtacttcggcggcttcaacttcagccaaatcctgcccgaccctagcaagcctagcaagagaagcttcatcgaggacctgctgttcaacaaggtgaccctggccgacgccggcttcatcaagcagtacggcgactgcctgggcgatattgccgctagagacctgatctgcgctcagaagttcaagggcctgaccgtgctgccccccctgctgaccgacgagatgatcgctcagtatacaagcgccctcctcgctgggaccatcacaagcggctggacattcggggccggcgctgccctgcagatccccttcgccatgcagatggcctacagattcaacggcatcggcgtgacacagaacgtgctgtacgagaatcagaagctgatcgccaatcagttcaacagcgccatcggcaagatccaagacagcctgagcagcaccgctagcgccctgggcaagctgcaagacgtggtgaaccacaacgcccaagccctgaacaccctggtgaagcagctgagcagcaagttcggcgccatcagcagcgtgctgaacgacatcttcagcagactggacccccccgaggccgaggtgcagatcgaccggctcatcaccggcagactgcagagcctgcagacctacgtgacacagcagctgatcagagccgccgagatcagagctagcgccaacctggccgccaccaagatgagcgagtgcgtgctggggcagagcaagagagtggacttctgcggcaagggctaccacctgatgagcttccctcagagcgccccccacggcgtggtgttcctgcacgtgacctacgtgcccgcccaagagaagaacttcaccaccgctcccgccatttgccacgacggcaaggcccacttccctagagagggcgtgttcgtgagcaacggcacccactggttcgtgacacagagaaacttctacgagcctcagatcatcaccaccgacaacaccttcgtcagcggcaactgtgacgtggtgatcggcatcgtgaacaataccgtgtacgaccccctgcagcccgaactggacagcttcaaggaggagctggacaagtacttcaagaaccacacaagccccgacgtggacctgggcgacattagcggcatcaacgctagcgtggtgaacattcagaaggagattgacagactgaacgaggtggccaagaacctgaacgagagcctgatcgacctgcaagagctgggcaagtacgagcagtacatcaagtggccctggtacatctggctgggcttcatcgccggcctgatcgccatcgtgatggtgaccatcatgctgtgctgcatgacaagctgctgtagctgcctgaaaggctgctgcagctgcggcagctgctgcaagttcgacgaggacgacagcgagcccgtgctgaagggcgtgaagctgcactacacctga

SEQ ID NO: 33 - protein, 1270 aa, synthetic construct
MFVFLVLLPLVSSQCVNLTTRTQLPPAYTNSFTRGVYYPDKVFRSSVLHSTQDLFLPFFSNVTWFHVISGTNGTKRFDNPVLPFNDGVYFASIEKSNIIRGWIFGTTLDSKTQSLLIVNNATNVVIKVCEFQFCNDPFLDHKNNKSWMESEFRVYSSANNCTFEYVSQPFLMDLEGKQGNFKNLREFVFKNIDGYFKIYSKHTPIIVREPEDLPQGFSALEPLVDLPIGINITRFQTLLALHRSYLTPGDSSSGWTAGAAAYYVGYLQPRTFLLKYNENGTITDAVDCALDPLSETKCTLKSFTVEKGIYQTSNFRVQPTESIVRFPNITNLCPFDEVFNATRFASVYAWNRKRISNCVADYSVLYNLAPFFTFKCYGVSPTKLNDLCFTNVYADSFVIRGDEVRQIAPGQTGNIADYNYKLPDDFTGCVIAWNSNKLDSKVSGNYNYLYRLFRKSNLKPFERDISTEIYQAGNKPCNGVAGFNCYFPLRSYSFRPTYGVGHQPYRVVVLSFELLHAPATVCGPKKSTNLVKNKCVNFNFNGLKGTGVLTESNKKFLPFQQFGRDIADTTDAVRDPQTLEILDITPCSFGGVSVITPGTNTSNQVAVLYQGVNCTEVPVAIHADQLTPTWRVYSTGSNVFQTRAGCLIGAEYVNNSYECDIPIGAGICASYQTQTKSHRRARSVASQSIIAYTMSLGAENSVAYSNNSIAIPTNFTISVTTEILPVSMTKTSVDCTMYICGDSTECSNLLLQYGSFCTQLKRALTGIAVEQDKNTQEVFAQVKQIYKTPPIKYFGGFNFSQILPDPSKPSKRSFIEDLLFNKVTLADAGFIKQYGDCLGDIAARDLICAQKFKGLTVLPPLLTDEMIAQYTSALLAGTITSGWTFGAGAALQIPFAMQMAYRFNGIGVTQNVLYENQKLIANQFNSAIGKIQDSLSSTASALGKLQDVVNHNAQALNTLVKQLSSKFGAISSVLNDIFSRLDPPEAEVQIDRLITGRLQSLQTYVTQQLIRAAEIRASANLAATKMSECVLGQSKRVDFCGKGYHLMSFPQSAPHGVVFLHVTYVPAQEKNFTTAPAICHDGKAHFPREGVFVSNGTHWFVTQRNFYEPQIITTDNTFVSGNCDVVIGIVNNTVYDPLQPELDSFKEELDKYFKNHTSPDVDLGDISGINASVVNIQKEIDRLNEVAKNLNESLIDLQELGKYEQYIKWPWYIWLGFIAGLIAIVMVTIMLCCMTSCCSCLKGCCSCGSCCKFDEDDSEPVLKGVKLHYT

SEQ ID NO: 34 - DNA, 3813 bp, synthetic construct
  source 1..3813: mol_type = other DNA
atgttcgtgttcctggtgctgctgcccctggtgagcagccaatgcgtgaacctgatcacaagaacacagagctacaccaacagcttcacaagaggcgtgtactaccccgacaaggtgttcagaagcagcgtcctccacagcacccaagacctgttcctgcctttctttagcaacgtgacctggttccacgccatccacgtgagcggcaccaacggcaccaagagattcgacaaccccgtgctgcccttcaacgacggcgtgtacttcgctagcaccgagaagagcaacatcatcagaggctggatcttcggcaccaccctggacagcaagacacagagcctgctgatcgtcaacaacgccaccaacgtggtgatcaaggtgtgcgagtttcagttctgcaacgaccccttcctggacgtgtactaccacaagaacaacaagagctggatggagagcgagttcagagtgtacagcagcgccaacaactgcaccttcgagtacgtgagccaacccttcctgatggacctggagggcaagcaaggcaacttcaaaaacctgagagagttcgtgttcaagaacatcgacggctacttcaagatctacagcaagcacacccccatcaacctgggcagagacctgccccaaggcttcagcgccctggagcccctggtggacctgcccatcggcatcaacatcacaagatttcagaccctgctggccctgcacagatcctacctcacacctggcgacagcagctccggctggaccgctggcgctgccgcttactacgtgggctacctgcagcctagaaccttcctgctgaagtacaacgagaacggcacaatcaccgatgccgtcgactgcgccctggaccccctgagcgagaccaagtgcaccctgaagagcttcaccgtggagaagggcatctatcagacaagcaacttcagagtgcagcccaccgagagcatcgtgagattccccaacatcaccaacctgtgccccttcgacgaggtgttcaacgccacaagattcgctagcgtgtacgcctggaacagaaaaagaatcagcaactgcgtggccgactacagcgtgctgtacaacttcgcccccttcttcgccttcaaatgctacggcgtgagccccaccaagctgaacgacctgtgcttcaccaacgtgtacgccgacagcttcgtgatcagaggcaacgaggtgagccaaatcgcccccgggcagaccggcaacatcgccgactacaactacaagctgcccgacgacttcaccggctgcgtgatcgcctggaactccaacaagctcgacagcaaggtgggcggcaactacaactacctgtacagactgttcagaaagagcaacctgaagcccttcgagagagacatcagcaccgagatctaccaagccggcaacaagccctgcaacggcgtggccggcttcaactgctacttccccctgagaagctacggcttcagacccacctacggcgtgggccatcagccctacagagtggtcgtgctgagcttcgagctgctgcacgcccccgccaccgtgtgcggccccaagaagagcaccaacctggtgaagaacaagtgcgtgaacttcaacttcaacggcctgaccggcaccggcgtgctgaccgagagcaacaagaagttcctcccctttcagcagttcggcagagacatcgccgacaccaccgacgccgtgagagaccctcagaccctggagatcctggacatcaccccctgcagcttcggcggcgtgagcgtgatcacccccggcaccaacacaagcaaccaagtggccgtgctgtaccaaggcgtgaactgcaccgaggtgcccgtggccatccacgccgatcagctgacccccacctggagagtgtactccaccggcagcaacgtgtttcagacaagagccggctgcctgatcggcgccgagtacgtgaacaacagctacgagtgcgacatccccatcggcgccggcatctgcgctagctatcagacacagaccaagagccacagaagagctagaagcgtggctagccaaagcatcatcgcctacaccatgagcctgggcgccgagaacagcgtggcctacagcaacaacagcatcgccatccccaccaacttcaccatcagcgtgaccaccgagatcctgcctgtgagcatgaccaagacaagcgtggactgcaccatgtacatctgcggcgacagcaccgagtgcagcaacctgctcctgcagtacggcagcttctgcacacagctgaagagagccctgaccggcatcgccgtggagcaagacaagaacacccaagaggtgttcgcccaagtgaagcagatctacaagaccccccccatcaagtacttcggcggcttcaacttcagccaaatcctgcccgaccctagcaagcctagcaagcggagcttcatcgaggacctgctgttcaacaaggtgaccctggccgacgccggcttcatcaagcagtacggcgactgcctcggcgacatcgccgctagagacctgatctgcgctcagaagttcaatggcctgaccgtgctgccccccctgctgaccgacgagatgatcgctcagtatacctccgccctgctcgccgggaccatcacaagcggctggaccttcggcgccggcgccgccctccaaatccccttcgccatgcagatggcctacagattcaacggcatcggcgtgacacagaacgtgctgtacgagaatcagaagctgatcgccaatcagttcaacagcgccatcggcaagatccaagacagcctgagcagcaccgctagcgccctgggcaagctgcaagacgtggtgaaccacaacgcccaagccctgaacaccctggtgaagcagctgagcagcaagttcggcgccatcagcagcgtgctgaacgatatcctgagcagactggacccccccgaggccgaggtgcagatcgatagactgatcaccggcagactgcagagcctgcagacctacgtgacacagcagctgatcagagccgccgagatcagagctagcgccaacctggccgccaccaagatgagcgagtgcgtgctggggcagagcaagagagtggacttctgcggcaagggctaccacctgatgagcttccctcagagcgccccccacggcgtggtgttcctgcacgtgacctacgtgcccgcccaagagaagaacttcacaaccgcccccgccatctgccacgacggcaaggcccacttccctagagagggcgtgttcgtgagcaacggcacccactggttcgtgacacagagaaacttctacgagcctcagatcatcaccaccgacaacaccttcgtgagcggcaactgcgacgtggtgatcgggatcgtgaacaacaccgtgtacgatcccctgcagcccgagctggacagcttcaaggaggagctggacaagtacttcaagaaccacacaagccccgacgtggacctgggcgacattagcggcatcaacgctagcgtggtgaacattcagaaggagatcgacagactgaatgaggtggccaagaacctgaacgagagcctgatcgacctgcaagagctgggcaagtacgagcagtacatcaagtggccctggtacatctggctgggcttcatcgccggcctgatcgccatcgtgatggtgaccatcatgctgtgctgcatgacaagctgctgtagctgcctgaagggctgctgcagctgcggctcctgctgcaagttcgacgaggacgacagcgagcccgtgctgaagggcgtgaagctgcactacacctga

SEQ ID NO: 35 - protein, 1270 aa, synthetic construct
MFVFLVLLPLVSSQCVNLITRTQSYTNSFTRGVYYPDKVFRSSVLHSTQDLFLPFFSNVTWFHAIHVSGTNGTKRFDNPVLPFNDGVYFASTEKSNIIRGWIFGTTLDSKTQSLLIVNNATNVVIKVCEFQFCNDPFLDVYYHKNNKSWMESEFRVYSSANNCTFEYVSQPFLMDLEGKQGNFKNLREFVFKNIDGYFKIYSKHTPINLGRDLPQGFSALEPLVDLPIGINITRFQTLLALHRSYLTPGDSSSGWTAGAAAYYVGYLQPRTFLLKYNENGTITDAVDCALDPLSETKCTLKSFTVEKGIYQTSNFRVQPTESIVRFPNITNLCPFDEVFNATRFASVYAWNRKRISNCVADYSVLYNFAPFFAFKCYGVSPTKLNDLCFTNVYADSFVIRGNEVSQIAPGQTGNIADYNYKLPDDFTGCVIAWNSNKLDSKVGGNYNYLYRLFRKSNLKPFERDISTEIYQAGNKPCNGVAGFNCYFPLRSYGFRPTYGVGHQPYRVVVLSFELLHAPATVCGPKKSTNLVKNKCVNFNFNGLTGTGVLTESNKKFLPFQQFGRDIADTTDAVRDPQTLEILDITPCSFGGVSVITPGTNTSNQVAVLYQGVNCTEVPVAIHADQLTPTWRVYSTGSNVFQTRAGCLIGAEYVNNSYECDIPIGAGICASYQTQTKSHRRARSVASQSIIAYTMSLGAENSVAYSNNSIAIPTNFTISVTTEILPVSMTKTSVDCTMYICGDSTECSNLLLQYGSFCTQLKRALTGIAVEQDKNTQEVFAQVKQIYKTPPIKYFGGFNFSQILPDPSKPSKRSFIEDLLFNKVTLADAGFIKQYGDCLGDIAARDLICAQKFNGLTVLPPLLTDEMIAQYTSALLAGTITSGWTFGAGAALQIPFAMQMAYRFNGIGVTQNVLYENQKLIANQFNSAIGKIQDSLSSTASALGKLQDVVNHNAQALNTLVKQLSSKFGAISSVLNDILSRLDPPEAEVQIDRLITGRLQSLQTYVTQQLIRAAEIRASANLAATKMSECVLGQSKRVDFCGKGYHLMSFPQSAPHGVVFLHVTYVPAQEKNFTTAPAICHDGKAHFPREGVFVSNGTHWFVTQRNFYEPQIITTDNTFVSGNCDVVIGIVNNTVYDPLQPELDSFKEELDKYFKNHTSPDVDLGDISGINASVVNIQKEIDRLNEVAKNLNESLIDLQELGKYEQYIKWPWYIWLGFIAGLIAIVMVTIMLCCMTSCCSCLKGCCSCGSCCKFDEDDSEPVLKGVKLHYT

SEQ ID NO: 36 - DNA, 3813 bp, synthetic construct
  source 1..3813: mol_type = other DNA
atgttcgtgttcctggtgctgctgcccctggtgagcagccaatgcgtgaacctgatcacaagaacacagagctacaccaacagcttcacaagaggcgtgtactaccccgacaaggtgttcagaagcagcgtcctccacagcacccaagacctgttcctgcctttctttagcaacgtgacctggttccacgccatccacgtgagcggcaccaacggcaccaagagattcgacaaccccgtgctgcccttcaacgacggcgtgtacttcgctagcaccgagaagagcaacatcatcagaggctggatcttcggcaccaccctggacagcaagacacagagcctgctgatcgtcaacaacgccaccaacgtggtgatcaaggtgtgcgagtttcagttctgcaacgaccccttcctggacgtgtactaccacaagaacaacaagagctggatggagagcgagttcagagtgtacagcagcgccaacaactgcaccttcgagtacgtgagccaacccttcctgatggacctggagggcaagcaaggcaacttcaaaaacctgagagagttcgtgttcaagaacatcgacggctacttcaagatctacagcaagcacacccccatcaacctgggcagagacctgccccaaggcttcagcgccctggagcccctggtggacctgcccatcggcatcaacatcacaagatttcagaccctgctggccctgcacagatcctacctcacacctggcgacagcagctccggctggaccgctggcgctgccgcttactacgtgggctacctgcagcctagaaccttcctgctgaagtacaacgagaacggcacaatcaccgatgccgtcgactgcgccctggaccccctgagcgagaccaagtgcaccctgaagagcttcaccgtggagaagggcatctatcagacaagcaacttcagagtgcagcccaccgagagcatcgtgagattccccaacatcaccaacctgtgccccttcgacgaggtgttcaacgccacaagattcgctagcgtgtacgcctggaacagaaaaagaatcagcaactgcgtggccgactacagcgtgctgtacaacttcgcccccttcttcgccttcaaatgctacggcgtgagccccaccaagctgaacgacctgtgcttcaccaacgtgtacgccgacagcttcgtgatcagaggcaacgaggtgagccaaatcgcccccgggcagaccggcaacatcgccgactacaactacaagctgcccgacgacttcaccggctgcgtgatcgcctggaactccaacaagctcgacagcaaggtgggcggcaactacaactatcagtacagactgttcagaaagagcaacctgaagcccttcgagagagacatcagcaccgagatctaccaagccggcaacaagccctgcaacggcgtggccggcttcaactgctacttccccctgagaagctacggcttcagacccacctacggcgtgggccatcagccctacagagtggtcgtgctgagcttcgagctgctgcacgcccccgccaccgtgtgcggccccaagaagagcaccaacctggtgaagaacaagtgcgtgaacttcaacttcaacggcctgaccggcaccggcgtgctgaccgagagcaacaagaagttcctcccctttcagcagttcggcagagacatcgccgacaccaccgacgccgtgagagaccctcagaccctggagatcctggacatcaccccctgcagcttcggcggcgtgagcgtgatcacccccggcaccaacacaagcaaccaagtggccgtgctgtaccaaggcgtgaactgcaccgaggtgcccgtggccatccacgccgatcagctgacccccacctggagagtgtactccaccggcagcaacgtgtttcagacaagagccggctgcctgatcggcgccgagtacgtgaacaacagctacgagtgcgacatccccatcggcgccggcatctgcgctagctatcagacacagaccaagagccacagaagagctagaagcgtggctagccaaagcatcatcgcctacaccatgagcctgggcgccgagaacctggtggcctacagcaacaacagcatcgccatccccaccaacttcaccatcagcgtgaccaccgagatcctgcctgtgagcatgaccaagacaagcgtggactgcaccatgtacatctgcggcgacagcaccgagtgcagcaacctgctcctgcagtacggcagcttctgcacacagctgaagagagccctgaccggcatcgccgtggagcaagacaagaacacccaagaggtgttcgcccaagtgaagcagatctacaagaccccccccatcaagtacttcggcggcttcaacttcagccaaatcctgcccgaccctagcaagcctagcaagcggagcttcatcgaggacctgctgttcaacaaggtgaccctggccgacgccggcttcatcaagcagtacggcgactgcctcggcgacatcgccgctagagacctgatctgcgctcagaagttcaatggcctgaccgtgctgccccccctgctgaccgacgagatgatcgctcagtatacctccgccctgctcgccgggaccatcacaagcggctggaccttcggcgccggcgccgccctccaaatccccttcgccatgcagatggcctacagattcaacggcatcggcgtgacacagaacgtgctgtacgagaatcagaagctgatcgccaatcagttcaacagcgccatcggcaagatccaagacagcctgagcagcaccgctagcgccctgggcaagctgcaagacgtggtgaaccacaacgcccaagccctgaacaccctggtgaagcagctgagcagcaagttcggcgccatcagcagcgtgctgaacgatatcctgagcagactggacccccccgaggccgaggtgcagatcgatagactgatcaccggcagactgcagagcctgcagacctacgtgacacagcagctgatcagagccgccgagatcagagctagcgccaacctggccgccaccaagatgagcgagtgcgtgctggggcagagcaagagagtggacttctgcggcaagggctaccacctgatgagcttccctcagagcgccccccacggcgtggtgttcctgcacgtgacctacgtgcccgcccaagagaagaacttcacaaccgcccccgccatctgccacgacggcaaggcccacttccctagagagggcgtgttcgtgagcaacggcacccactggttcgtgacacagagaaacttctacgagcctcagatcatcaccaccgacaacaccttcgtgagcggcaactgcgacgtggtgatcgggatcgtgaacaacaccgtgtacgatcccctgcagcccgagctggacagcttcaaggaggagctggacaagtacttcaagaaccacacaagccccgacgtggacctgggcgacattagcggcatcaacgctagcgtggtgaacattcagaaggagatcgacagactgaatgaggtggccaagaacctgaacgagagcctgatcgacctgcaagagctgggcaagtacgagcagtacatcaagtggccctggtacatctggctgggcttcatcgccggcctgatcgccatcgtgatggtgaccatcatgctgtgctgcatgacaagctgctgtagctgcctgaagggctgctgcagctgcggctcctgctgcaagttcgacgaggacgacagcgagcccgtgctgaagggcgtgaagctgcactacacctga

SEQ ID NO: 37 - protein, 1270 aa, synthetic construct
MFVFLVLLPLVSSQCVNLITRTQSYTNSFTRGVYYPDKVFRSSVLHSTQDLFLPFFSNVTWFHAIHVSGTNGTKRFDNPVLPFNDGVYFASTEKSNIIRGWIFGTTLDSKTQSLLIVNNATNVVIKVCEFQFCNDPFLDVYYHKNNKSWMESEFRVYSSANNCTFEYVSQPFLMDLEGKQGNFKNLREFVFKNIDGYFKIYSKHTPINLGRDLPQGFSALEPLVDLPIGINITRFQTLLALHRSYLTPGDSSSGWTAGAAAYYVGYLQPRTFLLKYNENGTITDAVDCALDPLSETKCTLKSFTVEKGIYQTSNFRVQPTESIVRFPNITNLCPFDEVFNATRFASVYAWNRKRISNCVADYSVLYNFAPFFAFKCYGVSPTKLNDLCFTNVYADSFVIRGNEVSQIAPGQTGNIADYNYKLPDDFTGCVIAWNSNKLDSKVGGNYNYQYRLFRKSNLKPFERDISTEIYQAGNKPCNGVAGFNCYFPLRSYGFRPTYGVGHQPYRVVVLSFELLHAPATVCGPKKSTNLVKNKCVNFNFNGLTGTGVLTESNKKFLPFQQFGRDIADTTDAVRDPQTLEILDITPCSFGGVSVITPGTNTSNQVAVLYQGVNCTEVPVAIHADQLTPTWRVYSTGSNVFQTRAGCLIGAEYVNNSYECDIPIGAGICASYQTQTKSHRRARSVASQSIIAYTMSLGAENLVAYSNNSIAIPTNFTISVTTEILPVSMTKTSVDCTMYICGDSTECSNLLLQYGSFCTQLKRALTGIAVEQDKNTQEVFAQVKQIYKTPPIKYFGGFNFSQILPDPSKPSKRSFIEDLLFNKVTLADAGFIKQYGDCLGDIAARDLICAQKFNGLTVLPPLLTDEMIAQYTSALLAGTITSGWTFGAGAALQIPFAMQMAYRFNGIGVTQNVLYENQKLIANQFNSAIGKIQDSLSSTASALGKLQDVVNHNAQALNTLVKQLSSKFGAISSVLNDILSRLDPPEAEVQIDRLITGRLQSLQTYVTQQLIRAAEIRASANLAATKMSECVLGQSKRVDFCGKGYHLMSFPQSAPHGVVFLHVTYVPAQEKNFTTAPAICHDGKAHFPREGVFVSNGTHWFVTQRNFYEPQIITTDNTFVSGNCDVVIGIVNNTVYDPLQPELDSFKEELDKYFKNHTSPDVDLGDISGINASVVNIQKEIDRLNEVAKNLNESLIDLQELGKYEQYIKWPWYIWLGFIAGLIAIVMVTIMLCCMTSCCSCLKGCCSCGSCCKFDEDDSEPVLKGVKLHYT

SEQ ID NO: 38 - DNA, 3807 bp, synthetic construct
  source 1..3807: mol_type = other DNA
atgttcgtgttcctggtgctgctgcccctggtgagcagccaatgcgtgaacctgatcacaagaacacagagctacaccaacagcttcacaagaggcgtgtactaccccgacaaggtgttcagaagcagcgtcctgcattccacccaagacctgtttctccccttcttcagcaacgtgacctggttccacgccatcagcggcaccaacggcaccaagagattcgacaaccccgtgctgcccttcaacgacggcgtgtacttcgctagcaccgagaagagcaacatcatcagaggctggatcttcggcaccaccctggacagcaagacacagagcctgctgatcgtgaacaacgccacaaacgtggtgatcaaggtgtgcgagtttcagttctgcaacgaccccttcctggacgtgtactaccacaagaacaacaagagctggatggagagcgagttccgggtgtacagcagcgccaacaactgcaccttcgagtacgtgagccaacccttcctgatggacctggagggcaagcaaggcaacttcaagaacctgagagagttcgtgttcaagaacatcgacggctacttcaagatctacagcaagcacacccccatcaacctgggcagagacctgccccaaggcttcagcgccctggagcccctggtggacctgcccatcggcatcaacatcacaagatttcagacactgctcgccctgcaccggagctacctcacccctggcgacagcagctccggctggaccgctggggctgccgcctactacgtgggctacctgcagcctagaaccttcctgctgaagtacaacgagaacggcaccatcaccgacgctgtggactgtgccctggaccccctgagcgagaccaagtgcaccctgaagagcttcaccgtggagaagggcatctatcagacaagcaacttcagagtgcagcccaccgagagcatcgtgagattccccaacatcaccaacctgtgccccttcgacgaggtgttcaacgccacaagattcgctagcgtgtacgcctggaacagaaagagaatcagcaactgcgtggccgactacagcgtgctgtacaacttcgcccccttcttcgccttcaaatgctacggcgtcagccccaccaagctgaacgacctgtgcttcaccaacgtgtacgccgacagcttcgtgatcagaggcaacgaggtgagccaaatcgcccccgggcagaccggcaacatcgccgactataactacaaactgcccgacgacttcaccggctgcgtgatcgcctggaactccaacaagctggacagcaaagtgggcggcaactacaactacagatacagactgttcagaaagagcaacctgaagcccttcgagagagacatcagcaccgagatctaccaagccggcaacaagccctgcaacggcgtggccggcgtgaactgctacttccccctgcagagctacggcttcagacccacctacggcgtgggccatcagccctacagagtggtcgtgctgagcttcgagctgctgcacgcccctgccacagtgtgcggccccaagaagagcaccaacctggtgaagaacaagtgcgtgaacttcaacttcaacggcctgaccggcaccggcgtgctgaccgagagcaacaagaagttcctgccctttcagcagttcggcagagacatcgccgacaccaccgatgctgtgagagaccctcagaccctggagatcctggacatcaccccttgcagcttcggcggcgtgagcgtgatcacccccggcaccaacacaagcaaccaagtggccgtgctgtaccaaggcgtcaactgcacagaggtgcccgtggccatccacgccgatcagctgacccccacctggagagtgtactccaccggcagcaacgtgtttcagacaagagccggctgcctgatcggcgccgagtacgtgaacaacagctacgagtgcgacatccccatcggcgccggcatctgcgctagctatcagacacagaccaagagccacagaagagctagaagcgtggctagccaaagcatcatcgcctacaccatgagcctgggcgccgagaacagcgtggcctacagcaacaacagcatcgccatccccaccaacttcaccatcagcgtgaccaccgagatcctgcctgtgagcatgaccaagacaagcgtggactgcaccatgtacatctgcggcgacagcaccgagtgcagcaacctgctcctgcagtacggcagcttctgcacacagctgaagagagccctgaccggcatcgccgtggagcaagacaagaacacccaagaggtgttcgcccaagtgaagcagatctacaagaccccccccatcaagtacttcggcggcttcaacttcagccaaatcctgcccgaccctagcaagcctagcaagcggagcttcatcgaggacctgctgttcaacaaggtgaccctggccgacgccggcttcatcaagcagtacggcgactgcctcggcgacatcgctgctagagacctgatctgcgctcagaagttcaacggcctcacagtgctgccccccctgctgaccgacgagatgatcgctcagtacacctccgctctgctggccggcacaattacatccggctggaccttcggcgccggcgccgccctgcaaatccccttcgccatgcagatggcctacagattcaacggcatcggcgtgacacagaacgtgctgtacgagaatcagaagctgatcgccaatcagttcaacagcgccatcggcaagatccaagacagcctgagcagcaccgctagcgccctgggcaagctgcaagacgtggtgaaccacaacgcccaagccctgaacaccctggtgaagcagctgagcagcaagttcggcgccatctcctccgtcctgaacgacatcctgagcagactggacccccccgaggccgaggtgcagattgacagactgattaccggcagactgcagagcctgcagacctacgtgacacagcagctgatcagagccgccgagatcagagctagcgccaacctggccgccaccaagatgagcgagtgcgtgctggggcagagcaagagagtggacttctgcggcaagggctaccacctgatgagcttccctcagagcgccccccacggcgtggtgttcctgcacgtgacctacgtgcccgcccaagagaagaacttcaccaccgctcccgccatctgccacgacggcaaggcccacttccctagagagggcgtgttcgtgagcaacggcacccactggttcgtgacacagagaaacttctacgagcctcagatcatcaccaccgacaacaccttcgtgagcggcaactgcgacgtggtgatcggcatcgtcaacaacaccgtgtacgaccccctgcaacccgagctggacagcttcaaggaggagctggacaagtactttaagaaccacacaagccccgacgtggacctgggggacatctccggcatcaacgctagcgtggtgaacattcagaaggaaattgacagactgaatgaggtggccaagaacctgaacgagagcctgatcgacctgcaagagctgggcaagtacgagcagtacatcaagtggccctggtacatctggctgggcttcatcgccggcctgatcgccatcgtgatggtgaccatcatgctgtgctgcatgacaagctgctgcagctgtctgaagggctgctgctcctgcggcagctgctgcaagttcgacgaggacgacagcgagcccgtgctgaagggcgtgaagctgcactacacctga

SEQ ID NO: 39 - protein, 1268 aa, synthetic construct
MFVFLVLLPLVSSQCVNLITRTQSYTNSFTRGVYYPDKVFRSSVLHSTQDLFLPFFSNVTWFHAISGTNGTKRFDNPVLPFNDGVYFASTEKSNIIRGWIFGTTLDSKTQSLLIVNNATNVVIKVCEFQFCNDPFLDVYYHKNNKSWMESEFRVYSSANNCTFEYVSQPFLMDLEGKQGNFKNLREFVFKNIDGYFKIYSKHTPINLGRDLPQGFSALEPLVDLPIGINITRFQTLLALHRSYLTPGDSSSGWTAGAAAYYVGYLQPRTFLLKYNENGTITDAVDCALDPLSETKCTLKSFTVEKGIYQTSNFRVQPTESIVRFPNITNLCPFDEVFNATRFASVYAWNRKRISNCVADYSVLYNFAPFFAFKCYGVSPTKLNDLCFTNVYADSFVIRGNEVSQIAPGQTGNIADYNYKLPDDFTGCVIAWNSNKLDSKVGGNYNYRYRLFRKSNLKPFERDISTEIYQAGNKPCNGVAGVNCYFPLQSYGFRPTYGVGHQPYRVVVLSFELLHAPATVCGPKKSTNLVKNKCVNFNFNGLTGTGVLTESNKKFLPFQQFGRDIADTTDAVRDPQTLEILDITPCSFGGVSVITPGTNTSNQVAVLYQGVNCTEVPVAIHADQLTPTWRVYSTGSNVFQTRAGCLIGAEYVNNSYECDIPIGAGICASYQTQTKSHRRARSVASQSIIAYTMSLGAENSVAYSNNSIAIPTNFTISVTTEILPVSMTKTSVDCTMYICGDSTECSNLLLQYGSFCTQLKRALTGIAVEQDKNTQEVFAQVKQIYKTPPIKYFGGFNFSQILPDPSKPSKRSFIEDLLFNKVTLADAGFIKQYGDCLGDIAARDLICAQKFNGLTVLPPLLTDEMIAQYTSALLAGTITSGWTFGAGAALQIPFAMQMAYRFNGIGVTQNVLYENQKLIANQFNSAIGKIQDSLSSTASALGKLQDVVNHNAQALNTLVKQLSSKFGAISSVLNDILSRLDPPEAEVQIDRLITGRLQSLQTYVTQQLIRAAEIRASANLAATKMSECVLGQSKRVDFCGKGYHLMSFPQSAPHGVVFLHVTYVPAQEKNFTTAPAICHDGKAHFPREGVFVSNGTHWFVTQRNFYEPQIITTDNTFVSGNCDVVIGIVNNTVYDPLQPELDSFKEELDKYFKNHTSPDVDLGDISGINASVVNIQKEIDRLNEVAKNLNESLIDLQELGKYEQYIKWPWYIWLGFIAGLIAIVMVTIMLCCMTSCCSCLKGCCSCGSCCKFDEDDSEPVLKGVKLHYT

SEQ ID NO: 40 - protein, 1273 aa, synthetic construct; identical to SEQ ID NO: 25

SEQ ID NO: 41 - DNA, 3822 bp, synthetic construct
  source 1..3822: mol_type = other DNA
atgttcgtgttcctggtgctgctgcccctggtgagcagccagtgcgtgaacctgaccaccagaacccagctgccccccgcctacaccaacagcttcaccagaggcgtgtactaccccgacaaggtgttcagaagcagcgtgctgcacagcacccaggacctgttcctgcccttcttcagcaacgtgacctggttccacgccatccacgtgagcggcaccaacggcaccaagagattcgacaaccccgtgctgcccttcaacgacggcgtgtacttcgccagcaccgagaagagcaacatcatcagaggctggatcttcggcaccaccctggacagcaagacccagagcctgctgatcgtgaacaacgccaccaacgtggtgatcaaggtgtgcgagttccagttctgcaacgaccccttcctgggcgtgtactaccacaagaacaacaagagctggatggagagcgagttcagagtgtacagcagcgccaacaactgcaccttcgagtacgtgagccagcccttcctgatggacctggagggcaagcagggcaacttcaagaacctgagagagttcgtgttcaagaacatcgacggctacttcaagatctacagcaagcacacccccatcaacctggtgagagacctgccccagggcttcagcgccctggagcccctggtggacctgcccatcggcatcaacatcaccagattccagaccctgctggccctgcacagaagctacctgacccccggcgacagcagcagcggctggaccgccggcgccgccgcctactacgtgggctacctgcagcccagaaccttcctgctgaagtacaacgagaacggcaccatcaccgacgccgtggactgcgccctggaccccctgagcgagaccaagtgcaccctgaagagcttcaccgtggagaagggcatctaccagaccagcaacttcagagtgcagcccaccgagagcatcgtgagattccccaacatcaccaacctgtgccccttcggcgaggtgttcaacgccaccagattcgccagcgtgtacgcctggaacagaaagagaatcagcaactgcgtggccgactacagcgtgctgtacaacagcgccagcttcagcaccttcaagtgctacggcgtgagccccaccaagctgaacgacctgtgcttcaccaacgtgtacgccgacagcttcgtgatcagaggcgacgaggtgagacagatcgcccccggccagaccggcaagatcgccgactacaactacaagctgcccgacgacttcaccggctgcgtgatcgcctggaacagcaacaacctggacagcaaggtgggcggcaactacaactacctgtacagactgttcagaaagagcaacctgaagcccttcgagagagacatcagcaccgagatctaccaggccggcagcaccccctgcaacggcgtggagggcttcaactgctacttccccctgcagagctacggcttccagcccaccaacggcgtgggctaccagccctacagagtggtggtgctgagcttcgagctgctgcacgcccccgccaccgtgtgcggccccaagaagagcaccaacctggtgaagaacaagtgcgtgaacttcaacttcaacggcctgaccggcaccggcgtgctgaccgagagcaacaagaagttcctgcccttccagcagttcggcagagacatcgccgacaccaccgacgccgtgagagacccccagaccctggagatcctggacatcaccccctgcagcttcggcggcgtgagcgtgatcacccccggcaccaacaccagcaaccaggtggccgtgctgtaccaggacgtgaactgcaccgaggtgcccgtggccatccacgccgaccagctgacccccacctggagagtgtacagcaccggcagcaacgtgttccagaccagagccggctgcctgatcggcgccgagcacgtgaacaacagctacgagtgcgacatccccatcggcgccggcatctgcgccagctaccagacccagaccaacagccccagaagagccagaagcgtggccagccagagcatcatcgcctacaccatgagcctgggcgccgagaacagcgtggcctacagcaacaacagcatcgccatccccaccaacttcaccatcagcgtgaccaccgagatcctgcccgtgagcatgaccaagaccagcgtggactgcaccatgtacatctgcggcgacagcaccgagtgcagcaacctgctgctgcagtacggcagcttctgcacccagctgaacagagccctgaccggcatcgccgtggagcaggacaagaacacccaggaggtgttcgcccaggtgaagcagatctacaagaccccccccatcaaggacttcggcggcttcaacttcagccagatcctgcccgaccccagcaagcccagcaagagaagcttcatcgaggacctgctgttcaacaaggtgaccctggccgacgccggcttcatcaagcagtacggcgactgcctgggcgacatcgccgccagagacctgatctgcgcccagaagttcaacggcctgaccgtgctgccccccctgctgaccgacgagatgatcgcccagtacaccagcgccctgctggccggcaccatcaccagcggctggaccttcggcgccggcgccgccctgcagatccccttcgccatgcagatggcctacagattcaacggcatcggcgtgacccagaacgtgctgtacgagaaccagaagctgatcgccaaccagttcaacagcgccatcggcaagatccaggacagcctgagcagcaccgccagcgccctgggcaagctgcaggacgtggtgaaccagaacgcccaggccctgaacaccctggtgaagcagctgagcagcaacttcggcgccatcagcagcgtgctgaacgacatcctgagcagactggacaaggtggaggccgaggtgcagatcgacagactgatcaccggcagactgcagagcctgcagacctacgtgacccagcagctgatcagagccgccgagatcagagccagcgccaacctggccgccaccaagatgagcgagtgcgtgctgggccagagcaagagagtggacttctgcggcaagggctaccacctgatgagcttcccccagagcgccccccacggcgtggtgttcctgcacgtgacctacgtgcccgcccaggagaagaacttcaccaccgcccccgccatctgccacgacggcaaggcccacttccccagagagggcgtgttcgtgagcaacggcacccactggttcgtgacccagagaaacttctacgagccccagatcatcaccaccgacaacaccttcgtgagcggcaactgcgacgtggtgatcggcatcgtgaacaacaccgtgtacgaccccctgcagcccgagctggacagcttcaaggaggagctggacaagtacttcaagaaccacaccagccccgacgtggacctgggcgacatcagcggcatcaacgccagcgtggtgaacatccagaaggagatcgacagactgaacgaggtggccaagaacctgaacgagagcctgatcgacctgcaggagctgggcaagtacgagcagtacatcaagtggccctggtacatctggctgggcttcatcgccggcctgatcgccatcgtgatggtgaccatcatgctgtgctgcatgaccagctgctgcagctgcctgaagggctgctgcagctgcggcagctgctgcaagttcgacgaggacgacagcgagcccgtgctgaagggcgtgaagctgcactacacctag

SEQ ID NO: 42 - DNA, 3822 bp, synthetic construct
  source 1..3822: mol_type = other DNA
atgttcgtgttcctggtgctgctgcccctggtgtcctcccagtgcgtgaacctgaccacccgtacccagctgccccccgcttacaccaactccttcacccgtggtgtgtactaccccgacaaggtgttccgttcctccgtgctgcactccacccaggacctgttcctgcccttcttctccaacgtgacctggttccacgctatccacgtgtccggtaccaacggtaccaagcgtttcgacaaccccgtgctgcccttcaacgacggtgtgtacttcgcttccaccgagaagtccaacatcatccgtggttggatcttcggtaccaccctggactccaagacccagtccctgctgatcgtgaacaacgctaccaacgtggtgatcaaggtgtgcgagttccagttctgcaacgaccccttcctgggtgtgtactaccacaagaacaacaagtcctggatggagtccgagttccgtgtgtactcctccgctaacaactgcaccttcgagtacgtgtcccagcccttcctgatggacctggagggtaagcagggtaacttcaagaacctgcgtgagttcgtgttcaagaacatcgacggttacttcaagatctactccaagcacacccccatcaacctggtgcgtgacctgccccagggtttctccgctctggagcccctggtggacctgcccatcggtatcaacatcacccgtttccagaccctgctggctctgcaccgttcctacctgacccccggtgactcctcctccggttggaccgctggtgctgctgcttactacgtgggttacctgcagccccgtaccttcctgctgaagtacaacgagaacggtaccatcaccgacgctgtggactgcgctctggaccccctgtccgagaccaagtgcaccctgaagtccttcaccgtggagaagggtatctaccagacctccaacttccgtgtgcagcccaccgagtccatcgtgcgtttccccaacatcaccaacctgtgccccttcggtgaggtgttcaacgctacccgtttcgcttccgtgtacgcttggaaccgtaagcgtatctccaactgcgtggctgactactccgtgctgtacaactccgcttccttctccaccttcaagtgctacggtgtgtcccccaccaagctgaacgacctgtgcttcaccaacgtgtacgctgactccttcgtgatccgtggtgacgaggtgcgtcagatcgctcccggtcagaccggtaagatcgctgactacaactacaagctgcccgacgacttcaccggttgcgtgatcgcttggaactccaacaacctggactccaaggtgggtggtaactacaactacctgtaccgtctgttccgtaagtccaacctgaagcccttcgagcgtgacatctccaccgagatctaccaggctggttccaccccctgcaacggtgtggagggtttcaactgctacttccccctgcagtcctacggtttccagcccaccaacggtgtgggttaccagccctaccgtgtggtggtgctgtccttcgagctgctgcacgctcccgctaccgtgtgcggtcccaagaagtccaccaacctggtgaagaacaagtgcgtgaacttcaacttcaacggtctgaccggtaccggtgtgctgaccgagtccaacaagaagttcctgcccttccagcagttcggtcgtgacatcgctgacaccaccgacgctgtgcgtgacccccagaccctggagatcctggacatcaccccctgctccttcggtggtgtgtccgtgatcacccccggtaccaacacctccaaccaggtggctgtgctgtaccaggacgtgaactgcaccgaggtgcccgtggctatccacgctgaccagctgacccccacctggcgtgtgtactccaccggttccaacgtgttccagacccgtgctggttgcctgatcggtgctgagcacgtgaacaactcctacgagtgcgacatccccatcggtgctggtatctgcgcttcctaccagacccagaccaactccccccgtcgtgctcgttccgtggcttcccagtccatcatcgcttacaccatgtccctgggtgctgagaactccgtggcttactccaacaactccatcgctatccccaccaacttcaccatctccgtgaccaccgagatcctgcccgtgtccatgaccaagacctccgtggactgcaccatgtacatctgcggtgactccaccgagtgctccaacctgctgctgcagtacggttccttctgcacccagctgaaccgtgctctgaccggtatcgctgtggagcaggacaagaacacccaggaggtgttcgctcaggtgaagcagatctacaagaccccccccatcaaggacttcggtggtttcaacttctcccagatcctgcccgacccctccaagccctccaagcgttccttcatcgaggacctgctgttcaacaaggtgaccctggctgacgctggtttcatcaagcagtacggtgactgcctgggtgacatcgctgctcgtgacctgatctgcgctcagaagttcaacggtctgaccgtgctgccccccctgctgaccgacgagatgatcgctcagtacacctccgctctgctggctggtaccatcacctccggttggaccttcggtgctggtgctgctctgcagatccccttcgctatgcagatggcttaccgtttcaacggtatcggtgtgacccagaacgtgctgtacgagaaccagaagctgatcgctaaccagttcaactccgctatcggtaagatccaggactccctgtcctccaccgcttccgctctgggtaagctgcaggacgtggtgaaccagaacgctcaggctctgaacaccctggtgaagcagctgtcctccaacttcggtgctatctcctccgtgctgaacgacatcctgtcccgtctggacaaggtggaggctgaggtgcagatcgaccgtctgatcaccggtcgtctgcagtccctgcagacctacgtgacccagcagctgatccgtgctgctgagatccgtgcttccgctaacctggctgctaccaagatgtccgagtgcgtgctgggtcagtccaagcgtgtggacttctgcggtaagggttaccacctgatgtccttcccccagtccgctccccacggtgtggtgttcctgcacgtgacctacgtgcccgctcaggagaagaacttcaccaccgctcccgctatctgccacgacggtaaggctcacttcccccgtgagggtgtgttcgtgtccaacggtacccactggttcgtgacccagcgtaacttctacgagccccagatcatcaccaccgacaacaccttcgtgtccggtaactgcgacgtggtgatcggtatcgtgaacaacaccgtgtacgaccccctgcagcccgagctggactccttcaaggaggagctggacaagtacttcaagaaccacacctcccccgacgtggacctgggtgacatctccggtatcaacgcttccgtggtgaacatccagaaggagatcgaccgtctgaacgaggtggctaagaacctgaacgagtccctgatcgacctgcaggagctgggtaagtacgagcagtacatcaagtggccctggtacatctggctgggtttcatcgctggtctgatcgctatcgtgatggtgaccatcatgctgtgctgcatgacctcctgctgctcctgcctgaagggttgctgctcctgcggttcctgctgcaagttcgacgaggacgactccgagcccgtgctgaagggtgtgaagctgcactacacctag

SEQ ID NO: 43 - protein, 1213 aa, synthetic construct
MFVFLVLLPLVSSQCVNLTTRTQLPPAYTNSFTRGVYYPDKVFRSSVLHSTQDLFLPFFSNVTWFHAIHVSGTNGTKRFDNPVLPFNDGVYFASTEKSNIIRGWIFGTTLDSKTQSLLIVNNATNVVIKVCEFQFCNDPFLGVYYHKNNKSWMESEFRVYSSANNCTFEYVSQPFLMDLEGKQGNFKNLREFVFKNIDGYFKIYSKHTPINLVRDLPQGFSALEPLVDLPIGINITRFQTLLALHRSYLTPGDSSSGWTAGAAAYYVGYLQPRTFLLKYNENGTITDAVDCALDPLSETKCTLKSFTVEKGIYQTSNFRVQPTESIVRFPNITNLCPFGEVFNATRFASVYAWNRKRISNCVADYSVLYNSASFSTFKCYGVSPTKLNDLCFTNVYADSFVIRGDEVRQIAPGQTGKIADYNYKLPDDFTGCVIAWNSNNLDSKVGGNYNYLYRLFRKSNLKPFERDISTEIYQAGSTPCNGVEGFNCYFPLQSYGFQPTNGVGYQPYRVVVLSFELLHAPATVCGPKKSTNLVKNKCVNFNFNGLTGTGVLTESNKKFLPFQQFGRDIADTTDAVRDPQTLEILDITPCSFGGVSVITPGTNTSNQVAVLYQDVNCTEVPVAIHADQLTPTWRVYSTGSNVFQTRAGCLIGAEHVNNSYECDIPIGAGICASYQTQTNSPRRARSVASQSIIAYTMSLGAENSVAYSNNSIAIPTNFTISVTTEILPVSMTKTSVDCTMYICGDSTECSNLLLQYGSFCTQLNRALTGIAVEQDKNTQEVFAQVKQIYKTPPIKDFGGFNFSQILPDPSKPSKRSFIEDLLFNKVTLADAGFIKQYGDCLGDIAARDLICAQKFNGLTVLPPLLTDEMIAQYTSALLAGTITSGWTFGAGAALQIPFAMQMAYRFNGIGVTQNVLYENQKLIANQFNSAIGKIQDSLSSTASALGKLQDVVNQNAQALNTLVKQLSSNFGAISSVLNDILSRLDKVEAEVQIDRLITGRLQSLQTYVTQQLIRAAEIRASANLAATKMSECVLGQSKRVDFCGKGYHLMSFPQSAPHGVVFLHVTYVPAQEKNFTTAPAICHDGKAHFPREGVFVSNGTHWFVTQRNFYEPQIITTDNTFVSGNCDVVIGIVNNTVYDPLQPELDSFKEELDKYFKNHTSPDVDLGDISGINASVVNIQKEIDRLNEVAKNLNESLIDLQELGKYEQYIKWP

SEQ ID NO: 44 - DNA, 3642 bp, synthetic construct
  source 1..3642: mol_type = other DNA
atgttcgtgttcctggtgctgctgcccctggtgagcagccagtgcgtgaacctgaccaccagaacccagctgccccccgcctacaccaacagcttcaccagaggcgtgtactaccccgacaaggtgttcagaagcagcgtgctgcacagcacccaggacctgttcctgcccttcttcagcaacgtgacctggttccacgccatccacgtgagcggcaccaacggcaccaagagattcgacaaccccgtgctgcccttcaacgacggcgtgtacttcgccagcaccgagaagagcaacatcatcagaggctggatcttcggcaccaccctggacagcaagacccagagcctgctgatcgtgaacaacgccaccaacgtggtgatcaaggtgtgcgagttccagttctgcaacgaccccttcctgggcgtgtactaccacaagaacaacaagagctggatggagagcgagttcagagtgtacagcagcgccaacaactgcaccttcgagtacgtgagccagcccttcctgatggacctggagggcaagcagggcaacttcaagaacctgagagagttcgtgttcaagaacatcgacggctacttcaagatctacagcaagcacacccccatcaacctggtgagagacctgccccagggcttcagcgccctggagcccctggtggacctgcccatcggcatcaacatcaccagattccagaccctgctggccctgcacagaagctacctgacccccggcgacagcagcagcggctggaccgccggcgccgccgcctactacgtgggctacctgcagcccagaaccttcctgctgaagtacaacgagaacggcaccatcaccgacgccgtggactgcgccctggaccccctgagcgagaccaagtgcaccctgaagagcttcaccgtggagaagggcatctaccagaccagcaacttcagagtgcagcccaccgagagcatcgtgagattccccaacatcaccaacctgtgccccttcggcgaggtgttcaacgccaccagattcgccagcgtgtacgcctggaacagaaagagaatcagcaactgcgtggccgactacagcgtgctgtacaacagcgccagcttcagcaccttcaagtgctacggcgtgagccccaccaagctgaacgacctgtgcttcaccaacgtgtacgccgacagcttcgtgatcagaggcgacgaggtgagacagatcgcccccggccagaccggcaagatcgccgactacaactacaagctgcccgacgacttcaccggctgcgtgatcgcctggaacagcaacaacctggacagcaaggtgggcggcaactacaactacctgtacagactgttcagaaagagcaacctgaagcccttcgagagagacatcagcaccgagatctaccaggccggcagcaccccctgcaacggcgtggagggcttcaactgctacttccccctgcagagctacggcttccagcccaccaacggcgtgggctaccagccctacagagtggtggtgctgagcttcgagctgctgcacgcccccgccaccgtgtgcggccccaagaagagcaccaacctggtgaagaacaagtgcgtgaacttcaacttcaacggcctgaccggcaccggcgtgctgaccgagagcaacaagaagttcctgcccttccagcagttcggcagagacatcgccgacaccaccgacgccgtgagagacccccagaccctggagatcctggacatcaccccctgcagcttcggcggcgtgagcgtgatcacccccggcaccaacaccagcaaccaggtggccgtgctgtaccaggacgtgaactgcaccgaggtgcccgtggccatccacgccgaccagctgacccccacctggagagtgtacagcaccggcagcaacgtgttccagaccagagccggctgcctgatcggcgccgagcacgtgaacaacagctacgagtgcgacatccccatcggcgccggcatctgcgccagctaccagacccagaccaacagccccagaagagccagaagcgtggccagccagagcatcatcgcctacaccatgagcctgggcgccgagaacagcgtggcctacagcaacaacagcatcgccatccccaccaacttcaccatcagcgtgaccaccgagatcctgcccgtgagcatgaccaagaccagcgtggactgcaccatgtacatctgcggcgacagcaccgagtgcagcaacctgctgctgcagtacggcagcttctgcacccagctgaacagagccctgaccggcatcgccgtggagcaggacaagaacacccaggaggtgttcgcccaggtgaagcagatctacaagaccccccccatcaaggacttcggcggcttcaacttcagccagatcctgcccgaccccagcaagcccagcaagagaagcttcatcgaggacctgctgttcaacaaggtgaccctggccgacgccggcttcatcaagcagtacggcgactgcctgggcgacatcgccgccagagacctgatctgcgcccagaagttcaacggcctgaccgtgctgccccccctgctgaccgacgagatgatcgcccagtacaccagcgccctgctggccggcaccatcaccagcggctggaccttcggcgccggcgccgccctgcagatccccttcgccatgcagatggcctacagattcaacggcatcggcgtgacccagaacgtgctgtacgagaaccagaagctgatcgccaaccagttcaacagcgccatcggcaagatccaggacagcctgagcagcaccgccagcgccctgggcaagctgcaggacgtggtgaaccagaacgcccaggccctgaacaccctggtgaagcagctgagcagcaacttcggcgccatcagcagcgtgctgaacgacatcctgagcagactggacaaggtggaggccgaggtgcagatcgacagactgatcaccggcagactgcagagcctgcagacctacgtgacccagcagctgatcagagccgccgagatcagagccagcgccaacctggccgccaccaagatgagcgagtgcgtgctgggccagagcaagagagtggacttctgcggcaagggctaccacctgatgagcttcccccagagcgccccccacggcgtggtgttcctgcacgtgacctacgtgcccgcccaggagaagaacttcaccaccgcccccgccatctgccacgacggcaaggcccacttccccagagagggcgtgttcgtgagcaacggcacccactggttcgtgacccagagaaacttctacgagccccagatcatcaccaccgacaacaccttcgtgagcggcaactgcgacgtggtgatcggcatcgtgaacaacaccgtgtacgaccccctgcagcccgagctggacagcttcaaggaggagctggacaagtacttcaagaaccacaccagccccgacgtggacctgggcgacatcagcggcatcaacgccagcgtggtgaacatccagaaggagatcgacagactgaacgaggtggccaagaacctgaacgagagcctgatcgacctgcaggagctgggcaagtacgagcagtacatcaagtggccctag

SEQ ID NO: 45 - DNA, 3642 bp, synthetic construct
  source 1..3642: mol_type = other DNA
atgttcgtgttcctggtgctgctgcccctggtgtcctcccagtgcgtgaacctgaccacccgtacccagctgccccccgcttacaccaactccttcacccgtggtgtgtactaccccgacaaggtgttccgttcctccgtgctgcactccacccaggacctgttcctgcccttcttctccaacgtgacctggttccacgctatccacgtgtccggtaccaacggtaccaagcgtttcgacaaccccgtgctgcccttcaacgacggtgtgtacttcgcttccaccgagaagtccaacatcatccgtggttggatcttcggtaccaccctggactccaagacccagtccctgctgatcgtgaacaacgctaccaacgtggtgatcaaggtgtgcgagttccagttctgcaacgaccccttcctgggtgtgtactaccacaagaacaacaagtcctggatggagtccgagttccgtgtgtactcctccgctaacaactgcaccttcgagtacgtgtcccagcccttcctgatggacctggagggtaagcagggtaacttcaagaacctgcgtgagttcgtgttcaagaacatcgacggttacttcaagatctactccaagcacacccccatcaacctggtgcgtgacctgccccagggtttctccgctctggagcccctggtggacctgcccatcggtatcaacatcacccgtttccagaccctgctggctctgcaccgttcctacctgacccccggtgactcctcctccggttggaccgctggtgctgctgcttactacgtgggttacctgcagccccgtaccttcctgctgaagtacaacgagaacggtaccatcaccgacgctgtggactgcgctctggaccccctgtccgagaccaagtgcaccctgaagtccttcaccgtggagaagggtatctaccagacctccaacttccgtgtgcagcccaccgagtccatcgtgcgtttccccaacatcaccaacctgtgccccttcggtgaggtgttcaacgctacccgtttcgcttccgtgtacgcttggaaccgtaagcgtatctccaactgcgtggctgactactccgtgctgtacaactccgcttccttctccaccttcaagtgctacggtgtgtcccccaccaagctgaacgacctgtgcttcaccaacgtgtacgctgactccttcgtgatccgtggtgacgaggtgcgtcagatcgctcccggtcagaccggtaagatcgctgactacaactacaagctgcccgacgacttcaccggttgcgtgatcgcttggaactccaacaacctggactccaaggtgggtggtaactacaactacctgtaccgtctgttccgtaagtccaacctgaagcccttcgagcgtgacatctccaccgagatctaccaggctggttccaccccctgcaacggtgtggagggtttcaactgctacttccccctgcagtcctacggtttccagcccaccaacggtgtgggttaccagccctaccgtgtggtggtgctgtccttcgagctgctgcacgctcccgctaccgtgtgcggtcccaagaagtccaccaacctggtgaagaacaagtgcgtgaacttcaacttcaacggtctgaccggtaccggtgtgctgaccgagtccaacaagaagttcctgcccttccagcagttcggtcgtgacatcgctgacaccaccgacgctgtgcgtgacccccagaccctggagatcctggacatcaccccctgctccttcggtggtgtgtccgtgatcacccccggtaccaacacctccaaccaggtggctgtgctgtaccaggacgtgaactgcaccgaggtgcccgtggctatccacgctgaccagctgacccccacctggcgtgtgtactccaccggttccaacgtgttccagacccgtgctggttgcctgatcggtgctgagcacgtgaacaactcctacgagtgcgacatccccatcggtgctggtatctgcgcttcctaccagacccagaccaactccccccgtcgtgctcgttccgtggcttcccagtccatcatcgcttacaccatgtccctgggtgctgagaactccgtggcttactccaacaactccatcgctatccccaccaacttcaccatctccgtgaccaccgagatcctgcccgtgtccatgaccaagacctccgtggactgcaccatgtacatctgcggtgactccaccgagtgctccaacctgctgctgcagtacggttccttctgcacccagctgaaccgtgctctgaccggtatcgctgtggagcaggacaagaacacccaggaggtgttcgctcaggtgaagcagatctacaagaccccccccatcaaggacttcggtggtttcaacttctcccagatcctgcccgacccctccaagccctccaagcgttccttcatcgaggacctgctgttcaacaaggtgaccctggctgacgctggtttcatcaagcagtacggtgactgcctgggtgacatcgctgctcgtgacctgatctgcgctcagaagttcaacggtctgaccgtgctgccccccctgctgaccgacgagatgatcgctcagtacacctccgctctgctggctggtaccatcacctccggttggaccttcggtgctggtgctgctctgcagatccccttcgctatgcagatggcttaccgtttcaacggtatcggtgtgacccagaacgtgctgtacgagaaccagaagctgatcgctaaccagttcaactccgctatcggtaagatccaggactccctgtcctccaccgcttccgctctgggtaagctgcaggacgtggtgaaccagaacgctcaggctctgaacaccctggtgaagcagctgtcctccaacttcggtgctatctcctccgtgctgaacgacatcctgtcccgtctggacaaggtggaggctgaggtgcagatcgaccgtctgatcaccggtcgtctgcagtccctgcagacctacgtgacccagcagctgatccgtgctgctgagatccgtgcttccgctaacctggctgctaccaagatgtccgagtgcgtgctgggtcagtccaagcgtgtggacttctgcggtaagggttaccacctgatgtccttcccccagtccgctccccacggtgtggtgttcctgcacgtgacctacgtgcccgctcaggagaagaacttcaccaccgctcccgctatctgccacgacggtaaggctcacttcccccgtgagggtgtgttcgtgtccaacggtacccactggttcgtgacccagcgtaacttctacgagccccagatcatcaccaccgacaacaccttcgtgtccggtaactgcgacgtggtgatcggtatcgtgaacaacaccgtgtacgaccccctgcagcccgagctggactccttcaaggaggagctggacaagtacttcaagaaccacacctcccccgacgtggacctgggtgacatctccggtatcaacgcttccgtggtgaacatccagaaggagatcgaccgtctgaacgaggtggctaagaacctgaacgagtccctgatcgacctgcaggagctgggtaagtacgagcagtacatcaagtggccctag

SEQ ID NO: 46 - protein, 1270 aa, synthetic construct
MFVFLVLLPLVSSQCVNLTTRTQLPPAYTNSFTRGVYYPDKVFRSSVLHSTQDLFLPFFSNVTWFHAIHVSGTNGTKRFANPVLPFNDGVYFASTEKSNIIRGWIFGTTLDSKTQSLLIVNNATNVVIKVCEFQFCNDPFLGVYYHKNNKSWMESEFRVYSSANNCTFEYVSQPFLMDLEGKQGNFKNLREFVFKNIDGYFKIYSKHTPINLVRGLPQGFSALEPLVDLPIGINITRFQTLHRSYLTPGDSSSGWTAGAAAYYVGYLQPRTFLLKYNENGTITDAVDCALDPLSETKCTLKSFTVEKGIYQTSNFRVQPTESIVRFPNITNLCPFGEVFNATRFASVYAWNRKRISNCVADYSVLYNSASFSTFKCYGVSPTKLNDLCFTNVYADSFVIRGDEVRQIAPGQTGNIADYNYKLPDDFTGCVIAWNSNNLDSKVGGNYNYLYRLFRKSNLKPFERDISTEIYQAGSTPCNGVKGFNCYFPLQSYGFQPTYGVGYQPYRVVVLSFELLHAPATVCGPKKSTNLVKNKCVNFNFNGLTGTGVLTESNKKFLPFQQFGRDIADTTDAVRDPQTLEILDITPCSFGGVSVITPGTNTSNQVAVLYQGVNCTEVPVAIHADQLTPTWRVYSTGSNVFQTRAGCLIGAEHVNNSYECDIPIGAGICASYQTQTNSPRRARSVASQSIIAYTMSLGVENSVAYSNNSIAIPTNFTISVTTEILPVSMTKTSVDCTMYICGDSTECSNLLLQYGSFCTQLNRALTGIAVEQDKNTQEVFAQVKQIYKTPPIKDFGGFNFSQILPDPSKPSKRSFIEDLLFNKVTLADAGFIKQYGDCLGDIAARDLICAQKFNGLTVLPPLLTDEMIAQYTSALLAGTITSGWTFGAGAALQIPFAMQMAYRFNGIGVTQNVLYENQKLIANQFNSAIGKIQDSLSSTASALGKLQDVVNQNAQALNTLVKQLSSNFGAISSVLNDILSRLDKVEAEVQIDRLITGRLQSLQTYVTQQLIRAAEIRASANLAATKMSECVLGQSKRVDFCGKGYHLMSFPQSAPHGVVFLHVTYVPAQEKNFTTAPAICHDGKAHFPREGVFVSNGTHWFVTQRNFYEPQIITTDNTFVSGNCDVVIGIVNNTVYDPLQPELDSFKEELDKYFKNHTSPDVDLGDISGINASVVNIQKEIDRLNEVAKNLNESLIDLQELGKYEQYIKWPWYIWLGFIAGLIAIVMVTIMLCCMTSCCSCLKGCCSCGSCCKFDEDDSEPVLKGVKLHYT

SEQ ID NO: 47 - DNA, 3813 bp, synthetic construct
  source 1..3813: mol_type = other DNA
atgttcgtgttcctggtgctgctgcccctggtgagcagccagtgcgtgaacctgaccaccagaacccagctgccccccgcctacaccaacagcttcaccagaggcgtgtactaccccgacaaggtgttcagaagcagcgtgctgcacagcacccaggacctgttcctgcccttcttcagcaacgtgacctggttccacgccatccacgtgagcggcaccaacggcaccaagagattcgccaaccccgtgctgcccttcaacgacggcgtgtacttcgccagcaccgagaagagcaacatcatcagaggctggatcttcggcaccaccctggacagcaagacccagagcctgctgatcgtgaacaacgccaccaacgtggtgatcaaggtgtgcgagttccagttctgcaacgaccccttcctgggcgtgtactaccacaagaacaacaagagctggatggagagcgagttcagagtgtacagcagcgccaacaactgcaccttcgagtacgtgagccagcccttcctgatggacctggagggcaagcagggcaacttcaagaacctgagagagttcgtgttcaagaacatcgacggctacttcaagatctacagcaagcacacccccatcaacctggtgagaggcctgccccagggcttcagcgccctggagcccctggtggacctgcccatcggcatcaacatcaccagattccagaccctgcacagaagctacctgacccccggcgacagcagcagcggctggaccgccggcgccgccgcctactacgtgggctacctgcagcccagaaccttcctgctgaagtacaacgagaacggcaccatcaccgacgccgtggactgcgccctggaccccctgagcgagaccaagtgcaccctgaagagcttcaccgtggagaagggcatctaccagaccagcaacttcagagtgcagcccaccgagagcatcgtgagattccccaacatcaccaacctgtgccccttcggcgaggtgttcaacgccaccagattcgccagcgtgtacgcctggaacagaaagagaatcagcaactgcgtggccgactacagcgtgctgtacaacagcgccagcttcagcaccttcaagtgctacggcgtgagccccaccaagctgaacgacctgtgcttcaccaacgtgtacgccgacagcttcgtgatcagaggcgacgaggtgagacagatcgcccccggccagaccggcaacatcgccgactacaactacaagctgcccgacgacttcaccggctgcgtgatcgcctggaacagcaacaacctggacagcaaggtgggcggcaactacaactacctgtacagactgttcagaaagagcaacctgaagcccttcgagagagacatcagcaccgagatctaccaggccggcagcaccccctgcaacggcgtgaagggcttcaactgctacttccccctgcagagctacggcttccagcccacctacggcgtgggctaccagccctacagagtggtggtgctgagcttcgagctgctgcacgcccccgccaccgtgtgcggccccaagaagagcaccaacctggtgaagaacaagtgcgtgaacttcaacttcaacggcctgaccggcaccggcgtgctgaccgagagcaacaagaagttcctgcccttccagcagttcggcagagacatcgccgacaccaccgacgccgtgagagacccccagaccctggagatcctggacatcaccccctgcagcttcggcggcgtgagcgtgatcacccccggcaccaacaccagcaaccaggtggccgtgctgtaccagggcgtgaactgcaccgaggtgcccgtggccatccacgccgaccagctgacccccacctggagagtgtacagcaccggcagcaacgtgttccagaccagagccggctgcctgatcggcgccgagcacgtgaacaacagctacgagtgcgacatccccatcggcgccggcatctgcgccagctaccagacccagaccaacagccccagaagagccagaagcgtggccagccagagcatcatcgcctacaccatgagcctgggcgtggagaacagcgtggcctacagcaacaacagcatcgccatccccaccaacttcaccatcagcgtgaccaccgagatcctgcccgtgagcatgaccaagaccagcgtggactgcaccatgtacatctgcggcgacagcaccgagtgcagcaacctgctgctgcagtacggcagcttctgcacccagctgaacagagccctgaccggcatcgccgtggagcaggacaagaacacccaggaggtgttcgcccaggtgaagcagatctacaagaccccccccatcaaggacttcggcggcttcaacttcagccagatcctgcccgaccccagcaagcccagcaagagaagcttcatcgaggacctgctgttcaacaaggtgaccctggccgacgccggcttcatcaagcagtacggcgactgcctgggcgacatcgccgccagagacctgatctgcgcccagaagttcaacggcctgaccgtgctgccccccctgctgaccgacgagatgatcgcccagtacaccagcgccctgctggccggcaccatcaccagcggctggaccttcggcgccggcgccgccctgcagatccccttcgccatgcagatggcctacagattcaacggcatcggcgtgacccagaacgtgctgtacgagaaccagaagctgatcgccaaccagttcaacagcgccatcggcaagatccaggacagcctgagcagcaccgccagcgccctgggcaagctgcaggacgtggtgaaccagaacgcccaggccctgaacaccctggtgaagcagctgagcagcaacttcggcgccatcagcagcgtgctgaacgacatcctgagcagactggacaaggtggaggccgaggtgcagatcgacagactgatcaccggcagactgcagagcctgcagacctacgtgacccagcagctgatcagagccgccgagatcagagccagcgccaacctggccgccaccaagatgagcgagtgcgtgctgggccagagcaagagagtggacttctgcggcaagggctaccacctgatgagcttcccccagagcgccccccacggcgtggtgttcctgcacgtgacctacgtgcccgcccaggagaagaacttcaccaccgcccccgccatctgccacgacggcaaggcccacttccccagagagggcgtgttcgtgagcaacggcacccactggttcgtgacccagagaaacttctacgagccccagatcatcaccaccgacaacaccttcgtgagcggcaactgcgacgtggtgatcggcatcgtgaacaacaccgtgtacgaccccctgcagcccgagctggacagcttcaaggaggagctggacaagtacttcaagaaccacaccagccccgacgtggacctgggcgacatcagcggcatcaacgccagcgtggtgaacatccagaaggagatcgacagactgaacgaggtggccaagaacctgaacgagagcctgatcgacctgcaggagctgggcaagtacgagcagtacatcaagtggccctggtacatctggctgggcttcatcgccggcctgatcgccatcgtgatggtgaccatcatgctgtgctgcatgaccagctgctgcagctgcctgaagggctgctgcagctgcggcagctgctgcaagttcgacgaggacgacagcgagcccgtgctgaagggcgtgaagctgcactacacctag

SEQ ID NO: 48 - DNA, 3813 bp, synthetic construct
  source 1..3813: mol_type = other DNA
atgttcgtgttcctggtgctgctgcccctggtgtcctcccagtgcgtgaacctgaccacccgtacccagctgccccccgcttacaccaactccttcacccgtggtgtgtactaccccgacaaggtgttccgttcctccgtgctgcactccacccaggacctgttcctgcccttcttctccaacgtgacctggttccacgctatccacgtgtccggtaccaacggtaccaagcgtttcgctaaccccgtgctgcccttcaacgacggtgtgtacttcgcttccaccgagaagtccaacatcatccgtggttggatcttcggtaccaccctggactccaagacccagtccctgctgatcgtgaacaacgctaccaacgtggtgatcaaggtgtgcgagttccagttctgcaacgaccccttcctgggtgtgtactaccacaagaacaacaagtcctggatggagtccgagttccgtgtgtactcctccgctaacaactgcaccttcgagtacgtgtcccagcccttcctgatggacctggagggtaagcagggtaacttcaagaacctgcgtgagttcgtgttcaagaacatcgacggttacttcaagatctactccaagcacacccccatcaacctggtgcgtggtctgccccagggtttctccgctctggagcccctggtggacctgcccatcggtatcaacatcacccgtttccagaccctgcaccgttcctacctgacccccggtgactcctcctccggttggaccgctggtgctgctgcttactacgtgggttacctgcagccccgtaccttcctgctgaagtacaacgagaacggtaccatcaccgacgctgtggactgcgctctggaccccctgtccgagaccaagtgcaccctgaagtccttcaccgtggagaagggtatctaccagacctccaacttccgtgtgcagcccaccgagtccatcgtgcgtttccccaacatcaccaacctgtgccccttcggtgaggtgttcaacgctacccgtttcgcttccgtgtacgcttggaaccgtaagcgtatctccaactgcgtggctgactactccgtgctgtacaactccgcttccttctccaccttcaagtgctacggtgtgtcccccaccaagctgaacgacctgtgcttcaccaacgtgtacgctgactccttcgtgatccgtggtgacgaggtgcgtcagatcgctcccggtcagaccggtaacatcgctgactacaactacaagctgcccgacgacttcaccggttgcgtgatcgcttggaactccaacaacctggactccaaggtgggtggtaactacaactacctgtaccgtctgttccgtaagtccaacctgaagcccttcgagcgtgacatctccaccgagatctaccaggctggttccaccccctgcaacggtgtgaagggtttcaactgctacttccccctgcagtcctacggtttccagcccacctacggtgtgggttaccagccctaccgtgtggtggtgctgtccttcgagctgctgcacgctcccgctaccgtgtgcggtcccaagaagtccaccaacctggtgaagaacaagtgcgtgaacttcaacttcaacggtctgaccggtaccggtgtgctgaccgagtccaacaagaagttcctgcccttccagcagttcggtcgtgacatcgctgacaccaccgacgctgtgcgtgacccccagaccctggagatcctggacatcaccccctgctccttcggtggtgtgtccgtgatcacccccggtaccaacacctccaaccaggtggctgtgctgtaccagggtgtgaactgcaccgaggtgcccgtggctatccacgctgaccagctgacccccacctggcgtgtgtactccaccggttccaacgtgttccagacccgtgctggttgcctgatcggtgctgagcacgtgaacaactcctacgagtgcgacatccccatcggtgctggtatctgcgcttcctaccagacccagaccaactccccccgtcgtgctcgttccgtggcttcccagtccatcatcgcttacaccatgtccctgggtgtggagaactccgtggcttactccaacaactccatcgctatccccaccaacttcaccatctccgtgaccaccgagatcctgcccgtgtccatgaccaagacctccgtggactgcaccatgtacatctgcggtgactccaccgagtgctccaacctgctgctgcagtacggttccttctgcacccagctgaaccgtgctctgaccggtatcgctgtggagcaggacaagaacacccaggaggtgttcgctcaggtgaagcagatctacaagaccccccccatcaaggacttcggtggtttcaacttctcccagatcctgcccgacccctccaagccctccaagcgttccttcatcgaggacctgctgttcaacaaggtgaccctggctgacgctggtttcatcaagcagtacggtgactgcctgggtgacatcgctgctcgtgacctgatctgcgctcagaagttcaacggtctgaccgtgctgccccccctgctgaccgacgagatgatcgctcagtacacctccgctctgctggctggtaccatcacctccggttggaccttcggtgctggtgctgctctgcagatccccttcgctatgcagatggcttaccgtttcaacggtatcggtgtgacccagaacgtgctgtacgagaaccagaagctgatcgctaaccagttcaactccgctatcggtaagatccaggactccctgtcctccaccgcttccgctctgggtaagctgcaggacgtggtgaaccagaacgctcaggctctgaacaccctggtgaagcagctgtcctccaacttcggtgctatctcctccgtgctgaacgacatcctgtcccgtctggacaaggtggaggctgaggtgcagatcgaccgtctgatcaccggtcgtctgcagtccctgcagacctacgtgacccagcagctgatccgtgctgctgagatccgtgcttccgctaacctggctgctaccaagatgtccgagtgcgtgctgggtcagtccaagcgtgtggacttctgcggtaagggttaccacctgatgtccttcccccagtccgctccccacggtgtggtgttcctgcacgtgacctacgtgcccgctcaggagaagaacttcaccaccgctcccgctatctgccacgacggtaaggctcacttcccccgtgagggtgtgttcgtgtccaacggtacccactggttcgtgacccagcgtaacttctacgagccccagatcatcaccaccgacaacaccttcgtgtccggtaactgcgacgtggtgatcggtatcgtgaacaacaccgtgtacgaccccctgcagcccgagctggactccttcaaggaggagctggacaagtacttcaagaaccacacctcccccgacgtggacctgggtgacatctccggtatcaacgcttccgtggtgaacatccagaaggagatcgaccgtctgaacgaggtggctaagaacctgaacgagtccctgatcgacctgcaggagctgggtaagtacgagcagtacatcaagtggccctggtacatctggctgggtttcatcgctggtctgatcgctatcgtgatggtgaccatcatgctgtgctgcatgacctcctgctgctcctgcctgaagggttgctgctcctgcggttcctgctgcaagttcgacgaggacgactccgagcccgtgctgaagggtgtgaagctgcactacacctag

SEQ ID NO: 49 - protein, 1210 aa, synthetic construct
MFVFLVLLPLVSSQCVNLTTRTQLPPAYTNSFTRGVYYPDKVFRSSVLHSTQDLFLPFFSNVTWFHAIHVSGTNGTKRFANPVLPFNDGVYFASTEKSNIIRGWIFGTTLDSKTQSLLIVNNATNVVIKVCEFQFCNDPFLGVYYHKNNKSWMESEFRVYSSANNCTFEYVSQPFLMDLEGKQGNFKNLREFVFKNIDGYFKIYSKHTPINLVRGLPQGFSALEPLVDLPIGINITRFQTLHRSYLTPGDSSSGWTAGAAAYYVGYLQPRTFLLKYNENGTITDAVDCALDPLSETKCTLKSFTVEKGIYQTSNFRVQPTESIVRFPNITNLCPFGEVFNATRFASVYAWNRKRISNCVADYSVLYNSASFSTFKCYGVSPTKLNDLCFTNVYADSFVIRGDEVRQIAPGQTGNIADYNYKLPDDFTGCVIAWNSNNLDSKVGGNYNYLYRLFRKSNLKPFERDISTEIYQAGSTPCNGVKGFNCYFPLQSYGFQPTYGVGYQPYRVVVLSFELLHAPATVCGPKKSTNLVKNKCVNFNFNGLTGTGVLTESNKKFLPFQQFGRDIADTTDAVRDPQTLEILDITPCSFGGVSVITPGTNTSNQVAVLYQGVNCTEVPVAIHADQLTPTWRVYSTGSNVFQTRAGCLIGAEHVNNSYECDIPIGAGICASYQTQTNSPRRARSVASQSIIAYTMSLGVENSVAYSNNSIAIPTNFTISVTTEILPVSMTKTSVDCTMYICGDSTECSNLLLQYGSFCTQLNRALTGIAVEQDKNTQEVFAQVKQIYKTPPIKDFGGFNFSQILPDPSKPSKRSFIEDLLFNKVTLADAGFIKQYGDCLGDIAARDLICAQKFNGLTVLPPLLTDEMIAQYTSALLAGTITSGWTFGAGAALQIPFAMQMAYRFNGIGVTQNVLYENQKLIANQFNSAIGKIQDSLSSTASALGKLQDVVNQNAQALNTLVKQLSSNFGAISSVLNDILSRLDKVEAEVQIDRLITGRLQSLQTYVTQQLIRAAEIRASANLAATKMSECVLGQSKRVDFCGKGYHLMSFPQSAPHGVVFLHVTYVPAQEKNFTTAPAICHDGKAHFPREGVFVSNGTHWFVTQRNFYEPQIITTDNTFVSGNCDVVIGIVNNTVYDPLQPELDSFKEELDKYFKNHTSPDVDLGDISGINASVVNIQKEIDRLNEVAKNLNESLIDLQELGKYEQYIKWP

SEQ ID NO: 50 - DNA, 3633 bp, synthetic construct
  source 1..3633: mol_type = other DNA
atgttcgtgttcctggtgctgctgcccctggtgagcagccagtgcgtgaacctgaccaccagaacccagctgccccccgcctacaccaacagcttcaccagaggcgtgtactaccccgacaaggtgttcagaagcagcgtgctgcacagcacccaggacctgttcctgcccttcttcagcaacgtgacctggttccacgccatccacgtgagcggcaccaacggcaccaagagattcgccaaccccgtgctgcccttcaacgacggcgtgtacttcgccagcaccgagaagagcaacatcatcagaggctggatcttcggcaccaccctggacagcaagacccagagcctgctgatcgtgaacaacgccaccaacgtggtgatcaaggtgtgcgagttccagttctgcaacgaccccttcctgggcgtgtactaccacaagaacaacaagagctggatggagagcgagttcagagtgtacagcagcgccaacaactgcaccttcgagtacgtgagccagcccttcctgatggacctggagggcaagcagggcaacttcaagaacctgagagagttcgtgttcaagaacatcgacggctacttcaagatctacagcaagcacacccccatcaacctggtgagaggcctgccccagggcttcagcgccctggagcccctggtggacctgcccatcggcatcaacatcaccagattccagaccctgcacagaagctacctgacccccggcgacagcagcagcggctggaccgccggcgccgccgcctactacgtgggctacctgcagcccagaaccttcctgctgaagtacaacgagaacggcaccatcaccgacgccgtggactgcgccctggaccccctgagcgagaccaagtgcaccctgaagagcttcaccgtggagaagggcatctaccagaccagcaacttcagagtgcagcccaccgagagcatcgtgagattccccaacatcaccaacctgtgccccttcggcgaggtgttcaacgccaccagattcgccagcgtgtacgcctggaacagaaagagaatcagcaactgcgtggccgactacagcgtgctgtacaacagcgccagcttcagcaccttcaagtgctacggcgtgagccccaccaagctgaacgacctgtgcttcaccaacgtgtacgccgacagcttcgtgatcagaggcgacgaggtgagacagatcgcccccggccagaccggcaacatcgccgactacaactacaagctgcccgacgacttcaccggctgcgtgatcgcctggaacagcaacaacctggacagcaaggtgggcggcaactacaactacctgtacagactgttcagaaagagcaacctgaagcccttcgagagagacatcagcaccgagatctaccaggccggcagcaccccctgcaacggcgtgaagggcttcaactgctacttccccctgcagagctacggcttccagcccacctacggcgtgggctaccagccctacagagtggtggtgctgagcttcgagctgctgcacgcccccgccaccgtgtgcggccccaagaagagcaccaacctggtgaagaacaagtgcgtgaacttcaacttcaacggcctgaccggcaccggcgtgctgaccgagagcaacaagaagttcctgcccttccagcagttcggcagagacatcgccgacaccaccgacgccgtgagagacccccagaccctggagatcctggacatcaccccctgcagcttcggcggcgtgagcgtgatcacccccggcaccaacaccagcaaccaggtggccgtgctgtaccagggcgtgaactgcaccgaggtgcccgtggccatccacgccgaccagctgacccccacctggagagtgtacagcaccggcagcaacgtgttccagaccagagccggctgcctgatcggcgccgagcacgtgaacaacagctacgagtgcgacatccccatcggcgccggcatctgcgccagctaccagacccagaccaacagccccagaagagccagaagcgtggccagccagagcatcatcgcctacaccatgagcctgggcgtggagaacagcgtggcctacagcaacaacagcatcgccatccccaccaacttcaccatcagcgtgaccaccgagatcctgcccgtgagcatgaccaagaccagcgtggactgcaccatgtacatctgcggcgacagcaccgagtgcagcaacctgctgctgcagtacggcagcttctgcacccagctgaacagagccctgaccggcatcgccgtggagcaggacaagaacacccaggaggtgttcgcccaggtgaagcagatctacaagaccccccccatcaaggacttcggcggcttcaacttcagccagatcctgcccgaccccagcaagcccagcaagagaagcttcatcgaggacctgctgttcaacaaggtgaccctggccgacgccggcttcatcaagcagtacggcgactgcctgggcgacatcgccgccagagacctgatctgcgcccagaagttcaacggcctgaccgtgctgccccccctgctgaccgacgagatgatcgcccagtacaccagcgccctgctggccggcaccatcaccagcggctggaccttcggcgccggcgccgccctgcagatccccttcgccatgcagatggcctacagattcaacggcatcggcgtgacccagaacgtgctgtacgagaaccagaagctgatcgccaaccagttcaacagcgccatcggcaagatccaggacagcctgagcagcaccgccagcgccctgggcaagctgcaggacgtggtgaaccagaacgcccaggccctgaacaccctggtgaagcagctgagcagcaacttcggcgccatcagcagcgtgctgaacgacatcctgagcagactggacaaggtggaggccgaggtgcagatcgacagactgatcaccggcagactgcagagcctgcagacctacgtgacccagcagctgatcagagccgccgagatcagagccagcgccaacctggccgccaccaagatgagcgagtgcgtgctgggccagagcaagagagtggacttctgcggcaagggctaccacctgatgagcttcccccagagcgccccccacggcgtggtgttcctgcacgtgacctacgtgcccgcccaggagaagaacttcaccaccgcccccgccatctgccacgacggcaaggcccacttccccagagagggcgtgttcgtgagcaacggcacccactggttcgtgacccagagaaacttctacgagccccagatcatcaccaccgacaacaccttcgtgagcggcaactgcgacgtggtgatcggcatcgtgaacaacaccgtgtacgaccccctgcagcccgagctggacagcttcaaggaggagctggacaagtacttcaagaaccacaccagccccgacgtggacctgggcgacatcagcggcatcaacgccagcgtggtgaacatccagaaggagatcgacagactgaacgaggtggccaagaacctgaacgagagcctgatcgacctgcaggagctgggcaagtacgagcagtacatcaagtggccctag

SEQ ID NO: 51 - DNA, 3633 bp, synthetic construct
  source 1..3633: mol_type = other DNA
atgttcgtgttcctggtgctgctgcccctggtgtcctcccagtgcgtgaacctgaccacccgtacccagctgccccccgcttacaccaactccttcacccgtggtgtgtactaccccgacaaggtgttccgttcctccgtgctgcactccacccaggacctgttcctgcccttcttctccaacgtgacctggttccacgctatccacgtgtccggtaccaacggtaccaagcgtttcgctaaccccgtgctgcccttcaacgacggtgtgtacttcgcttccaccgagaagtccaacatcatccgtggttggatcttcggtaccaccctggactccaagacccagtccctgctgatcgtgaacaacgctaccaacgtggtgatcaaggtgtgcgagttccagttctgcaacgaccccttcctgggtgtgtactaccacaagaacaacaagtcctggatggagtccgagttccgtgtgtactcctccgctaacaactgcaccttcgagtacgtgtcccagcccttcctgatggacctggagggtaagcagggtaacttcaagaacctgcgtgagttcgtgttcaagaacatcgacggttacttcaagatctactccaagcacacccccatcaacctggtgcgtggtctgccccagggtttctccgctctggagcccctggtggacctgcccatcggtatcaacatcacccgtttccagaccctgcaccgttcctacctgacccccggtgactcctcctccggttggaccgctggtgctgctgcttactacgtgggttacctgcagccccgtaccttcctgctgaagtacaacgagaacggtaccatcaccgacgctgtggactgcgctctggaccccctgtccgagaccaagtgcaccctgaagtccttcaccgtggagaagggtatctaccagacctccaacttccgtgtgcagcccaccgagtccatcgtgcgtttccccaacatcaccaacctgtgccccttcggtgaggtgttcaacgctacccgtttcgcttccgtgtacgcttggaaccgtaagcgtatctccaactgcgtggctgactactccgtgctgtacaactccgcttccttctccaccttcaagtgctacggtgtgtcccccaccaagctgaacgacctgtgcttcaccaacgtgtacgctgactccttcgtgatccgtggtgacgaggtgcgtcagatcgctcccggtcagaccggtaacatcgctgactacaactacaagctgcccgacgacttcaccggttgcgtgatcgcttggaactccaacaacctggactccaaggtgggtggtaactacaactacctgtaccgtctgttccgtaagtccaacctgaagcccttcgagcgtgacatctccaccgagatctaccaggctggttccaccccctgcaacggtgtgaagggtttcaactgctacttccccctgcagtcctacggtttccagcccacctacggtgtgggttaccagccctaccgtgtggtggtgctgtccttcgagctgctgcacgctcccgctaccgtgtgcggtcccaagaagtccaccaacctggtgaagaacaagtgcgtgaacttcaacttcaacggtctgaccggtaccggtgtgctgaccgagtccaacaagaagttcctgcccttccagcagttcggtcgtgacatcgctgacaccaccgacgctgtgcgtgacccccagaccctggagatcctggacatcaccccctgctccttcggtggtgtgtccgtgatcacccccggtaccaacacctccaaccaggtggctgtgctgtaccagggtgtgaactgcaccgaggtgcccgtggctatccacgctgaccagctgacccccacctggcgtgtgtactccaccggttccaacgtgttccagacccgtgctggttgcctgatcggtgctgagcacgtgaacaactcctacgagtgcgacatccccatcggtgctggtatctgcgcttcctaccagacccagaccaactccccccgtcgtgctcgttccgtggcttcccagtccatcatcgcttacaccatgtccctgggtgtggagaactccgtggcttactccaacaactccatcgctatccccaccaacttcaccatctccgtgaccaccgagatcctgcccgtgtccatgaccaagacctccgtggactgcaccatgtacatctgcggtgactccaccgagtgctccaacctgctgctgcagtacggttccttctgcacccagctgaaccgtgctctgaccggtatcgctgtggagcaggacaagaacacccaggaggtgttcgctcaggtgaagcagatctacaagaccccccccatcaaggacttcggtggtttcaacttctcccagatcctgcccgacccctccaagccctccaagcgttccttcatcgaggacctgctgttcaacaaggtgaccctggctgacgctggtttcatcaagcagtacggtgactgcctgggtgacatcgctgctcgtgacctgatctgcgctcagaagttcaacggtctgaccgtgctgccccccctgctgaccgacgagatgatcgctcagtacacctccgctctgctggctggtaccatcacctccggttggaccttcggtgctggtgctgctctgcagatccccttcgctatgcagatggcttaccgtttcaacggtatcggtgtgacccagaacgtgctgtacgagaaccagaagctgatcgctaaccagttcaactccgctatcggtaagatccaggactccctgtcctccaccgcttccgctctgggtaagctgcaggacgtggtgaaccagaacgctcaggctctgaacaccctggtgaagcagctgtcctccaacttcggtgctatctcctccgtgctgaacgacatcctgtcccgtctggacaaggtggaggctgaggtgcagatcgaccgtctgatcaccggtcgtctgcagtccctgcagacctacgtgacccagcagctgatccgtgctgctgagatccgtgcttccgctaacctggctgctaccaagatgtccgagtgcgtgctgggtcagtccaagcgtgtggacttctgcggtaagggttaccacctgatgtccttcccccagtccgctccccacggtgtggtgttcctgcacgtgacctacgtgcccgctcaggagaagaacttcaccaccgctcccgctatctgccacgacggtaaggctcacttcccccgtgagggtgtgttcgtgtccaacggtacccactggttcgtgacccagcgtaacttctacgagccccagatcatcaccaccgacaacaccttcgtgtccggtaactgcgacgtggtgatcggtatcgtgaacaacaccgtgtacgaccccctgcagcccgagctggactccttcaaggaggagctggacaagtacttcaagaaccacacctcccccgacgtggacctgggtgacatctccggtatcaacgcttccgtggtgaacatccagaaggagatcgaccgtctgaacgaggtggctaagaacctgaacgagtccctgatcgacctgcaggagctgggtaagtacgagcagtacatcaagtggccctag

SEQ ID NO: 52 - protein, 1271 aa, synthetic construct
MFVFLVLLPLVSSQCVNLRTRTQLPPAYTNSFTRGVYYPDKVFRSSVLHSTQDLFLPFFSNVTWFHAIHVSGTNGTKRFDNPVLPFNDGVYFASTEKSNIIRGWIFGTTLDSKTQSLLIVNNATNVVIKVCEFQFCNDPFLDVYYHKNNKSWMESGVYSSANNCTFEYVSQPFLMDLEGKQGNFKNLREFVFKNIDGYFKIYSKHTPINLVRDLPQGFSALEPLVDLPIGINITRFQTLLALHRSYLTPGDSSSGWTAGAAAYYVGYLQPRTFLLKYNENGTITDAVDCALDPLSETKCTLKSFTVEKGIYQTSNFRVQPTESIVRFPNITNLCPFGEVFNATRFASVYAWNRKRISNCVADYSVLYNSASFSTFKCYGVSPTKLNDLCFTNVYADSFVIRGDEVRQIAPGQTGKIADYNYKLPDDFTGCVIAWNSNNLDSKVGGNYNYRYRLFRKSNLKPFERDISTEIYQAGSKPCNGVEGFNCYFPLQSYGFQPTNGVGYQPYRVVVLSFELLHAPATVCGPKKSTNLVKNKCVNFNFNGLTGTGVLTESNKKFLPFQQFGRDIADTTDAVRDPQTLEILDITPCSFGGVSVITPGTNTSNQVAVLYQGVNCTEVPVAIHADQLTPTWRVYSTGSNVFQTRAGCLIGAEHVNNSYECDIPIGAGICASYQTQTNSRRRARSVASQSIIAYTMSLGAENSVAYSNNSIAIPTNFTISVTTEILPVSMTKTSVDCTMYICGDSTECSNLLLQYGSFCTQLNRALTGIAVEQDKNTQEVFAQVKQIYKTPPIKDFGGFNFSQILPDPSKPSKRSFIEDLLFNKVTLADAGFIKQYGDCLGDIAARDLICAQKFNGLTVLPPLLTDEMIAQYTSALLAGTITSGWTFGAGAALQIPFAMQMAYRFNGIGVTQNVLYENQKLIANQFNSAIGKIQDSLSSTASALGKLQNVVNQNAQALNTLVKQLSSNFGAISSVLNDILSRLDKVEAEVQIDRLITGRLQSLQTYVTQQLIRAAEIRASANLAATKMSECVLGQSKRVDFCGKGYHLMSFPQSAPHGVVFLHVTYVPAQEKNFTTAPAICHDGKAHFPREGVFVSNGTHWFVTQRNFYEPQIITTDNTFVSGNCDVVIGIVNNTVYDPLQPELDSFKEELDKYFKNHTSPDVDLGDISGINASVVNIQKEIDRLNEVAKNLNESLIDLQELGKYEQYIKWPWYIWLGFIAGLIAIVMVTIMLCCMTSCCSCLKGCCSCGSCCKFDEDDSEPVLKGVKLHYT

SEQ ID NO: 53 - DNA, 3816 bp, synthetic construct
  source 1..3816: mol_type = other DNA
atgttcgtgttcctggtgctgctgcccctggtgagcagccagtgcgtgaacctgagaaccagaacccagctgccccccgcctacaccaacagcttcaccagaggcgtgtactaccccgacaaggtgttcagaagcagcgtgctgcacagcacccaggacctgttcctgcccttcttcagcaacgtgacctggttccacgccatccacgtgagcggcaccaacggcaccaagagattcgacaaccccgtgctgcccttcaacgacggcgtgtacttcgccagcaccgagaagagcaacatcatcagaggctggatcttcggcaccaccctggacagcaagacccagagcctgctgatcgtgaacaacgccaccaacgtggtgatcaaggtgtgcgagttccagttctgcaacgaccccttcctggacgtgtactaccacaagaacaacaagagctggatggagagcggcgtgtacagcagcgccaacaactgcaccttcgagtacgtgagccagcccttcctgatggacctggagggcaagcagggcaacttcaagaacctgagagagttcgtgttcaagaacatcgacggctacttcaagatctacagcaagcacacccccatcaacctggtgagagacctgccccagggcttcagcgccctggagcccctggtggacctgcccatcggcatcaacatcaccagattccagaccctgctggccctgcacagaagctacctgacccccggcgacagcagcagcggctggaccgccggcgccgccgcctactacgtgggctacctgcagcccagaaccttcctgctgaagtacaacgagaacggcaccatcaccgacgccgtggactgcgccctggaccccctgagcgagaccaagtgcaccctgaagagcttcaccgtggagaagggcatctaccagaccagcaacttcagagtgcagcccaccgagagcatcgtgagattccccaacatcaccaacctgtgccccttcggcgaggtgttcaacgccaccagattcgccagcgtgtacgcctggaacagaaagagaatcagcaactgcgtggccgactacagcgtgctgtacaacagcgccagcttcagcaccttcaagtgctacggcgtgagccccaccaagctgaacgacctgtgcttcaccaacgtgtacgccgacagcttcgtgatcagaggcgacgaggtgagacagatcgcccccggccagaccggcaagatcgccgactacaactacaagctgcccgacgacttcaccggctgcgtgatcgcctggaacagcaacaacctggacagcaaggtgggcggcaactacaactacagatacagactgttcagaaagagcaacctgaagcccttcgagagagacatcagcaccgagatctaccaggccggcagcaagccctgcaacggcgtggagggcttcaactgctacttccccctgcagagctacggcttccagcccaccaacggcgtgggctaccagccctacagagtggtggtgctgagcttcgagctgctgcacgcccccgccaccgtgtgcggccccaagaagagcaccaacctggtgaagaacaagtgcgtgaacttcaacttcaacggcctgaccggcaccggcgtgctgaccgagagcaacaagaagttcctgcccttccagcagttcggcagagacatcgccgacaccaccgacgccgtgagagacccccagaccctggagatcctggacatcaccccctgcagcttcggcggcgtgagcgtgatcacccccggcaccaacaccagcaaccaggtggccgtgctgtaccagggcgtgaactgcaccgaggtgcccgtggccatccacgccgaccagctgacccccacctggagagtgtacagcaccggcagcaacgtgttccagaccagagccggctgcctgatcggcgccgagcacgtgaacaacagctacgagtgcgacatccccatcggcgccggcatctgcgccagctaccagacccagaccaacagcagaagaagagccagaagcgtggccagccagagcatcatcgcctacaccatgagcctgggcgccgagaacagcgtggcctacagcaacaacagcatcgccatccccaccaacttcaccatcagcgtgaccaccgagatcctgcccgtgagcatgaccaagaccagcgtggactgcaccatgtacatctgcggcgacagcaccgagtgcagcaacctgctgctgcagtacggcagcttctgcacccagctgaacagagccctgaccggcatcgccgtggagcaggacaagaacacccaggaggtgttcgcccaggtgaagcagatctacaagaccccccccatcaaggacttcggcggcttcaacttcagccagatcctgcccgaccccagcaagcccagcaagagaagcttcatcgaggacctgctgttcaacaaggtgaccctggccgacgccggcttcatcaagcagtacggcgactgcctgggcgacatcgccgccagagacctgatctgcgcccagaagttcaacggcctgaccgtgctgccccccctgctgaccgacgagatgatcgcccagtacaccagcgccctgctggccggcaccatcaccagcggctggaccttcggcgccggcgccgccctgcagatccccttcgccatgcagatggcctacagattcaacggcatcggcgtgacccagaacgtgctgtacgagaaccagaagctgatcgccaaccagttcaacagcgccatcggcaagatccaggacagcctgagcagcaccgccagcgccctgggcaagctgcagaacgtggtgaaccagaacgcccaggccctgaacaccctggtgaagcagctgagcagcaacttcggcgccatcagcagcgtgctgaacgacatcctgagcagactggacaaggtggaggccgaggtgcagatcgacagactgatcaccggcagactgcagagcctgcagacctacgtgacccagcagctgatcagagccgccgagatcagagccagcgccaacctggccgccaccaagatgagcgagtgcgtgctgggccagagcaagagagtggacttctgcggcaagggctaccacctgatgagcttcccccagagcgccccccacggcgtggtgttcctgcacgtgacctacgtgcccgcccaggagaagaacttcaccaccgcccccgccatctgccacgacggcaaggcccacttccccagagagggcgtgttcgtgagcaacggcacccactggttcgtgacccagagaaacttctacgagccccagatcatcaccaccgacaacaccttcgtgagcggcaactgcgacgtggtgatcggcatcgtgaacaacaccgtgtacgaccccctgcagcccgagctggacagcttcaaggaggagctggacaagtacttcaagaaccacaccagccccgacgtggacctgggcgacatcagcggcatcaacgccagcgtggtgaacatccagaaggagatcgacagactgaacgaggtggccaagaacctgaacgagagcctgatcgacctgcaggagctgggcaagtacgagcagtacatcaagtggccctggtacatctggctgggcttcatcgccggcctgatcgccatcgtgatggtgaccatcatgctgtgctgcatgaccagctgctgcagctgcctgaagggctgctgcagctgcggcagctgctgcaagttcgacgaggacgacagcgagcccgtgctgaagggcgtgaagctgcactacacctag

SEQ ID NO: 54 - DNA, 3816 bp, synthetic construct
  source 1..3816: mol_type = other DNA
atgttcgtgttcctggtgctgctgcccctggtgtcctcccagtgcgtgaacctgcgtacccgtacccagctgccccccgcttacaccaactccttcacccgtggtgtgtactaccccgacaaggtgttccgttcctccgtgctgcactccacccaggacctgttcctgcccttcttctccaacgtgacctggttccacgctatccacgtgtccggtaccaacggtaccaagcgtttcgacaaccccgtgctgcccttcaacgacggtgtgtacttcgcttccaccgagaagtccaacatcatccgtggttggatcttcggtaccaccctggactccaagacccagtccctgctgatcgtgaacaacgctaccaacgtggtgatcaaggtgtgcgagttccagttctgcaacgaccccttcctggacgtgtactaccacaagaacaacaagtcctggatggagtccggtgtgtactcctccgctaacaactgcaccttcgagtacgtgtcccagcccttcctgatggacctggagggtaagcagggtaacttcaagaacctgcgtgagttcgtgttcaagaacatcgacggttacttcaagatctactccaagcacacccccatcaacctggtgcgtgacctgccccagggtttctccgctctggagcccctggtggacctgcccatcggtatcaacatcacccgtttccagaccctgctggctctgcaccgttcctacctgacccccggtgactcctcctccggttggaccgctggtgctgctgcttactacgtgggttacctgcagccccgtaccttcctgctgaagtacaacgagaacggtaccatcaccgacgctgtggactgcgctctggaccccctgtccgagaccaagtgcaccctgaagtccttcaccgtggagaagggtatctaccagacctccaacttccgtgtgcagcccaccgagtccatcgtgcgtttccccaacatcaccaacctgtgccccttcggtgaggtgttcaacgctacccgtttcgcttccgtgtacgcttggaaccgtaagcgtatctccaactgcgtggctgactactccgtgctgtacaactccgcttccttctccaccttcaagtgctacggtgtgtcccccaccaagctgaacgacctgtgcttcaccaacgtgtacgctgactccttcgtgatccgtggtgacgaggtgcgtcagatcgctcccggtcagaccggtaagatcgctgactacaactacaagctgcccgacgacttcaccggttgcgtgatcgcttggaactccaacaacctggactccaaggtgggtggtaactacaactaccgttaccgtctgttccgtaagtccaacctgaagcccttcgagcgtgacatctccaccgagatctaccaggctggttccaagccctgcaacggtgtggagggtttcaactgctacttccccctgcagtcctacggtttccagcccaccaacggtgtgggttaccagccctaccgtgtggtggtgctgtccttcgagctgctgcacgctcccgctaccgtgtgcggtcccaagaagtccaccaacctggtgaagaacaagtgcgtgaacttcaacttcaacggtctgaccggtaccggtgtgctgaccgagtccaacaagaagttcctgcccttccagcagttcggtcgtgacatcgctgacaccaccgacgctgtgcgtgacccccagaccctggagatcctggacatcaccccctgctccttcggtggtgtgtccgtgatcacccccggtaccaacacctccaaccaggtggctgtgctgtaccagggtgtgaactgcaccgaggtgcccgtggctatccacgctgaccagctgacccccacctggcgtgtgtactccaccggttccaacgtgttccagacccgtgctggttgcctgatcggtgctgagcacgtgaacaactcctacgagtgcgacatccccatcggtgctggtatctgcgcttcctaccagacccagaccaactcccgtcgtcgtgctcgttccgtggcttcccagtccatcatcgcttacaccatgtccctgggtgctgagaactccgtggcttactccaacaactccatcgctatccccaccaacttcaccatctccgtgaccaccgagatcctgcccgtgtccatgaccaagacctccgtggactgcaccatgtacatctgcggtgactccaccgagtgctccaacctgctgctgcagtacggttccttctgcacccagctgaaccgtgctctgaccggtatcgctgtggagcaggacaagaacacccaggaggtgttcgctcaggtgaagcagatctacaagaccccccccatcaaggacttcggtggtttcaacttctcccagatcctgcccgacccctccaagccctccaagcgttccttcatcgaggacctgctgttcaacaaggtgaccctggctgacgctggtttcatcaagcagtacggtgactgcctgggtgacatcgctgctcgtgacctgatctgcgctcagaagttcaacggtctgaccgtgctgccccccctgctgaccgacgagatgatcgctcagtacacctccgctctgctggctggtaccatcacctccggttggaccttcggtgctggtgctgctctgcagatccccttcgctatgcagatggcttaccgtttcaacggtatcggtgtgacccagaacgtgctgtacgagaaccagaagctgatcgctaaccagttcaactccgctatcggtaagatccaggactccctgtcctccaccgcttccgctctgggtaagctgcagaacgtggtgaaccagaacgctcaggctctgaacaccctggtgaagcagctgtcctccaacttcggtgctatctcctccgtgctgaacgacatcctgtcccgtctggacaaggtggaggctgaggtgcagatcgaccgtctgatcaccggtcgtctgcagtccctgcagacctacgtgacccagcagctgatccgtgctgctgagatccgtgcttccgctaacctggctgctaccaagatgtccgagtgcgtgctgggtcagtccaagcgtgtggacttctgcggtaagggttaccacctgatgtccttcccccagtccgctccccacggtgtggtgttcctgcacgtgacctacgtgcccgctcaggagaagaacttcaccaccgctcccgctatctgccacgacggtaaggctcacttcccccgtgagggtgtgttcgtgtccaacggtacccactggttcgtgacccagcgtaacttctacgagccccagatcatcaccaccgacaacaccttcgtgtccggtaactgcgacgtggtgatcggtatcgtgaacaacaccgtgtacgaccccctgcagcccgagctggactccttcaaggaggagctggacaagtacttcaagaaccacacctcccccgacgtggacctgggtgacatctccggtatcaacgcttccgtggtgaacatccagaaggagatcgaccgtctgaacgaggtggctaagaacctgaacgagtccctgatcgacctgcaggagctgggtaagtacgagcagtacatcaagtggccctggtacatctggctgggtttcatcgctggtctgatcgctatcgtgatggtgaccatcatgctgtgctgcatgacctcctgctgctcctgcctgaagggttgctgctcctgcggttcctgctgcaagttcgacgaggacgactccgagcccgtgctgaagggtgtgaagctgcactacacctag

SEQ ID NO: 55 - protein, 1211 aa, synthetic construct
MFVFLVLLPLVSSQCVNLRTRTQLPPAYTNSFTRGVYYPDKVFRSSVLHSTQDLFLPFFSNVTWFHAIHVSGTNGTKRFDNPVLPFNDGVYFASTEKSNIIRGWIFGTTLDSKTQSLLIVNNATNVVIKVCEFQFCNDPFLDVYYHKNNKSWMESGVYSSANNCTFEYVSQPFLMDLEGKQGNFKNLREFVFKNIDGYFKIYSKHTPINLVRDLPQGFSALEPLVDLPIGINITRFQTLLALHRSYLTPGDSSSGWTAGAAAYYVGYLQPRTFLLKYNENGTITDAVDCALDPLSETKCTLKSFTVEKGIYQTSNFRVQPTESIVRFPNITNLCPFGEVFNATRFASVYAWNRKRISNCVADYSVLYNSASFSTFKCYGVSPTKLNDLCFTNVYADSFVIRGDEVRQIAPGQTGKIADYNYKLPDDFTGCVIAWNSNNLDSKVGGNYNYRYRLFRKSNLKPFERDISTEIYQAGSKPCNGVEGFNCYFPLQSYGFQPTNGVGYQPYRVVVLSFELLHAPATVCGPKKSTNLVKNKCVNFNFNGLTGTGVLTESNKKFLPFQQFGRDIADTTDAVRDPQTLEILDITPCSFGGVSVITPGTNTSNQVAVLYQGVNCTEVPVAIHADQLTPTWRVYSTGSNVFQTRAGCLIGAEHVNNSYECDIPIGAGICASYQTQTNSRRRARSVASQSIIAYTMSLGAENSVAYSNNSIAIPTNFTISVTTEILPVSMTKTSVDCTMYICGDSTECSNLLLQYGSFCTQLNRALTGIAVEQDKNTQEVFAQVKQIYKTPPIKDFGGFNFSQILPDPSKPSKRSFIEDLLFNKVTLADAGFIKQYGDCLGDIAARDLICAQKFNGLTVLPPLLTDEMIAQYTSALLAGTITSGWTFGAGAALQIPFAMQMAYRFNGIGVTQNVLYENQKLIANQFNSAIGKIQDSLSSTASALGKLQNVVNQNAQALNTLVKQLSSNFGAISSVLNDILSRLDKVEAEVQIDRLITGRLQSLQTYVTQQLIRAAEIRASANLAATKMSECVLGQSKRVDFCGKGYHLMSFPQSAPHGVVFLHVTYVPAQEKNFTTAPAICHDGKAHFPREGVFVSNGTHWFVTQRNFYEPQIITTDNTFVSGNCDVVIGIVNNTVYDPLQPELDSFKEELDKYFKNHTSPDVDLGDISGINASVVNIQKEIDRLNEVAKNLNESLIDLQELGKYEQYIKWP

SEQ ID NO: 56 - DNA, 3636 bp, synthetic construct
  source 1..3636: mol_type = other DNA
atgttcgtgttcctggtgctgctgcccctggtgagcagccagtgcgtgaacctgagaaccagaacccagctgccccccgcctacaccaacagcttcaccagaggcgtgtactaccccgacaaggtgttcagaagcagcgtgctgcacagcacccaggacctgttcctgcccttcttcagcaacgtgacctggttccacgccatccacgtgagcggcaccaacggcaccaagagattcgacaaccccgtgctgcccttcaacgacggcgtgtacttcgccagcaccgagaagagcaacatcatcagaggctggatcttcggcaccaccctggacagcaagacccagagcctgctgatcgtgaacaacgccaccaacgtggtgatcaaggtgtgcgagttccagttctgcaacgaccccttcctggacgtgtactaccacaagaacaacaagagctggatggagagcggcgtgtacagcagcgccaacaactgcaccttcgagtacgtgagccagcccttcctgatggacctggagggcaagcagggcaacttcaagaacctgagagagttcgtgttcaagaacatcgacggctacttcaagatctacagcaagcacacccccatcaacctggtgagagacctgccccagggcttcagcgccctggagcccctggtggacctgcccatcggcatcaacatcaccagattccagaccctgctggccctgcacagaagctacctgacccccggcgacagcagcagcggctggaccgccggcgccgccgcctactacgtgggctacctgcagcccagaaccttcctgctgaagtacaacgagaacggcaccatcaccgacgccgtggactgcgccctggaccccctgagcgagaccaagtgcaccctgaagagcttcaccgtggagaagggcatctaccagaccagcaacttcagagtgcagcccaccgagagcatcgtgagattccccaacatcaccaacctgtgccccttcggcgaggtgttcaacgccaccagattcgccagcgtgtacgcctggaacagaaagagaatcagcaactgcgtggccgactacagcgtgctgtacaacagcgccagcttcagcaccttcaagtgctacggcgtgagccccaccaagctgaacgacctgtgcttcaccaacgtgtacgccgacagcttcgtgatcagaggcgacgaggtgagacagatcgcccccggccagaccggcaagatcgccgactacaactacaagctgcccgacgacttcaccggctgcgtgatcgcctggaacagcaacaacctggacagcaaggtgggcggcaactacaactacagatacagactgttcagaaagagcaacctgaagcccttcgagagagacatcagcaccgagatctaccaggccggcagcaagccctgcaacggcgtggagggcttcaactgctacttccccctgcagagctacggcttccagcccaccaacggcgtgggctaccagccctacagagtggtggtgctgagcttcgagctgctgcacgcccccgccaccgtgtgcggccccaagaagagcaccaacctggtgaagaacaagtgcgtgaacttcaacttcaacggcctgaccggcaccggcgtgctgaccgagagcaacaagaagttcctgcccttccagcagttcggcagagacatcgccgacaccaccgacgccgtgagagacccccagaccctggagatcctggacatcaccccctgcagcttcggcggcgtgagcgtgatcacccccggcaccaacaccagcaaccaggtggccgtgctgtaccagggcgtgaactgcaccgaggtgcccgtggccatccacgccgaccagctgacccccacctggagagtgtacagcaccggcagcaacgtgttccagaccagagccggctgcctgatcggcgccgagcacgtgaacaacagctacgagtgcgacatccccatcggcgccggcatctgcgccagctaccagacccagaccaacagcagaagaagagccagaagcgtggccagccagagcatcatcgcctacaccatgagcctgggcgccgagaacagcgtggcctacagcaacaacagcatcgccatccccaccaacttcaccatcagcgtgaccaccgagatcctgcccgtgagcatgaccaagaccagcgtggactgcaccatgtacatctgcggcgacagcaccgagtgcagcaacctgctgctgcagtacggcagcttctgcacccagctgaacagagccctgaccggcatcgccgtggagcaggacaagaacacccaggaggtgttcgcccaggtgaagcagatctacaagaccccccccatcaaggacttcggcggcttcaacttcagccagatcctgcccgaccccagcaagcccagcaagagaagcttcatcgaggacctgctgttcaacaaggtgaccctggccgacgccggcttcatcaagcagtacggcgactgcctgggcgacatcgccgccagagacctgatctgcgcccagaagttcaacggcctgaccgtgctgccccccctgctgaccgacgagatgatcgcccagtacaccagcgccctgctggccggcaccatcaccagcggctggaccttcggcgccggcgccgccctgcagatccccttcgccatgcagatggcctacagattcaacggcatcggcgtgacccagaacgtgctgtacgagaaccagaagctgatcgccaaccagttcaacagcgccatcggcaagatccaggacagcctgagcagcaccgccagcgccctgggcaagctgcagaacgtggtgaaccagaacgcccaggccctgaacaccctggtgaagcagctgagcagcaacttcggcgccatcagcagcgtgctgaacgacatcctgagcagactggacaaggtggaggccgaggtgcagatcgacagactgatcaccggcagactgcagagcctgcagacctacgtgacccagcagctgatcagagccgccgagatcagagccagcgccaacctggccgccaccaagatgagcgagtgcgtgctgggccagagcaagagagtggacttctgcggcaagggctaccacctgatgagcttcccccagagcgccccccacggcgtggtgttcctgcacgtgacctacgtgcccgcccaggagaagaacttcaccaccgcccccgccatctgccacgacggcaaggcccacttccccagagagggcgtgttcgtgagcaacggcacccactggttcgtgacccagagaaacttctacgagccccagatcatcaccaccgacaacaccttcgtgagcggcaactgcgacgtggtgatcggcatcgtgaacaacaccgtgtacgaccccctgcagcccgagctggacagcttcaaggaggagctggacaagtacttcaagaaccacaccagccccgacgtggacctgggcgacatcagcggcatcaacgccagcgtggtgaacatccagaaggagatcgacagactgaacgaggtggccaagaacctgaacgagagcctgatcgacctgcaggagctgggcaagtacgagcagtacatcaagtggccctag

SEQ ID NO: 57 - DNA, 3636 bp, synthetic construct
  source 1..3636: mol_type = other DNA
atgttcgtgttcctggtgctgctgcccctggtgtcctcccagtgcgtgaacctgcgtacccgtacccagctgccccccgcttacaccaactccttcacccgtggtgtgtactaccccgacaaggtgttccgttcctccgtgctgcactccacccaggacctgttcctgcccttcttctccaacgtgacctggttccacgctatccacgtgtccggtaccaacggtaccaagcgtttcgacaaccccgtgctgcccttcaacgacggtgtgtacttcgcttccaccgagaagtccaacatcatccgtggttggatcttcggtaccaccctggactccaagacccagtccctgctgatcgtgaacaacgctaccaacgtggtgatcaaggtgtgcgagttccagttctgcaacgaccccttcctggacgtgtactaccacaagaacaacaagtcctggatggagtccggtgtgtactcctccgctaacaactgcaccttcgagtacgtgtcccagcccttcctgatggacctggagggtaagcagggtaacttcaagaacctgcgtgagttcgtgttcaagaacatcgacggttacttcaagatctactccaagcacacccccatcaacctggtgcgtgacctgccccagggtttctccgctctggagcccctggtggacctgcccatcggtatcaacatcacccgtttccagaccctgctggctctgcaccgttcctacctgacccccggtgactcctcctccggttggaccgctggtgctgctgcttactacgtgggttacctgcagccccgtaccttcctgctgaagtacaacgagaacggtaccatcaccgacgctgtggactgcgctctggaccccctgtccgagaccaagtgcaccctgaagtccttcaccgtggagaagggtatctaccagacctccaacttccgtgtgcagcccaccgagtccatcgtgcgtttccccaacatcaccaacctgtgccccttcggtgaggtgttcaacgctacccgtttcgcttccgtgtacgcttggaaccgtaagcgtatctccaactgcgtggctgactactccgtgctgtacaactccgcttccttctccaccttcaagtgctacggtgtgtcccccaccaagctgaacgacctgtgcttcaccaacgtgtacgctgactccttcgtgatccgtggtgacgaggtgcgtcagatcgctcccggtcagaccggtaagatcgctgactacaactacaagctgcccgacgacttcaccggttgcgtgatcgcttggaactccaacaacctggactccaaggtgggtggtaactacaactaccgttaccgtctgttccgtaagtccaacctgaagcccttcgagcgtgacatctccaccgagatctaccaggctggttccaagccctgcaacggtgtggagggtttcaactgctacttccccctgcagtcctacggtttccagcccaccaacggtgtgggttaccagccctaccgtgtggtggtgctgtccttcgagctgctgcacgctcccgctaccgtgtgcggtcccaagaagtccaccaacctggtgaagaacaagtgcgtgaacttcaacttcaacggtctgaccggtaccggtgtgctgaccgagtccaacaagaagttcctgcccttccagcagttcggtcgtgacatcgctgacaccaccgacgctgtgcgtgacccccagaccctggagatcctggacatcaccccctgctccttcggtggtgtgtccgtgatcacccccggtaccaacacctccaaccaggtggctgtgctgtaccagggtgtgaactgcaccgaggtgcccgtggctatccacgctgaccagctgacccccacctggcgtgtgtactccaccggttccaacgtgttccagacccgtgctggttgcctgatcggtgctgagcacgtgaacaactcctacgagtgcgacatccccatcggtgctggtatctgcgcttcctaccagacccagaccaactcccgtcgtcgtgctcgttccgtggcttcccagtccatcatcgcttacaccatgtccctgggtgctgagaactccgtggcttactccaacaactccatcgctatccccaccaacttcaccatctccgtgaccaccgagatcctgcccgtgtccatgaccaagacctccgtggactgcaccatgtacatctgcggtgactccaccgagtgctccaacctgctgctgcagtacggttccttctgcacccagctgaaccgtgctctgaccggtatcgctgtggagcaggacaagaacacccaggaggtgttcgctcaggtgaagcagatctacaagaccccccccatcaaggacttcggtggtttcaacttctcccagatcctgcccgacccctccaagccctccaagcgttccttcatcgaggacctgctgttcaacaaggtgaccctggctgacgctggtttcatcaagcagtacggtgactgcctgggtgacatcgctgctcgtgacctgatctgcgctcagaagttcaacggtctgaccgtgctgccccccctgctgaccgacgagatgatcgctcagtacacctccgctctgctggctggtaccatcacctccggttggaccttcggtgctggtgctgctctgcagatccccttcgctatgcagatggcttaccgtttcaacggtatcggtgtgacccagaacgtgctgtacgagaaccagaagctgatcgctaaccagttcaactccgctatcggtaagatccaggactccctgtcctccaccgcttccgctctgggtaagctgcagaacgtggtgaaccagaacgctcaggctctgaacaccctggtgaagcagctgtcctccaacttcggtgctatctcctccgtgctgaacgacatcctgtcccgtctggacaaggtggaggctgaggtgcagatcgaccgtctgatcaccggtcgtctgcagtccctgcagacctacgtgacccagcagctgatccgtgctgctgagatccgtgcttccgctaacctggctgctaccaagatgtccgagtgcgtgctgggtcagtccaagcgtgtggacttctgcggtaagggttaccacctgatgtccttcccccagtccgctccccacggtgtggtgttcctgcacgtgacctacgtgcccgctcaggagaagaacttcaccaccgctcccgctatctgccacgacggtaaggctcacttcccccgtgagggtgtgttcgtgtccaacggtacccactggttcgtgacccagcgtaacttctacgagccccagatcatcaccaccgacaacaccttcgtgtccggtaactgcgacgtggtgatcggtatcgtgaacaacaccgtgtacgaccccctgcagcccgagctggactccttcaaggaggagctggacaagtacttcaagaaccacacctcccccgacgtggacctgggtgacatctccggtatcaacgcttccgtggtgaacatccagaaggagatcgaccgtctgaacgaggtggctaagaacctgaacgagtccctgatcgacctgcaggagctgggtaagtacgagcagtacatcaagtggccctag

SEQ ID NO: 58 - protein, 1267 aa, synthetic construct
MFVFLVLLPLVSSQCVNLTTRTQLPPAYTNSFTRGVYYPDKVFRSSVLHSTQDLFLPFFSNVTWFHVISGTNGTKRFDNPVLPFNDGVYFASIEKSNIIRGWIFGTTLDSKTQSLLIVNNATNVVIKVCEFQFCNDPFLDHKNNKSWMESEFRVYSSANNCTFEYVSQPFLMDLEGKQGNFKNLREFVFKNIDGYFKIYSKHTPIIVRDLPQGFSALEPLVDLPIGINITRFQTLLALHRSYLTPGDSSSGWTAGAAAYYVGYLQPRTFLLKYNENGTITDAVDCALDPLSETKCTLKSFTVEKGIYQTSNFRVQPTESIVRFPNITNLCPFDEVFNATRFASVYAWNRKRISNCVADYSVLYNLAPFFTFKCYGVSPTKLNDLCFTNVYADSFVIRGDEVRQIAPGQTGNIADYNYKLPDDFTGCVIAWNSNKLDSKVSGNYNYLYRLFRKSNLKPFERDISTEIYQAGNKPCNGVAGFNCYFPLRSYSFRPTYGVGHQPYRVVVLSFELLHAPATVCGPKKSTNLVKNKCVNFNFNGLKGTGVLTESNKKFLPFQQFGRDIADTTDAVRDPQTLEILDITPCSFGGVSVITPGTNTSNQVAVLYQGVNCTEVPVAIHADQLTPTWRVYSTGSNVFQTRAGCLIGAEYVNNSYECDIPIGAGICASYQTQTKSHRRARSVASQSIIAYTMSLGAENSVAYSNNSIAIPTNFTISVTTEILPVSMTKTSVDCTMYICGDSTECSNLLLQYGSFCTQLKRALTGIAVEQDKNTQEVFAQVKQIYKTPPIKYFGGFNFSQILPDPSKPSKRSFIEDLLFNKVTLADAGFIKQYGDCLGDIAARDLICAQKFKGLTVLPPLLTDEMIAQYTSALLAGTITSGWTFGAGAALQIPFAMQMAYRFNGIGVTQNVLYENQKLIANQFNSAIGKIQDSLSSTASALGKLQDVVNHNAQALNTLVKQLSSKFGAISSVLNDIFSRLDKVEAEVQIDRLITGRLQSLQTYVTQQLIRAAEIRASANLAATKMSECVLGQSKRVDFCGKGYHLMSFPQSAPHGVVFLHVTYVPAQEKNFTTAPAICHDGKAHFPREGVFVSNGTHWFVTQRNFYEPQIITTDNTFVSGNCDVVIGIVNNTVYDPLQPELDSFKEELDKYFKNHTSPDVDLGDISGINASVVNIQKEIDRLNEVAKNLNESLIDLQELGKYEQYIKWPWYIWLGFIAGLIAIVMVTIMLCCMTSCCSCLKGCCSCGSCCKFDEDDSEPVLKGVKLHYT

SEQ ID NO: 59 - DNA, 3804 bp, synthetic construct
  source 1..3804: mol_type = other DNA
atgttcgtgttcctggtgctgctgcccctggtgagcagccagtgcgtgaacctgaccaccagaacccagctgccccccgcctacaccaacagcttcaccagaggcgtgtactaccccgacaaggtgttcagaagcagcgtgctgcacagcacccaggacctgttcctgcccttcttcagcaacgtgacctggttccacgtgatcagcggcaccaacggcaccaagagattcgacaaccccgtgctgcccttcaacgacggcgtgtacttcgccagcatcgagaagagcaacatcatcagaggctggatcttcggcaccaccctggacagcaagacccagagcctgctgatcgtgaacaacgccaccaacgtggtgatcaaggtgtgcgagttccagttctgcaacgaccccttcctggaccacaagaacaacaagagctggatggagagcgagttcagagtgtacagcagcgccaacaactgcaccttcgagtacgtgagccagcccttcctgatggacctggagggcaagcagggcaacttcaagaacctgagagagttcgtgttcaagaacatcgacggctacttcaagatctacagcaagcacacccccatcatcgtgagagacctgccccagggcttcagcgccctggagcccctggtggacctgcccatcggcatcaacatcaccagattccagaccctgctggccctgcacagaagctacctgacccccggcgacagcagcagcggctggaccgccggcgccgccgcctactacgtgggctacctgcagcccagaaccttcctgctgaagtacaacgagaacggcaccatcaccgacgccgtggactgcgccctggaccccctgagcgagaccaagtgcaccctgaagagcttcaccgtggagaagggcatctaccagaccagcaacttcagagtgcagcccaccgagagcatcgtgagattccccaacatcaccaacctgtgccccttcgacgaggtgttcaacgccaccagattcgccagcgtgtacgcctggaacagaaagagaatcagcaactgcgtggccgactacagcgtgctgtacaacctggcccccttcttcaccttcaagtgctacggcgtgagccccaccaagctgaacgacctgtgcttcaccaacgtgtacgccgacagcttcgtgatcagaggcgacgaggtgagacagatcgcccccggccagaccggcaacatcgccgactacaactacaagctgcccgacgacttcaccggctgcgtgatcgcctggaacagcaacaagctggacagcaaggtgagcggcaactacaactacctgtacagactgttcagaaagagcaacctgaagcccttcgagagagacatcagcaccgagatctaccaggccggcaacaagccctgcaacggcgtggccggcttcaactgctacttccccctgagaagctacagcttcagacccacctacggcgtgggccaccagccctacagagtggtggtgctgagcttcgagctgctgcacgcccccgccaccgtgtgcggccccaagaagagcaccaacctggtgaagaacaagtgcgtgaacttcaacttcaacggcctgaagggcaccggcgtgctgaccgagagcaacaagaagttcctgcccttccagcagttcggcagagacatcgccgacaccaccgacgccgtgagagacccccagaccctggagatcctggacatcaccccctgcagcttcggcggcgtgagcgtgatcacccccggcaccaacaccagcaaccaggtggccgtgctgtaccagggcgtgaactgcaccgaggtgcccgtggccatccacgccgaccagctgacccccacctggagagtgtacagcaccggcagcaacgtgttccagaccagagccggctgcctgatcggcgccgagtacgtgaacaacagctacgagtgcgacatccccatcggcgccggcatctgcgccagctaccagacccagaccaagagccacagaagagccagaagcgtggccagccagagcatcatcgcctacaccatgagcctgggcgccgagaacagcgtggcctacagcaacaacagcatcgccatccccaccaacttcaccatcagcgtgaccaccgagatcctgcccgtgagcatgaccaagaccagcgtggactgcaccatgtacatctgcggcgacagcaccgagtgcagcaacctgctgctgcagtacggcagcttctgcacccagctgaagagagccctgaccggcatcgccgtggagcaggacaagaacacccaggaggtgttcgcccaggtgaagcagatctacaagaccccccccatcaagtacttcggcggcttcaacttcagccagatcctgcccgaccccagcaagcccagcaagagaagcttcatcgaggacctgctgttcaacaaggtgaccctggccgacgccggcttcatcaagcagtacggcgactgcctgggcgacatcgccgccagagacctgatctgcgcccagaagttcaagggcctgaccgtgctgccccccctgctgaccgacgagatgatcgcccagtacaccagcgccctgctggccggcaccatcaccagcggctggaccttcggcgccggcgccgccctgcagatccccttcgccatgcagatggcctacagattcaacggcatcggcgtgacccagaacgtgctgtacgagaaccagaagctgatcgccaaccagttcaacagcgccatcggcaagatccaggacagcctgagcagcaccgccagcgccctgggcaagctgcaggacgtggtgaaccacaacgcccaggccctgaacaccctggtgaagcagctgagcagcaagttcggcgccatcagcagcgtgctgaacgacatcttcagcagactggacaaggtggaggccgaggtgcagatcgacagactgatcaccggcagactgcagagcctgcagacctacgtgacccagcagctgatcagagccgccgagatcagagccagcgccaacctggccgccaccaagatgagcgagtgcgtgctgggccagagcaagagagtggacttctgcggcaagggctaccacctgatgagcttcccccagagcgccccccacggcgtggtgttcctgcacgtgacctacgtgcccgcccaggagaagaacttcaccaccgcccccgccatctgccacgacggcaaggcccacttccccagagagggcgtgttcgtgagcaacggcacccactggttcgtgacccagagaaacttctacgagccccagatcatcaccaccgacaacaccttcgtgagcggcaactgcgacgtggtgatcggcatcgtgaacaacaccgtgtacgaccccctgcagcccgagctggacagcttcaaggaggagctggacaagtacttcaagaaccacaccagccccgacgtggacctgggcgacatcagcggcatcaacgccagcgtggtgaacatccagaaggagatcgacagactgaacgaggtggccaagaacctgaacgagagcctgatcgacctgcaggagctgggcaagtacgagcagtacatcaagtggccctggtacatctggctgggcttcatcgccggcctgatcgccatcgtgatggtgaccatcatgctgtgctgcatgaccagctgctgcagctgcctgaagggctgctgcagctgcggcagctgctgcaagttcgacgaggacgacagcgagcccgtgctgaagggcgtgaagctgcactacacctag

SEQ ID NO: 60 - DNA, 3804 bp, synthetic construct
  source 1..3804: mol_type = other DNA
atgttcgtgttcctggtgctgctgcccctggtgtcctcccagtgcgtgaacctgaccacccgtacccagctgccccccgcttacaccaactccttcacccgtggtgtgtactaccccgacaaggtgttccgttcctccgtgctgcactccacccaggacctgttcctgcccttcttctccaacgtgacctggttccacgtgatctccggtaccaacggtaccaagcgtttcgacaaccccgtgctgcccttcaacgacggtgtgtacttcgcttccatcgagaagtccaacatcatccgtggttggatcttcggtaccaccctggactccaagacccagtccctgctgatcgtgaacaacgctaccaacgtggtgatcaaggtgtgcgagttccagttctgcaacgaccccttcctggaccacaagaacaacaagtcctggatggagtccgagttccgtgtgtactcctccgctaacaactgcaccttcgagtacgtgtcccagcccttcctgatggacctggagggtaagcagggtaacttcaagaacctgcgtgagttcgtgttcaagaacatcgacggttacttcaagatctactccaagcacacccccatcatcgtgcgtgacctgccccagggtttctccgctctggagcccctggtggacctgcccatcggtatcaacatcacccgtttccagaccctgctggctctgcaccgttcctacctgacccccggtgactcctcctccggttggaccgctggtgctgctgcttactacgtgggttacctgcagccccgtaccttcctgctgaagtacaacgagaacggtaccatcaccgacgctgtggactgcgctctggaccccctgtccgagaccaagtgcaccctgaagtccttcaccgtggagaagggtatctaccagacctccaacttccgtgtgcagcccaccgagtccatcgtgcgtttccccaacatcaccaacctgtgccccttcgacgaggtgttcaacgctacccgtttcgcttccgtgtacgcttggaaccgtaagcgtatctccaactgcgtggctgactactccgtgctgtacaacctggctcccttcttcaccttcaagtgctacggtgtgtcccccaccaagctgaacgacctgtgcttcaccaacgtgtacgctgactccttcgtgatccgtggtgacgaggtgcgtcagatcgctcccggtcagaccggtaacatcgctgactacaactacaagctgcccgacgacttcaccggttgcgtgatcgcttggaactccaacaagctggactccaaggtgtccggtaactacaactacctgtaccgtctgttccgtaagtccaacctgaagcccttcgagcgtgacatctccaccgagatctaccaggctggtaacaagccctgcaacggtgtggctggtttcaactgctacttccccctgcgttcctactccttccgtcccacctacggtgtgggtcaccagccctaccgtgtggtggtgctgtccttcgagctgctgcacgctcccgctaccgtgtgcggtcccaagaagtccaccaacctggtgaagaacaagtgcgtgaacttcaacttcaacggtctgaagggtaccggtgtgctgaccgagtccaacaagaagttcctgcccttccagcagttcggtcgtgacatcgctgacaccaccgacgctgtgcgtgacccccagaccctggagatcctggacatcaccccctgctccttcggtggtgtgtccgtgatcacccccggtaccaacacctccaaccaggtggctgtgctgtaccagggtgtgaactgcaccgaggtgcccgtggctatccacgctgaccagctgacccccacctggcgtgtgtactccaccggttccaacgtgttccagacccgtgctggttgcctgatcggtgctgagtacgtgaacaactcctacgagtgcgacatccccatcggtgctggtatctgcgcttcctaccagacccagaccaagtcccaccgtcgtgctcgttccgtggcttcccagtccatcatcgcttacaccatgtccctgggtgctgagaactccgtggcttactccaacaactccatcgctatccccaccaacttcaccatctccgtgaccaccgagatcctgcccgtgtccatgaccaagacctccgtggactgcaccatgtacatctgcggtgactccaccgagtgctccaacctgctgctgcagtacggttccttctgcacccagctgaagcgtgctctgaccggtatcgctgtggagcaggacaagaacacccaggaggtgttcgctcaggtgaagcagatctacaagaccccccccatcaagtacttcggtggtttcaacttctcccagatcctgcccgacccctccaagccctccaagcgttccttcatcgaggacctgctgttcaacaaggtgaccctggctgacgctggtttcatcaagcagtacggtgactgcctgggtgacatcgctgctcgtgacctgatctgcgctcagaagttcaagggtctgaccgtgctgccccccctgctgaccgacgagatgatcgctcagtacacctccgctctgctggctggtaccatcacctccggttggaccttcggtgctggtgctgctctgcagatccccttcgctatgcagatggcttaccgtttcaacggtatcggtgtgacccagaacgtgctgtacgagaaccagaagctgatcgctaaccagttcaactccgctatcggtaagatccaggactccctgtcctccaccgcttccgctctgggtaagctgcaggacgtggtgaaccacaacgctcaggctctgaacaccctggtgaagcagctgtcctccaagttcggtgctatctcctccgtgctgaacgacatcttctcccgtctggacaaggtggaggctgaggtgcagatcgaccgtctgatcaccggtcgtctgcagtccctgcagacctacgtgacccagcagctgatccgtgctgctgagatccgtgcttccgctaacctggctgctaccaagatgtccgagtgcgtgctgggtcagtccaagcgtgtggacttctgcggtaagggttaccacctgatgtccttcccccagtccgctccccacggtgtggtgttcctgcacgtgacctacgtgcccgctcaggagaagaacttcaccaccgctcccgctatctgccacgacggtaaggctcacttcccccgtgagggtgtgttcgtgtccaacggtacccactggttcgtgacccagcgtaacttctacgagccccagatcatcaccaccgacaacaccttcgtgtccggtaactgcgacgtggtgatcggtatcgtgaacaacaccgtgtacgaccccctgcagcccgagctggactccttcaaggaggagctggacaagtacttcaagaaccacacctcccccgacgtggacctgggtgacatctccggtatcaacgcttccgtggtgaacatccagaaggagatcgaccgtctgaacgaggtggctaagaacctgaacgagtccctgatcgacctgcaggagctgggtaagtacgagcagtacatcaagtggccctggtacatctggctgggtttcatcgctggtctgatcgctatcgtgatggtgaccatcatgctgtgctgcatgacctcctgctgctcctgcctgaagggttgctgctcctgcggttcctgctgcaagttcgacgaggacgactccgagcccgtgctgaagggtgtgaagctgcactacacctag

SEQ ID NO: 61 - protein, 1207 aa, synthetic construct
MFVFLVLLPLVSSQCVNLTTRTQLPPAYTNSFTRGVYYPDKVFRSSVLHSTQDLFLPFFSNVTWFHVISGTNGTKRFDNPVLPFNDGVYFASIEKSNIIRGWIFGTTLDSKTQSLLIVNNATNVVIKVCEFQFCNDPFLDHKNNKSWMESEFRVYSSANNCTFEYVSQPFLMDLEGKQGNFKNLREFVFKNIDGYFKIYSKHTPIIVRDLPQGFSALEPLVDLPIGINITRFQTLLALHRSYLTPGDSSSGWTAGAAAYYVGYLQPRTFLLKYNENGTITDAVDCALDPLSETKCTLKSFTVEKGIYQTSNFRVQPTESIVRFPNITNLCPFDEVFNATRFASVYAWNRKRISNCVADYSVLYNLAPFFTFKCYGVSPTKLNDLCFTNVYADSFVIRGDEVRQIAPGQTGNIADYNYKLPDDFTGCVIAWNSNKLDSKVSGNYNYLYRLFRKSNLKPFERDISTEIYQAGNKPCNGVAGFNCYFPLRSYSFRPTYGVGHQPYRVVVLSFELLHAPATVCGPKKSTNLVKNKCVNFNFNGLKGTGVLTESNKKFLPFQQFGRDIADTTDAVRDPQTLEILDITPCSFGGVSVITPGTNTSNQVAVLYQGVNCTEVPVAIHADQLTPTWRVYSTGSNVFQTRAGCLIGAEYVNNSYECDIPIGAGICASYQTQTKSHRRARSVASQSIIAYTMSLGAENSVAYSNNSIAIPTNFTISVTTEILPVSMTKTSVDCTMYICGDSTECSNLLLQYGSFCTQLKRALTGIAVEQDKNTQEVFAQVKQIYKTPPIKYFGGFNFSQILPDPSKPSKRSFIEDLLFNKVTLADAGFIKQYGDCLGDIAARDLICAQKFKGLTVLPPLLTDEMIAQYTSALLAGTITSGWTFGAGAALQIPFAMQMAYRFNGIGVTQNVLYENQKLIANQFNSAIGKIQDSLSSTASALGKLQDVVNHNAQALNTLVKQLSSKFGAISSVLNDIFSRLDKVEAEVQIDRLITGRLQSLQTYVTQQLIRAAEIRASANLAATKMSECVLGQSKRVDFCGKGYHLMSFPQSAPHGVVFLHVTYVPAQEKNFTTAPAICHDGKAHFPREGVFVSNGTHWFVTQRNFYEPQIITTDNTFVSGNCDVVIGIVNNTVYDPLQPELDSFKEELDKYFKNHTSPDVDLGDISGINASVVNIQKEIDRLNEVAKNLNESLIDLQELGKYEQYIKWP

SEQ ID NO: 62 - DNA, 3624 bp, synthetic construct
  source 1..3624: mol_type = other DNA
atgttcgtgttcctggtgctgctgcccctggtgagcagccagtgcgtgaacctgaccaccagaacccagctgccccccgcctacaccaacagcttcaccagaggcgtgtactaccccgacaaggtgttcagaagcagcgtgctgcacagcacccaggacctgttcctgcccttcttcagcaacgtgacctggttccacgtgatcagcggcaccaacggcaccaagagattcgacaaccccgtgctgcccttcaacgacggcgtgtacttcgccagcatcgagaagagcaacatcatcagaggctggatcttcggcaccaccctggacagcaagacccagagcctgctgatcgtgaacaacgccaccaacgtggtgatcaaggtgtgcgagttccagttctgcaacgaccccttcctggaccacaagaacaacaagagctggatggagagcgagttcagagtgtacagcagcgccaacaactgcaccttcgagtacgtgagccagcccttcctgatggacctggagggcaagcagggcaacttcaagaacctgagagagttcgtgttcaagaacatcgacggctacttcaagatctacagcaagcacacccccatcatcgtgagagacctgccccagggcttcagcgccctggagcccctggtggacctgcccatcggcatcaacatcaccagattccagaccctgctggccctgcacagaagctacctgacccccggcgacagcagcagcggctggaccgccggcgccgccgcctactacgtgggctacctgcagcccagaaccttcctgctgaagtacaacgagaacggcaccatcaccgacgccgtggactgcgccctggaccccctgagcgagaccaagtgcaccctgaagagcttcaccgtggagaagggcatctaccagaccagcaacttcagagtgcagcccaccgagagcatcgtgagattccccaacatcaccaacctgtgccccttcgacgaggtgttcaacgccaccagattcgccagcgtgtacgcctggaacagaaagagaatcagcaactgcgtggccgactacagcgtgctgtacaacctggcccccttcttcaccttcaagtgctacggcgtgagccccaccaagctgaacgacctgtgcttcaccaacgtgtacgccgacagcttcgtgatcagaggcgacgaggtgagacagatcgcccccggccagaccggcaacatcgccgactacaactacaagctgcccgacgacttcaccggctgcgtgatcgcctggaacagcaacaagctggacagcaaggtgagcggcaactacaactacctgtacagactgttcagaaagagcaacctgaagcccttcgagagagacatcagcaccgagatctaccaggccggcaacaagccctgcaacggcgtggccggcttcaactgctacttccccctgagaagctacagcttcagacccacctacggcgtgggccaccagccctacagagtggtggtgctgagcttcgagctgctgcacgcccccgccaccgtgtgcggccccaagaagagcaccaacctggtgaagaacaagtgcgtgaacttcaacttcaacggcctgaagggcaccggcgtgctgaccgagagcaacaagaagttcctgcccttccagcagttcggcagagacatcgccgacaccaccgacgccgtgagagacccccagaccctggagatcctggacatcaccccctgcagcttcggcggcgtgagcgtgatcacccccggcaccaacaccagcaaccaggtggccgtgctgtaccagggcgtgaactgcaccgaggtgcccgtggccatccacgccgaccagctgacccccacctggagagtgtacagcaccggcagcaacgtgttccagaccagagccggctgcctgatcggcgccgagtacgtgaacaacagctacgagtgcgacatccccatcggcgccggcatctgcgccagctaccagacccagaccaagagccacagaagagccagaagcgtggccagccagagcatcatcgcctacaccatgagcctgggcgccgagaacagcgtggcctacagcaacaacagcatcgccatccccaccaacttcaccatcagcgtgaccaccgagatcctgcccgtgagcatgaccaagaccagcgtggactgcaccatgtacatctgcggcgacagcaccgagtgcagcaacctgctgctgcagtacggcagcttctgcacccagctgaagagagccctgaccggcatcgccgtggagcaggacaagaacacccaggaggtgttcgcccaggtgaagcagatctacaagaccccccccatcaagtacttcggcggcttcaacttcagccagatcctgcccgaccccagcaagcccagcaagagaagcttcatcgaggacctgctgttcaacaaggtgaccctggccgacgccggcttcatcaagcagtacggcgactgcctgggcgacatcgccgccagagacctgatctgcgcccagaagttcaagggcctgaccgtgctgccccccctgctgaccgacgagatgatcgcccagtacaccagcgccctgctggccggcaccatcaccagcggctggaccttcggcgccggcgccgccctgcagatccccttcgccatgcagatggcctacagattcaacggcatcggcgtgacccagaacgtgctgtacgagaaccagaagctgatcgccaaccagttcaacagcgccatcggcaagatccaggacagcctgagcagcaccgccagcgccctgggcaagctgcaggacgtggtgaaccacaacgcccaggccctgaacaccctggtgaagcagctgagcagcaagttcggcgccatcagcagcgtgctgaacgacatcttcagcagactggacaaggtggaggccgaggtgcagatcgacagactgatcaccggcagactgcagagcctgcagacctacgtgacccagcagctgatcagagccgccgagatcagagccagcgccaacctggccgccaccaagatgagcgagtgcgtgctgggccagagcaagagagtggacttctgcggcaagggctaccacctgatgagcttcccccagagcgccccccacggcgtggtgttcctgcacgtgacctacgtgcccgcccaggagaagaacttcaccaccgcccccgccatctgccacgacggcaaggcccacttccccagagagggcgtgttcgtgagcaacggcacccactggttcgtgacccagagaaacttctacgagccccagatcatcaccaccgacaacaccttcgtgagcggcaactgcgacgtggtgatcggcatcgtgaacaacaccgtgtacgaccccctgcagcccgagctggacagcttcaaggaggagctggacaagtacttcaagaaccacaccagccccgacgtggacctgggcgacatcagcggcatcaacgccagcgtggtgaacatccagaaggagatcgacagactgaacgaggtggccaagaacctgaacgagagcctgatcgacctgcaggagctgggcaagtacgagcagtacatcaagtggccctag

SEQ ID NO: 63 - DNA, 3624 bp, synthetic construct
  source 1..3624: mol_type = other DNA
atgttcgtgttcctggtgctgctgcccctggtgtcctcccagtgcgtgaacctgaccacccgtacccagctgccccccgcttacaccaactccttcacccgtggtgtgtactaccccgacaaggtgttccgttcctccgtgctgcactccacccaggacctgttcctgcccttcttctccaacgtgacctggttccacgtgatctccggtaccaacggtaccaagcgtttcgacaaccccgtgctgcccttcaacgacggtgtgtacttcgcttccatcgagaagtccaacatcatccgtggttggatcttcggtaccaccctggactccaagacccagtccctgctgatcgtgaacaacgctaccaacgtggtgatcaaggtgtgcgagttccagttctgcaacgaccccttcctggaccacaagaacaacaagtcctggatggagtccgagttccgtgtgtactcctccgctaacaactgcaccttcgagtacgtgtcccagcccttcctgatggacctggagggtaagcagggtaacttcaagaacctgcgtgagttcgtgttcaagaacatcgacggttacttcaagatctactccaagcacacccccatcatcgtgcgtgacctgccccagggtttctccgctctggagcccctggtggacctgcccatcggtatcaacatcacccgtttccagaccctgctggctctgcaccgttcctacctgacccccggtgactcctcctccggttggaccgctggtgctgctgcttactacgtgggttacctgcagccccgtaccttcctgctgaagtacaacgagaacggtaccatcaccgacgctgtggactgcgctctggaccccctgtccgagaccaagtgcaccctgaagtccttcaccgtggagaagggtatctaccagacctccaacttccgtgtgcagcccaccgagtccatcgtgcgtttccccaacatcaccaacctgtgccccttcgacgaggtgttcaacgctacccgtttcgcttccgtgtacgcttggaaccgtaagcgtatctccaactgcgtggctgactactccgtgctgtacaacctggctcccttcttcaccttcaagtgctacggtgtgtcccccaccaagctgaacgacctgtgcttcaccaacgtgtacgctgactccttcgtgatccgtggtgacgaggtgcgtcagatcgctcccggtcagaccggtaacatcgctgactacaactacaagctgcccgacgacttcaccggttgcgtgatcgcttggaactccaacaagctggactccaaggtgtccggtaactacaactacctgtaccgtctgttccgtaagtccaacctgaagcccttcgagcgtgacatctccaccgagatctaccaggctggtaacaagccctgcaacggtgtggctggtttcaactgctacttccccctgcgttcctactccttccgtcccacctacggtgtgggtcaccagccctaccgtgtggtggtgctgtccttcgagctgctgcacgctcccgctaccgtgtgcggtcccaagaagtccaccaacctggtgaagaacaagtgcgtgaacttcaacttcaacggtctgaagggtaccggtgtgctgaccgagtccaacaagaagttcctgcccttccagcagttcggtcgtgacatcgctgacaccaccgacgctgtgcgtgacccccagaccctggagatcctggacatcaccccctgctccttcggtggtgtgtccgtgatcacccccggtaccaacacctccaaccaggtggctgtgctgtaccagggtgtgaactgcaccgaggtgcccgtggctatccacgctgaccagctgacccccacctggcgtgtgtactccaccggttccaacgtgttccagacccgtgctggttgcctgatcggtgctgagtacgtgaacaactcctacgagtgcgacatccccatcggtgctggtatctgcgcttcctaccagacccagaccaagtcccaccgtcgtgctcgttccgtggcttcccagtccatcatcgcttacaccatgtccctgggtgctgagaactccgtggcttactccaacaactccatcgctatccccaccaacttcaccatctccgtgaccaccgagatcctgcccgtgtccatgaccaagacctccgtggactgcaccatgtacatctgcggtgactccaccgagtgctccaacctgctgctgcagtacggttccttctgcacccagctgaagcgtgctctgaccggtatcgctgtggagcaggacaagaacacccaggaggtgttcgctcaggtgaagcagatctacaagaccccccccatcaagtacttcggtggtttcaacttctcccagatcctgcccgacccctccaagccctccaagcgttccttcatcgaggacctgctgttcaacaaggtgaccctggctgacgctggtttcatcaagcagtacggtgactgcctgggtgacatcgctgctcgtgacctgatctgcgctcagaagttcaagggtctgaccgtgctgccccccctgctgaccgacgagatgatcgctcagtacacctccgctctgctggctggtaccatcacctccggttggaccttcggtgctggtgctgctctgcagatccccttcgctatgcagatggcttaccgtttcaacggtatcggtgtgacccagaacgtgctgtacgagaaccagaagctgatcgctaaccagttcaactccgctatcggtaagatccaggactccctgtcctccaccgcttccgctctgggtaagctgcaggacgtggtgaaccacaacgctcaggctctgaacaccctggtgaagcagctgtcctccaagttcggtgctatctcctccgtgctgaacgacatcttctcccgtctggacaaggtggaggctgaggtgcagatcgaccgtctgatcaccggtcgtctgcagtccctgcagacctacgtgacccagcagctgatccgtgctgctgagatccgtgcttccgctaacctggctgctaccaagatgtccgagtgcgtgctgggtcagtccaagcgtgtggacttctgcggtaagggttaccacctgatgtccttcccccagtccgctccccacggtgtggtgttcctgcacgtgacctacgtgcccgctcaggagaagaacttcaccaccgctcccgctatctgccacgacggtaaggctcacttcccccgtgagggtgtgttcgtgtccaacggtacccactggttcgtgacccagcgtaacttctacgagccccagatcatcaccaccgacaacaccttcgtgtccggtaactgcgacgtggtgatcggtatcgtgaacaacaccgtgtacgaccccctgcagcccgagctggactccttcaaggaggagctggacaagtacttcaagaaccacacctcccccgacgtggacctgggtgacatctccggtatcaacgcttccgtggtgaacatccagaaggagatcgaccgtctgaacgaggtggctaagaacctgaacgagtccctgatcgacctgcaggagctgggtaagtacgagcagtacatcaagtggccctag

SEQ ID NO: 64 - protein, 1270 aa, synthetic construct
MFVFLVLLPLVSSQCVNLITRTQSYTNSFTRGVYYPDKVFRSSVLHSTQDLFLPFFSNVTWFHAIHVSGTNGTKRFDNPVLPFNDGVYFASTEKSNIIRGWIFGTTLDSKTQSLLIVNNATNVVIKVCEFQFCNDPFLDVYYHKNNKSWMESEFRVYSSANNCTFEYVSQPFLMDLEGKQGNFKNLREFVFKNIDGYFKIYSKHTPINLGRDLPQGFSALEPLVDLPIGINITRFQTLLALHRSYLTPGDSSSGWTAGAAAYYVGYLQPRTFLLKYNENGTITDAVDCALDPLSETKCTLKSFTVEKGIYQTSNFRVQPTESIVRFPNITNLCPFDEVFNATRFASVYAWNRKRISNCVADYSVLYNFAPFFAFKCYGVSPTKLNDLCFTNVYADSFVIRGNEVSQIAPGQTGNIADYNYKLPDDFTGCVIAWNSNKLDSKVGGNYNYLYRLFRKSNLKPFERDISTEIYQAGNKPCNGVAGFNCYFPLRSYGFRPTYGVGHQPYRVVVLSFELLHAPATVCGPKKSTNLVKNKCVNFNFNGLTGTGVLTESNKKFLPFQQFGRDIADTTDAVRDPQTLEILDITPCSFGGVSVITPGTNTSNQVAVLYQGVNCTEVPVAIHADQLTPTWRVYSTGSNVFQTRAGCLIGAEYVNNSYECDIPIGAGICASYQTQTKSHRRARSVASQSIIAYTMSLGAENSVAYSNNSIAIPTNFTISVTTEILPVSMTKTSVDCTMYICGDSTECSNLLLQYGSFCTQLKRALTGIAVEQDKNTQEVFAQVKQIYKTPPIKYFGGFNFSQILPDPSKPSKRSFIEDLLFNKVTLADAGFIKQYGDCLGDIAARDLICAQKFNGLTVLPPLLTDEMIAQYTSALLAGTITSGWTFGAGAALQIPFAMQMAYRFNGIGVTQNVLYENQKLIANQFNSAIGKIQDSLSSTASALGKLQDVVNHNAQALNTLVKQLSSKFGAISSVLNDILSRLDKVEAEVQIDRLITGRLQSLQTYVTQQLIRAAEIRASANLAATKMSECVLGQSKRVDFCGKGYHLMSFPQSAPHGVVFLHVTYVPAQEKNFTTAPAICHDGKAHFPREGVFVSNGTHWFVTQRNFYEPQIITTDNTFVSGNCDVVIGIVNNTVYDPLQPELDSFKEELDKYFKNHTSPDVDLGDISGINASVVNIQKEIDRLNEVAKNLNESLIDLQELGKYEQYIKWPWYIWLGFIAGLIAIVMVTIMLCCMTSCCSCLKGCCSCGSCCKFDEDDSEPVLKGVKLHYT

SEQ ID NO: 65 - DNA, 3813 bp, synthetic construct
  source 1..3813: mol_type = other DNA
atgttcgtgttcctggtgctgctgcccctggtgagcagccagtgcgtgaacctgatcaccagaacccagagctacaccaacagcttcaccagaggcgtgtactaccccgacaaggtgttcagaagcagcgtgctgcacagcacccaggacctgttcctgcccttcttcagcaacgtgacctggttccacgccatccacgtgagcggcaccaacggcaccaagagattcgacaaccccgtgctgcccttcaacgacggcgtgtacttcgccagcaccgagaagagcaacatcatcagaggctggatcttcggcaccaccctggacagcaagacccagagcctgctgatcgtgaacaacgccaccaacgtggtgatcaaggtgtgcgagttccagttctgcaacgaccccttcctggacgtgtactaccacaagaacaacaagagctggatggagagcgagttcagagtgtacagcagcgccaacaactgcaccttcgagtacgtgagccagcccttcctgatggacctggagggcaagcagggcaacttcaagaacctgagagagttcgtgttcaagaacatcgacggctacttcaagatctacagcaagcacacccccatcaacctgggcagagacctgccccagggcttcagcgccctggagcccctggtggacctgcccatcggcatcaacatcaccagattccagaccctgctggccctgcacagaagctacctgacccccggcgacagcagcagcggctggaccgccggcgccgccgcctactacgtgggctacctgcagcccagaaccttcctgctgaagtacaacgagaacggcaccatcaccgacgccgtggactgcgccctggaccccctgagcgagaccaagtgcaccctgaagagcttcaccgtggagaagggcatctaccagaccagcaacttcagagtgcagcccaccgagagcatcgtgagattccccaacatcaccaacctgtgccccttcgacgaggtgttcaacgccaccagattcgccagcgtgtacgcctggaacagaaagagaatcagcaactgcgtggccgactacagcgtgctgtacaacttcgcccccttcttcgccttcaagtgctacggcgtgagccccaccaagctgaacgacctgtgcttcaccaacgtgtacgccgacagcttcgtgatcagaggcaacgaggtgagccagatcgcccccggccagaccggcaacatcgccgactacaactacaagctgcccgacgacttcaccggctgcgtgatcgcctggaacagcaacaagctggacagcaaggtgggcggcaactacaactacctgtacagactgttcagaaagagcaacctgaagcccttcgagagagacatcagcaccgagatctaccaggccggcaacaagccctgcaacggcgtggccggcttcaactgctacttccccctgagaagctacggcttcagacccacctacggcgtgggccaccagccctacagagtggtggtgctgagcttcgagctgctgcacgcccccgccaccgtgtgcggccccaagaagagcaccaacctggtgaagaacaagtgcgtgaacttcaacttcaacggcctgaccggcaccggcgtgctgaccgagagcaacaagaagttcctgcccttccagcagttcggcagagacatcgccgacaccaccgacgccgtgagagacccccagaccctggagatcctggacatcaccccctgcagcttcggcggcgtgagcgtgatcacccccggcaccaacaccagcaaccaggtggccgtgctgtaccagggcgtgaactgcaccgaggtgcccgtggccatccacgccgaccagctgacccccacctggagagtgtacagcaccggcagcaacgtgttccagaccagagccggctgcctgatcggcgccgagtacgtgaacaacagctacgagtgcgacatccccatcggcgccggcatctgcgccagctaccagacccagaccaagagccacagaagagccagaagcgtggccagccagagcatcatcgcctacaccatgagcctgggcgccgagaacagcgtggcctacagcaacaacagcatcgccatccccaccaacttcaccatcagcgtgaccaccgagatcctgcccgtgagcatgaccaagaccagcgtggactgcaccatgtacatctgcggcgacagcaccgagtgcagcaacctgctgctgcagtacggcagcttctgcacccagctgaagagagccctgaccggcatcgccgtggagcaggacaagaacacccaggaggtgttcgcccaggtgaagcagatctacaagaccccccccatcaagtacttcggcggcttcaacttcagccagatcctgcccgaccccagcaagcccagcaagagaagcttcatcgaggacctgctgttcaacaaggtgaccctggccgacgccggcttcatcaagcagtacggcgactgcctgggcgacatcgccgccagagacctgatctgcgcccagaagttcaacggcctgaccgtgctgccccccctgctgaccgacgagatgatcgcccagtacaccagcgccctgctggccggcaccatcaccagcggctggaccttcggcgccggcgccgccctgcagatccccttcgccatgcagatggcctacagattcaacggcatcggcgtgacccagaacgtgctgtacgagaaccagaagctgatcgccaaccagttcaacagcgccatcggcaagatccaggacagcctgagcagcaccgccagcgccctgggcaagctgcaggacgtggtgaaccacaacgcccaggccctgaacaccctggtgaagcagctgagcagcaagttcggcgccatcagcagcgtgctgaacgacatcctgagcagactggacaaggtggaggccgaggtgcagatcgacagactgatcaccggcagactgcagagcctgcagacctacgtgacccagcagctgatcagagccgccgagatcagagccagcgccaacctggccgccaccaagatgagcgagtgcgtgctgggccagagcaagagagtggacttctgcggcaagggctaccacctgatgagcttcccccagagcgccccccacggcgtggtgttcctgcacgtgacctacgtgcccgcccaggagaagaacttcaccaccgcccccgccatctgccacgacggcaaggcccacttccccagagagggcgtgttcgtgagcaacggcacccactggttcgtgacccagagaaacttctacgagccccagatcatcaccaccgacaacaccttcgtgagcggcaactgcgacgtggtgatcggcatcgtgaacaacaccgtgtacgaccccctgcagcccgagctggacagcttcaaggaggagctggacaagtacttcaagaaccacaccagccccgacgtggacctgggcgacatcagcggcatcaacgccagcgtggtgaacatccagaaggagatcgacagactgaacgaggtggccaagaacctgaacgagagcctgatcgacctgcaggagctgggcaagtacgagcagtacatcaagtggccctggtacatctggctgggcttcatcgccggcctgatcgccatcgtgatggtgaccatcatgctgtgctgcatgaccagctgctgcagctgcctgaagggctgctgcagctgcggcagctgctgcaagttcgacgaggacgacagcgagcccgtgctgaagggcgtgaagctgcactacacctag

SEQ ID NO: 66 - DNA, 3813 bp, synthetic construct
  source 1..3813: mol_type = other DNA
atgttcgtgttcctggtgctgctgcccctggtgtcctcccagtgcgtgaacctgatcacccgtacccagtcctacaccaactccttcacccgtggtgtgtactaccccgacaaggtgttccgttcctccgtgctgcactccacccaggacctgttcctgcccttcttctccaacgtgacctggttccacgctatccacgtgtccggtaccaacggtaccaagcgtttcgacaaccccgtgctgcccttcaacgacggtgtgtacttcgcttccaccgagaagtccaacatcatccgtggttggatcttcggtaccaccctggactccaagacccagtccctgctgatcgtgaacaacgctaccaacgtggtgatcaaggtgtgcgagttccagttctgcaacgaccccttcctggacgtgtactaccacaagaacaacaagtcctggatggagtccgagttccgtgtgtactcctccgctaacaactgcaccttcgagtacgtgtcccagcccttcctgatggacctggagggtaagcagggtaacttcaagaacctgcgtgagttcgtgttcaagaacatcgacggttacttcaagatctactccaagcacacccccatcaacctgggtcgtgacctgccccagggtttctccgctctggagcccctggtggacctgcccatcggtatcaacatcacccgtttccagaccctgctggctctgcaccgttcctacctgacccccggtgactcctcctccggttggaccgctggtgctgctgcttactacgtgggttacctgcagccccgtaccttcctgctgaagtacaacgagaacggtaccatcaccgacgctgtggactgcgctctggaccccctgtccgagaccaagtgcaccctgaagtccttcaccgtggagaagggtatctaccagacctccaacttccgtgtgcagcccaccgagtccatcgtgcgtttccccaacatcaccaacctgtgccccttcgacgaggtgttcaacgctacccgtttcgcttccgtgtacgcttggaaccgtaagcgtatctccaactgcgtggctgactactccgtgctgtacaacttcgctcccttcttcgctttcaagtgctacggtgtgtcccccaccaagctgaacgacctgtgcttcaccaacgtgtacgctgactccttcgtgatccgtggtaacgaggtgtcccagatcgctcccggtcagaccggtaacatcgctgactacaactacaagctgcccgacgacttcaccggttgcgtgatcgcttggaactccaacaagctggactccaaggtgggtggtaactacaactacctgtaccgtctgttccgtaagtccaacctgaagcccttcgagcgtgacatctccaccgagatctaccaggctggtaacaagccctgcaacggtgtggctggtttcaactgctacttccccctgcgttcctacggtttccgtcccacctacggtgtgggtcaccagccctaccgtgtggtggtgctgtccttcgagctgctgcacgctcccgctaccgtgtgcggtcccaagaagtccaccaacctggtgaagaacaagtgcgtgaacttcaacttcaacggtctgaccggtaccggtgtgctgaccgagtccaacaagaagttcctgcccttccagcagttcggtcgtgacatcgctgacaccaccgacgctgtgcgtgacccccagaccctggagatcctggacatcaccccctgctccttcggtggtgtgtccgtgatcacccccggtaccaacacctccaaccaggtggctgtgctgtaccagggtgtgaactgcaccgaggtgcccgtggctatccacgctgaccagctgacccccacctggcgtgtgtactccaccggttccaacgtgttccagacccgtgctggttgcctgatcggtgctgagtacgtgaacaactcctacgagtgcgacatccccatcggtgctggtatctgcgcttcctaccagacccagaccaagtcccaccgtcgtgctcgttccgtggcttcccagtccatcatcgcttacaccatgtccctgggtgctgagaactccgtggcttactccaacaactccatcgctatccccaccaacttcaccatctccgtgaccaccgagatcctgcccgtgtccatgaccaagacctccgtggactgcaccatgtacatctgcggtgactccaccgagtgctccaacctgctgctgcagtacggttccttctgcacccagctgaagcgtgctctgaccggtatcgctgtggagcaggacaagaacacccaggaggtgttcgctcaggtgaagcagatctacaagaccccccccatcaagtacttcggtggtttcaacttctcccagatcctgcccgacccctccaagccctccaagcgttccttcatcgaggacctgctgttcaacaaggtgaccctggctgacgctggtttcatcaagcagtacggtgactgcctgggtgacatcgctgctcgtgacctgatctgcgctcagaagttcaacggtctgaccgtgctgccccccctgctgaccgacgagatgatcgctcagtacacctccgctctgctggctggtaccatcacctccggttggaccttcggtgctggtgctgctctgcagatccccttcgctatgcagatggcttaccgtttcaacggtatcggtgtgacccagaacgtgctgtacgagaaccagaagctgatcgctaaccagttcaactccgctatcggtaagatccaggactccctgtcctccaccgcttccgctctgggtaagctgcaggacgtggtgaaccacaacgctcaggctctgaacaccctggtgaagcagctgtcctccaagttcggtgctatctcctccgtgctgaacgacatcctgtcccgtctggacaaggtggaggctgaggtgcagatcgaccgtctgatcaccggtcgtctgcagtccctgcagacctacgtgacccagcagctgatccgtgctgctgagatccgtgcttccgctaacctggctgctaccaagatgtccgagtgcgtgctgggtcagtccaagcgtgtggacttctgcggtaagggttaccacctgatgtccttcccccagtccgctccccacggtgtggtgttcctgcacgtgacctacgtgcccgctcaggagaagaacttcaccaccgctcccgctatctgccacgacggtaaggctcacttcccccgtgagggtgtgttcgtgtccaacggtacccactggttcgtgacccagcgtaacttctacgagccccagatcatcaccaccgacaacaccttcgtgtccggtaactgcgacgtggtgatcggtatcgtgaacaacaccgtgtacgaccccctgcagcccgagctggactccttcaaggaggagctggacaagtacttcaagaaccacacctcccccgacgtggacctgggtgacatctccggtatcaacgcttccgtggtgaacatccagaaggagatcgaccgtctgaacgaggtggctaagaacctgaacgagtccctgatcgacctgcaggagctgggtaagtacgagcagtacatcaagtggccctggtacatctggctgggtttcatcgctggtctgatcgctatcgtgatggtgaccatcatgctgtgctgcatgacctcctgctgctcctgcctgaagggttgctgctcctgcggttcctgctgcaagttcgacgaggacgactccgagcccgtgctgaagggtgtgaagctgcactacacctag

SEQ ID NO: 67 - protein, 1210 aa, synthetic construct
MFVFLVLLPLVSSQCVNLITRTQSYTNSFTRGVYYPDKVFRSSVLHSTQDLFLPFFSNVTWFHAIHVSGTNGTKRFDNPVLPFNDGVYFASTEKSNIIRGWIFGTTLDSKTQSLLIVNNATNVVIKVCEFQFCNDPFLDVYYHKNNKSWMESEFRVYSSANNCTFEYVSQPFLMDLEGKQGNFKNLREFVFKNIDGYFKIYSKHTPINLGRDLPQGFSALEPLVDLPIGINITRFQTLLALHRSYLTPGDSSSGWTAGAAAYYVGYLQPRTFLLKYNENGTITDAVDCALDPLSETKCTLKSFTVEKGIYQTSNFRVQPTESIVRFPNITNLCPFDEVFNATRFASVYAWNRKRISNCVADYSVLYNFAPFFAFKCYGVSPTKLNDLCFTNVYADSFVIRGNEVSQIAPGQTGNIADYNYKLPDDFTGCVIAWNSNKLDSKVGGNYNYLYRLFRKSNLKPFERDISTEIYQAGNKPCNGVAGFNCYFPLRSYGFRPTYGVGHQPYRVVVLSFELLHAPATVCGPKKSTNLVKNKCVNFNFNGLTGTGVLTESNKKFLPFQQFGRDIADTTDAVRDPQTLEILDITPCSFGGVSVITPGTNTSNQVAVLYQGVNCTEVPVAIHADQLTPTWRVYSTGSNVFQTRAGCLIGAEYVNNSYECDIPIGAGICASYQTQTKSHRRARSVASQSIIAYTMSLGAENSVAYSNNSIAIPTNFTISVTTEILPVSMTKTSVDCTMYICGDSTECSNLLLQYGSFCTQLKRALTGIAVEQDKNTQEVFAQVKQIYKTPPIKYFGGFNFSQILPDPSKPSKRSFIEDLLFNKVTLADAGFIKQYGDCLGDIAARDLICAQKFNGLTVLPPLLTDEMIAQYTSALLAGTITSGWTFGAGAALQIPFAMQMAYRFNGIGVTQNVLYENQKLIANQFNSAIGKIQDSLSSTASALGKLQDVVNHNAQALNTLVKQLSSKFGAISSVLNDILSRLDKVEAEVQIDRLITGRLQSLQTYVTQQLIRAAEIRASANLAATKMSECVLGQSKRVDFCGKGYHLMSFPQSAPHGVVFLHVTYVPAQEKNFTTAPAICHDGKAHFPREGVFVSNGTHWFVTQRNFYEPQIITTDNTFVSGNCDVVIGIVNNTVYDPLQPELDSFKEELDKYFKNHTSPDVDLGDISGINASVVNIQKEIDRLNEVAKNLNESLIDLQELGKYEQYIKWP

SEQ ID NO: 68 - DNA, 3633 bp, synthetic construct
  source 1..3633: mol_type = other DNA
atgttcgtgttcctggtgctgctgcccctggtgagcagccagtgcgtgaacctgatcaccagaacccagagctacaccaacagcttcaccagaggcgtgtactaccccgacaaggtgttcagaagcagcgtgctgcacagcacccaggacctgttcctgcccttcttcagcaacgtgacctggttccacgccatccacgtgagcggcaccaacggcaccaagagattcgacaaccccgtgctgcccttcaacgacggcgtgtacttcgccagcaccgagaagagcaacatcatcagaggctggatcttcggcaccaccctggacagcaagacccagagcctgctgatcgtgaacaacgccaccaacgtggtgatcaaggtgtgcgagttccagttctgcaacgaccccttcctggacgtgtactaccacaagaacaacaagagctggatggagagcgagttcagagtgtacagcagcgccaacaactgcaccttcgagtacgtgagccagcccttcctgatggacctggagggcaagcagggcaacttcaagaacctgagagagttcgtgttcaagaacatcgacggctacttcaagatctacagcaagcacacccccatcaacctgggcagagacctgccccagggcttcagcgccctggagcccctggtggacctgcccatcggcatcaacatcaccagattccagaccctgctggccctgcacagaagctacctgacccccggcgacagcagcagcggctggaccgccggcgccgccgcctactacgtgggctacctgcagcccagaaccttcctgctgaagtacaacgagaacggcaccatcaccgacgccgtggactgcgccctggaccccctgagcgagaccaagtgcaccctgaagagcttcaccgtggagaagggcatctaccagaccagcaacttcagagtgcagcccaccgagagcatcgtgagattccccaacatcaccaacctgtgccccttcgacgaggtgttcaacgccaccagattcgccagcgtgtacgcctggaacagaaagagaatcagcaactgcgtggccgactacagcgtgctgtacaacttcgcccccttcttcgccttcaagtgctacggcgtgagccccaccaagctgaacgacctgtgcttcaccaacgtgtacgccgacagcttcgtgatcagaggcaacgaggtgagccagatcgcccccggccagaccggcaacatcgccgactacaactacaagctgcccgacgacttcaccggctgcgtgatcgcctggaacagcaacaagctggacagcaaggtgggcggcaactacaactacctgtacagactgttcagaaagagcaacctgaagcccttcgagagagacatcagcaccgagatctaccaggccggcaacaagccctgcaacggcgtggccggcttcaactgctacttccccctgagaagctacggcttcagacccacctacggcgtgggccaccagccctacagagtggtggtgctgagcttcgagctgctgcacgcccccgccaccgtgtgcggccccaagaagagcaccaacctggtgaagaacaagtgcgtgaacttcaacttcaacggcctgaccggcaccggcgtgctgaccgagagcaacaagaagttcctgcccttccagcagttcggcagagacatcgccgacaccaccgacgccgtgagagacccccagaccctggagatcctggacatcaccccctgcagcttcggcggcgtgagcgtgatcacccccggcaccaacaccagcaaccaggtggccgtgctgtaccagggcgtgaactgcaccgaggtgcccgtggccatccacgccgaccagctgacccccacctggagagtgtacagcaccggcagcaacgtgttccagaccagagccggctgcctgatcggcgccgagtacgtgaacaacagctacgagtgcgacatccccatcggcgccggcatctgcgccagctaccagacccagaccaagagccacagaagagccagaagcgtggccagccagagcatcatcgcctacaccatgagcctgggcgccgagaacagcgtggcctacagcaacaacagcatcgccatccccaccaacttcaccatcagcgtgaccaccgagatcctgcccgtgagcatgaccaagaccagcgtggactgcaccatgtacatctgcggcgacagcaccgagtgcagcaacctgctgctgcagtacggcagcttctgcacccagctgaagagagccctgaccggcatcgccgtggagcaggacaagaacacccaggaggtgttcgcccaggtgaagcagatctacaagaccccccccatcaagtacttcggcggcttcaacttcagccagatcctgcccgaccccagcaagcccagcaagagaagcttcatcgaggacctgctgttcaacaaggtgaccctggccgacgccggcttcatcaagcagtacggcgactgcctgggcgacatcgccgccagagacctgatctgcgcccagaagttcaacggcctgaccgtgctgccccccctgctgaccgacgagatgatcgcccagtacaccagcgccctgctggccggcaccatcaccagcggctggaccttcggcgccggcgccgccctgcagatccccttcgccatgcagatggcctacagattcaacggcatcggcgtgacccagaacgtgctgtacgagaaccagaagctgatcgccaaccagttcaacagcgccatcggcaagatccaggacagcctgagcagcaccgccagcgccctgggcaagctgcaggacgtggtgaaccacaacgcccaggccctgaacaccctggtgaagcagctgagcagcaagttcggcgccatcagcagcgtgctgaacgacatcctgagcagactggacaaggtggaggccgaggtgcagatcgacagactgatcaccggcagactgcagagcctgcagacctacgtgacccagcagctgatcagagccgccgagatcagagccagcgccaacctggccgccaccaagatgagcgagtgcgtgctgggccagagcaagagagtggacttctgcggcaagggctaccacctgatgagcttcccccagagcgccccccacggcgtggtgttcctgcacgtgacctacgtgcccgcccaggagaagaacttcaccaccgcccccgccatctgccacgacggcaaggcccacttccccagagagggcgtgttcgtgagcaacggcacccactggttcgtgacccagagaaacttctacgagccccagatcatcaccaccgacaacaccttcgtgagcggcaactgcgacgtggtgatcggcatcgtgaacaacaccgtgtacgaccccctgcagcccgagctggacagcttcaaggaggagctggacaagtacttcaagaaccacaccagccccgacgtggacctgggcgacatcagcggcatcaacgccagcgtggtgaacatccagaaggagatcgacagactgaacgaggtggccaagaacctgaacgagagcctgatcgacctgcaggagctgggcaagtacgagcagtacatcaagtggccctag

SEQ ID NO: 69 - DNA, 3633 bp, synthetic construct
  source 1..3633: mol_type = other DNA
atgttcgtgttcctggtgctgctgcccctggtgtcctcccagtgcgtgaacctgatcacccgtacccagtcctacaccaactccttcacccgtggtgtgtactaccccgacaaggtgttccgttcctccgtgctgcactccacccaggacctgttcctgcccttcttctccaacgtgacctggttccacgctatccacgtgtccggtaccaacggtaccaagcgtttcgacaaccccgtgctgcccttcaacgacggtgtgtacttcgcttccaccgagaagtccaacatcatccgtggttggatcttcggtaccaccctggactccaagacccagtccctgctgatcgtgaacaacgctaccaacgtggtgatcaaggtgtgcgagttccagttctgcaacgaccccttcctggacgtgtactaccacaagaacaacaagtcctggatggagtccgagttccgtgtgtactcctccgctaacaactgcaccttcgagtacgtgtcccagcccttcctgatggacctggagggtaagcagggtaacttcaagaacctgcgtgagttcgtgttcaagaacatcgacggttacttcaagatctactccaagcacacccccatcaacctgggtcgtgacctgccccagggtttctccgctctggagcccctggtggacctgcccatcggtatcaacatcacccgtttccagaccctgctggctctgcaccgttcctacctgacccccggtgactcctcctccggttggaccgctggtgctgctgcttactacgtgggttacctgcagccccgtaccttcctgctgaagtacaacgagaacggtaccatcaccgacgctgtggactgcgctctggaccccctgtccgagaccaagtgcaccctgaagtccttcaccgtggagaagggtatctaccagacctccaacttccgtgtgcagcccaccgagtccatcgtgcgtttccccaacatcaccaacctgtgccccttcgacgaggtgttcaacgctacccgtttcgcttccgtgtacgcttggaaccgtaagcgtatctccaactgcgtggctgactactccgtgctgtacaacttcgctcccttcttcgctttcaagtgctacggtgtgtcccccaccaagctgaacgacctgtgcttcaccaacgtgtacgctgactccttcgtgatccgtggtaacgaggtgtcccagatcgctcccggtcagaccggtaacatcgctgactacaactacaagctgcccgacgacttcaccggttgcgtgatcgcttggaactccaacaagctggactccaaggtgggtggtaactacaactacctgtaccgtctgttccgtaagtccaacctgaagcccttcgagcgtgacatctccaccgagatctaccaggctggtaacaagccctgcaacggtgtggctggtttcaactgctacttccccctgcgttcctacggtttccgtcccacctacggtgtgggtcaccagccctaccgtgtggtggtgctgtccttcgagctgctgcacgctcccgctaccgtgtgcggtcccaagaagtccaccaacctggtgaagaacaagtgcgtgaacttcaacttcaacggtctgaccggtaccggtgtgctgaccgagtccaacaagaagttcctgcccttccagcagttcggtcgtgacatcgctgacaccaccgacgctgtgcgtgacccccagaccctggagatcctggacatcaccccctgctccttcggtggtgtgtccgtgatcacccccggtaccaacacctccaaccaggtggctgtgctgtaccagggtgtgaactgcaccgaggtgcccgtggctatccacgctgaccagctgacccccacctggcgtgtgtactccaccggttccaacgtgttccagacccgtgctggttgcctgatcggtgctgagtacgtgaacaactcctacgagtgcgacatccccatcggtgctggtatctgcgcttcctaccagacccagaccaagtcccaccgtcgtgctcgttccgtggcttcccagtccatcatcgcttacaccatgtccctgggtgctgagaactccgtggcttactccaacaactccatcgctatccccaccaacttcaccatctccgtgaccaccgagatcctgcccgtgtccatgaccaagacctccgtggactgcaccatgtacatctgcggtgactccaccgagtgctccaacctgctgctgcagtacggttccttctgcacccagctgaagcgtgctctgaccggtatcgctgtggagcaggacaagaacacccaggaggtgttcgctcaggtgaagcagatctacaagaccccccccatcaagtacttcggtggtttcaacttctcccagatcctgcccgacccctccaagccctccaagcgttccttcatcgaggacctgctgttcaacaaggtgaccctggctgacgctggtttcatcaagcagtacggtgactgcctgggtgacatcgctgctcgtgacctgatctgcgctcagaagttcaacggtctgaccgtgctgccccccctgctgaccgacgagatgatcgctcagtacacctccgctctgctggctggtaccatcacctccggttggaccttcggtgctggtgctgctctgcagatccccttcgctatgcagatggcttaccgtttcaacggtatcggtgtgacccagaacgtgctgtacgagaaccagaagctgatcgctaaccagttcaactccgctatcggtaagatccaggactccctgtcctccaccgcttccgctctgggtaagctgcaggacgtggtgaaccacaacgctcaggctctgaacaccctggtgaagcagctgtcctccaagttcggtgctatctcctccgtgctgaacgacatcctgtcccgtctggacaaggtggaggctgaggtgcagatcgaccgtctgatcaccggtcgtctgcagtccctgcagacctacgtgacccagcagctgatccgtgctgctgagatccgtgcttccgctaacctggctgctaccaagatgtccgagtgcgtgctgggtcagtccaagcgtgtggacttctgcggtaagggttaccacctgatgtccttcccccagtccgctccccacggtgtggtgttcctgcacgtgacctacgtgcccgctcaggagaagaacttcaccaccgctcccgctatctgccacgacggtaaggctcacttcccccgtgagggtgtgttcgtgtccaacggtacccactggttcgtgacccagcgtaacttctacgagccccagatcatcaccaccgacaacaccttcgtgtccggtaactgcgacgtggtgatcggtatcgtgaacaacaccgtgtacgaccccctgcagcccgagctggactccttcaaggaggagctggacaagtacttcaagaaccacacctcccccgacgtggacctgggtgacatctccggtatcaacgcttccgtggtgaacatccagaaggagatcgaccgtctgaacgaggtggctaagaacctgaacgagtccctgatcgacctgcaggagctgggtaagtacgagcagtacatcaagtggccctag

SEQ ID NO: 70 - protein, 1268 aa, synthetic construct
MFVFLVLLPLVSSQCVNLITRTQSYTNSFTRGVYYPDKVFRSSVLHSTQDLFLPFFSNVTWFHAISGTNGTKRFDNPVLPFNDGVYFASTEKSNIIRGWIFGTTLDSKTQSLLIVNNATNVVIKVCEFQFCNDPFLDVYYHKNNKSWMESEFRVYSSANNCTFEYVSQPFLMDLEGKQGNFKNLREFVFKNIDGYFKIYSKHTPINLGRDLPQGFSALEPLVDLPIGINITRFQTLLALHRSYLTPGDSSSGWTAGAAAYYVGYLQPRTFLLKYNENGTITDAVDCALDPLSETKCTLKSFTVEKGIYQTSNFRVQPTESIVRFPNITNLCPFDEVFNATRFASVYAWNRKRISNCVADYSVLYNFAPFFAFKCYGVSPTKLNDLCFTNVYADSFVIRGNEVSQIAPGQTGNIADYNYKLPDDFTGCVIAWNSNKLDSKVGGNYNYRYRLFRKSNLKPFERDISTEIYQAGNKPCNGVAGVNCYFPLQSYGFRPTYGVGHQPYRVVVLSFELLHAPATVCGPKKSTNLVKNKCVNFNFNGLTGTGVLTESNKKFLPFQQFGRDIADTTDAVRDPQTLEILDITPCSFGGVSVITPGTNTSNQVAVLYQGVNCTEVPVAIHADQLTPTWRVYSTGSNVFQTRAGCLIGAEYVNNSYECDIPIGAGICASYQTQTKSHRRARSVASQSIIAYTMSLGAENSVAYSNNSIAIPTNFTISVTTEILPVSMTKTSVDCTMYICGDSTECSNLLLQYGSFCTQLKRALTGIAVEQDKNTQEVFAQVKQIYKTPPIKYFGGFNFSQILPDPSKPSKRSFIEDLLFNKVTLADAGFIKQYGDCLGDIAARDLICAQKFNGLTVLPPLLTDEMIAQYTSALLAGTITSGWTFGAGAALQIPFAMQMAYRFNGIGVTQNVLYENQKLIANQFNSAIGKIQDSLSSTASALGKLQDVVNHNAQALNTLVKQLSSKFGAISSVLNDILSRLDKVEAEVQIDRLITGRLQSLQTYVTQQLIRAAEIRASANLAATKMSECVLGQSKRVDFCGKGYHLMSFPQSAPHGVVFLHVTYVPAQEKNFTTAPAICHDGKAHFPREGVFVSNGTHWFVTQRNFYEPQIITTDNTFVSGNCDVVIGIVNNTVYDPLQPELDSFKEELDKYFKNHTSPDVDLGDISGINASVVNIQKEIDRLNEVAKNLNESLIDLQELGKYEQYIKWPWYIWLGFIAGLIAIVMVTIMLCCMTSCCSCLKGCCSCGSCCKFDEDDSEPVLKGVKLHYT

SEQ ID NO: 71 - DNA, 3807 bp, synthetic construct
  source 1..3807: mol_type = other DNA
atgttcgtgttcctggtgctgctgcccctggtgagcagccagtgcgtgaacctgatcaccagaacccagagctacaccaacagcttcaccagaggcgtgtactaccccgacaaggtgttcagaagcagcgtgctgcacagcacccaggacctgttcctgcccttcttcagcaacgtgacctggttccacgccatcagcggcaccaacggcaccaagagattcgacaaccccgtgctgcccttcaacgacggcgtgtacttcgccagcaccgagaagagcaacatcatcagaggctggatcttcggcaccaccctggacagcaagacccagagcctgctgatcgtgaacaacgccaccaacgtggtgatcaaggtgtgcgagttccagttctgcaacgaccccttcctggacgtgtactaccacaagaacaacaagagctggatggagagcgagttcagagtgtacagcagcgccaacaactgcaccttcgagtacgtgagccagcccttcctgatggacctggagggcaagcagggcaacttcaagaacctgagagagttcgtgttcaagaacatcgacggctacttcaagatctacagcaagcacacccccatcaacctgggcagagacctgccccagggcttcagcgccctggagcccctggtggacctgcccatcggcatcaacatcaccagattccagaccctgctggccctgcacagaagctacctgacccccggcgacagcagcagcggctggaccgccggcgccgccgcctactacgtgggctacctgcagcccagaaccttcctgctgaagtacaacgagaacggcaccatcaccgacgccgtggactgcgccctggaccccctgagcgagaccaagtgcaccctgaagagcttcaccgtggagaagggcatctaccagaccagcaacttcagagtgcagcccaccgagagcatcgtgagattccccaacatcaccaacctgtgccccttcgacgaggtgttcaacgccaccagattcgccagcgtgtacgcctggaacagaaagagaatcagcaactgcgtggccgactacagcgtgctgtacaacttcgcccccttcttcgccttcaagtgctacggcgtgagccccaccaagctgaacgacctgtgcttcaccaacgtgtacgccgacagcttcgtgatcagaggcaacgaggtgagccagatcgcccccggccagaccggcaacatcgccgactacaactacaagctgcccgacgacttcaccggctgcgtgatcgcctggaacagcaacaagctggacagcaaggtgggcggcaactacaactacagatacagactgttcagaaagagcaacctgaagcccttcgagagagacatcagcaccgagatctaccaggccggcaacaagccctgcaacggcgtggccggcgtgaactgctacttccccctgcagagctacggcttcagacccacctacggcgtgggccaccagccctacagagtggtggtgctgagcttcgagctgctgcacgcccccgccaccgtgtgcggccccaagaagagcaccaacctggtgaagaacaagtgcgtgaacttcaacttcaacggcctgaccggcaccggcgtgctgaccgagagcaacaagaagttcctgcccttccagcagttcggcagagacatcgccgacaccaccgacgccgtgagagacccccagaccctggagatcctggacatcaccccctgcagcttcggcggcgtgagcgtgatcacccccggcaccaacaccagcaaccaggtggccgtgctgtaccagggcgtgaactgcaccgaggtgcccgtggccatccacgccgaccagctgacccccacctggagagtgtacagcaccggcagcaacgtgttccagaccagagccggctgcctgatcggcgccgagtacgtgaacaacagctacgagtgcgacatccccatcggcgccggcatctgcgccagctaccagacccagaccaagagccacagaagagccagaagcgtggccagccagagcatcatcgcctacaccatgagcctgggcgccgagaacagcgtggcctacagcaacaacagcatcgccatccccaccaacttcaccatcagcgtgaccaccgagatcctgcccgtgagcatgaccaagaccagcgtggactgcaccatgtacatctgcggcgacagcaccgagtgcagcaacctgctgctgcagtacggcagcttctgcacccagctgaagagagccctgaccggcatcgccgtggagcaggacaagaacacccaggaggtgttcgcccaggtgaagcagatctacaagaccccccccatcaagtacttcggcggcttcaacttcagccagatcctgcccgaccccagcaagcccagcaagagaagcttcatcgaggacctgctgttcaacaaggtgaccctggccgacgccggcttcatcaagcagtacggcgactgcctgggcgacatcgccgccagagacctgatctgcgcccagaagttcaacggcctgaccgtgctgccccccctgctgaccgacgagatgatcgcccagtacaccagcgccctgctggccggcaccatcaccagcggctggaccttcggcgccggcgccgccctgcagatccccttcgccatgcagatggcctacagattcaacggcatcggcgtgacccagaacgtgctgtacgagaaccagaagctgatcgccaaccagttcaacagcgccatcggcaagatccaggacagcctgagcagcaccgccagcgccctgggcaagctgcaggacgtggtgaaccacaacgcccaggccctgaacaccctggtgaagcagctgagcagcaagttcggcgccatcagcagcgtgctgaacgacatcctgagcagactggacaaggtggaggccgaggtgcagatcgacagactgatcaccggcagactgcagagcctgcagacctacgtgacccagcagctgatcagagccgccgagatcagagccagcgccaacctggccgccaccaagatgagcgagtgcgtgctgggccagagcaagagagtggacttctgcggcaagggctaccacctgatgagcttcccccagagcgccccccacggcgtggtgttcctgcacgtgacctacgtgcccgcccaggagaagaacttcaccaccgcccccgccatctgccacgacggcaaggcccacttccccagagagggcgtgttcgtgagcaacggcacccactggttcgtgacccagagaaacttctacgagccccagatcatcaccaccgacaacaccttcgtgagcggcaactgcgacgtggtgatcggcatcgtgaacaacaccgtgtacgaccccctgcagcccgagctggacagcttcaaggaggagctggacaagtacttcaagaaccacaccagccccgacgtggacctgggcgacatcagcggcatcaacgccagcgtggtgaacatccagaaggagatcgacagactgaacgaggtggccaagaacctgaacgagagcctgatcgacctgcaggagctgggcaagtacgagcagtacatcaagtggccctggtacatctggctgggcttcatcgccggcctgatcgccatcgtgatggtgaccatcatgctgtgctgcatgaccagctgctgcagctgcctgaagggctgctgcagctgcggcagctgctgcaagttcgacgaggacgacagcgagcccgtgctgaagggcgtgaagctgcactacacctag

SEQ ID NO: 72 - DNA, 3807 bp, synthetic construct
  source 1..3807: mol_type = other DNA
atgttcgtgttcctggtgctgctgcccctggtgtcctcccagtgcgtgaacctgatcacccgtacccagtcctacaccaactccttcacccgtggtgtgtactaccccgacaaggtgttccgttcctccgtgctgcactccacccaggacctgttcctgcccttcttctccaacgtgacctggttccacgctatctccggtaccaacggtaccaagcgtttcgacaaccccgtgctgcccttcaacgacggtgtgtacttcgcttccaccgagaagtccaacatcatccgtggttggatcttcggtaccaccctggactccaagacccagtccctgctgatcgtgaacaacgctaccaacgtggtgatcaaggtgtgcgagttccagttctgcaacgaccccttcctggacgtgtactaccacaagaacaacaagtcctggatggagtccgagttccgtgtgtactcctccgctaacaactgcaccttcgagtacgtgtcccagcccttcctgatggacctggagggtaagcagggtaacttcaagaacctgcgtgagttcgtgttcaagaacatcgacggttacttcaagatctactccaagcacacccccatcaacctgggtcgtgacctgccccagggtttctccgctctggagcccctggtggacctgcccatcggtatcaacatcacccgtttccagaccctgctggctctgcaccgttcctacctgacccccggtgactcctcctccggttggaccgctggtgctgctgcttactacgtgggttacctgcagccccgtaccttcctgctgaagtacaacgagaacggtaccatcaccgacgctgtggactgcgctctggaccccctgtccgagaccaagtgcaccctgaagtccttcaccgtggagaagggtatctaccagacctccaacttccgtgtgcagcccaccgagtccatcgtgcgtttccccaacatcaccaacctgtgccccttcgacgaggtgttcaacgctacccgtttcgcttccgtgtacgcttggaaccgtaagcgtatctccaactgcgtggctgactactccgtgctgtacaacttcgctcccttcttcgctttcaagtgctacggtgtgtcccccaccaagctgaacgacctgtgcttcaccaacgtgtacgctgactccttcgtgatccgtggtaacgaggtgtcccagatcgctcccggtcagaccggtaacatcgctgactacaactacaagctgcccgacgacttcaccggttgcgtgatcgcttggaactccaacaagctggactccaaggtgggtggtaactacaactaccgttaccgtctgttccgtaagtccaacctgaagcccttcgagcgtgacatctccaccgagatctaccaggctggtaacaagccctgcaacggtgtggctggtgtgaactgctacttccccctgcagtcctacggtttccgtcccacctacggtgtgggtcaccagccctaccgtgtggtggtgctgtccttcgagctgctgcacgctcccgctaccgtgtgcggtcccaagaagtccaccaacctggtgaagaacaagtgcgtgaacttcaacttcaacggtctgaccggtaccggtgtgctgaccgagtccaacaagaagttcctgcccttccagcagttcggtcgtgacatcgctgacaccaccgacgctgtgcgtgacccccagaccctggagatcctggacatcaccccctgctccttcggtggtgtgtccgtgatcacccccggtaccaacacctccaaccaggtggctgtgctgtaccagggtgtgaactgcaccgaggtgcccgtggctatccacgctgaccagctgacccccacctggcgtgtgtactccaccggttccaacgtgttccagacccgtgctggttgcctgatcggtgctgagtacgtgaacaactcctacgagtgcgacatccccatcggtgctggtatctgcgcttcctaccagacccagaccaagtcccaccgtcgtgctcgttccgtggcttcccagtccatcatcgcttacaccatgtccctgggtgctgagaactccgtggcttactccaacaactccatcgctatccccaccaacttcaccatctccgtgaccaccgagatcctgcccgtgtccatgaccaagacctccgtggactgcaccatgtacatctgcggtgactccaccgagtgctccaacctgctgctgcagtacggttccttctgcacccagctgaagcgtgctctgaccggtatcgctgtggagcaggacaagaacacccaggaggtgttcgctcaggtgaagcagatctacaagaccccccccatcaagtacttcggtggtttcaacttctcccagatcctgcccgacccctccaagccctccaagcgttccttcatcgaggacctgctgttcaacaaggtgaccctggctgacgctggtttcatcaagcagtacggtgactgcctgggtgacatcgctgctcgtgacctgatctgcgctcagaagttcaacggtctgaccgtgctgccccccctgctgaccgacgagatgatcgctcagtacacctccgctctgctggctggtaccatcacctccggttggaccttcggtgctggtgctgctctgcagatccccttcgctatgcagatggcttaccgtttcaacggtatcggtgtgacccagaacgtgctgtacgagaaccagaagctgatcgctaaccagttcaactccgctatcggtaagatccaggactccctgtcctccaccgcttccgctctgggtaagctgcaggacgtggtgaaccacaacgctcaggctctgaacaccctggtgaagcagctgtcctccaagttcggtgctatctcctccgtgctgaacgacatcctgtcccgtctggacaaggtggaggctgaggtgcagatcgaccgtctgatcaccggtcgtctgcagtccctgcagacctacgtgacccagcagctgatccgtgctgctgagatccgtgcttccgctaacctggctgctaccaagatgtccgagtgcgtgctgggtcagtccaagcgtgtggacttctgcggtaagggttaccacctgatgtccttcccccagtccgctccccacggtgtggtgttcctgcacgtgacctacgtgcccgctcaggagaagaacttcaccaccgctcccgctatctgccacgacggtaaggctcacttcccccgtgagggtgtgttcgtgtccaacggtacccactggttcgtgacccagcgtaacttctacgagccccagatcatcaccaccgacaacaccttcgtgtccggtaactgcgacgtggtgatcggtatcgtgaacaacaccgtgtacgaccccctgcagcccgagctggactccttcaaggaggagctggacaagtacttcaagaaccacacctcccccgacgtggacctgggtgacatctccggtatcaacgcttccgtggtgaacatccagaaggagatcgaccgtctgaacgaggtggctaagaacctgaacgagtccctgatcgacctgcaggagctgggtaagtacgagcagtacatcaagtggccctggtacatctggctgggtttcatcgctggtctgatcgctatcgtgatggtgaccatcatgctgtgctgcatgacctcctgctgctcctgcctgaagggttgctgctcctgcggttcctgctgcaagttcgacgaggacgactccgagcccgtgctgaagggtgtgaagctgcactacacctag

SEQ ID NO: 73 - protein, 1208 aa, synthetic construct
MFVFLVLLPLVSSQCVNLITRTQSYTNSFTRGVYYPDKVFRSSVLHSTQDLFLPFFSNVTWFHAISGTNGTKRFDNPVLPFNDGVYFASTEKSNIIRGWIFGTTLDSKTQSLLIVNNATNVVIKVCEFQFCNDPFLDVYYHKNNKSWMESEFRVYSSANNCTFEYVSQPFLMDLEGKQGNFKNLREFVFKNIDGYFKIYSKHTPINLGRDLPQGFSALEPLVDLPIGINITRFQTLLALHRSYLTPGDSSSGWTAGAAAYYVGYLQPRTFLLKYNENGTITDAVDCALDPLSETKCTLKSFTVEKGIYQTSNFRVQPTESIVRFPNITNLCPFDEVFNATRFASVYAWNRKRISNCVADYSVLYNFAPFFAFKCYGVSPTKLNDLCFTNVYADSFVIRGNEVSQIAPGQTGNIADYNYKLPDDFTGCVIAWNSNKLDSKVGGNYNYRYRLFRKSNLKPFERDISTEIYQAGNKPCNGVAGVNCYFPLQSYGFRPTYGVGHQPYRVVVLSFELLHAPATVCGPKKSTNLVKNKCVNFNFNGLTGTGVLTESNKKFLPFQQFGRDIADTTDAVRDPQTLEILDITPCSFGGVSVITPGTNTSNQVAVLYQGVNCTEVPVAIHADQLTPTWRVYSTGSNVFQTRAGCLIGAEYVNNSYECDIPIGAGICASYQTQTKSHRRARSVASQSIIAYTMSLGAENSVAYSNNSIAIPTNFTISVTTEILPVSMTKTSVDCTMYICGDSTECSNLLLQYGSFCTQLKRALTGIAVEQDKNTQEVFAQVKQIYKTPPIKYFGGFNFSQILPDPSKPSKRSFIEDLLFNKVTLADAGFIKQYGDCLGDIAARDLICAQKFNGLTVLPPLLTDEMIAQYTSALLAGTITSGWTFGAGAALQIPFAMQMAYRFNGIGVTQNVLYENQKLIANQFNSAIGKIQDSLSSTASALGKLQDVVNHNAQALNTLVKQLSSKFGAISSVLNDILSRLDKVEAEVQIDRLITGRLQSLQTYVTQQLIRAAEIRASANLAATKMSECVLGQSKRVDFCGKGYHLMSFPQSAPHGVVFLHVTYVPAQEKNFTTAPAICHDGKAHFPREGVFVSNGTHWFVTQRNFYEPQIITTDNTFVSGNCDVVIGIVNNTVYDPLQPELDSFKEELDKYFKNHTSPDVDLGDISGINASVVNIQKEIDRLNEVAKNLNESLIDLQELGKYEQYIKWP

SEQ ID NO: 74 - DNA, 3627 bp, synthetic construct
  source 1..3627: mol_type = other DNA
atgttcgtgttcctggtgctgctgcccctggtgagcagccagtgcgtgaacctgatcaccagaacccagagctacaccaacagcttcaccagaggcgtgtactaccccgacaaggtgttcagaagcagcgtgctgcacagcacccaggacctgttcctgcccttcttcagcaacgtgacctggttccacgccatcagcggcaccaacggcaccaagagattcgacaaccccgtgctgcccttcaacgacggcgtgtacttcgccagcaccgagaagagcaacatcatcagaggctggatcttcggcaccaccctggacagcaagacccagagcctgctgatcgtgaacaacgccaccaacgtggtgatcaaggtgtgcgagttccagttctgcaacgaccccttcctggacgtgtactaccacaagaacaacaagagctggatggagagcgagttcagagtgtacagcagcgccaacaactgcaccttcgagtacgtgagccagcccttcctgatggacctggagggcaagcagggcaacttcaagaacctgagagagttcgtgttcaagaacatcgacggctacttcaagatctacagcaagcacacccccatcaacctgggcagagacctgccccagggcttcagcgccctggagcccctggtggacctgcccatcggcatcaacatcaccagattccagaccctgctggccctgcacagaagctacctgacccccggcgacagcagcagcggctggaccgccggcgccgccgcctactacgtgggctacctgcagcccagaaccttcctgctgaagtacaacgagaacggcaccatcaccgacgccgtggactgcgccctggaccccctgagcgagaccaagtgcaccctgaagagcttcaccgtggagaagggcatctaccagaccagcaacttcagagtgcagcccaccgagagcatcgtgagattccccaacatcaccaacctgtgccccttcgacgaggtgttcaacgccaccagattcgccagcgtgtacgcctggaacagaaagagaatcagcaactgcgtggccgactacagcgtgctgtacaacttcgcccccttcttcgccttcaagtgctacggcgtgagccccaccaagctgaacgacctgtgcttcaccaacgtgtacgccgacagcttcgtgatcagaggcaacgaggtgagccagatcgcccccggccagaccggcaacatcgccgactacaactacaagctgcccgacgacttcaccggctgcgtgatcgcctggaacagcaacaagctggacagcaaggtgggcggcaactacaactacagatacagactgttcagaaagagcaacctgaagcccttcgagagagacatcagcaccgagatctaccaggccggcaacaagccctgcaacggcgtggccggcgtgaactgctacttccccctgcagagctacggcttcagacccacctacggcgtgggccaccagccctacagagtggtggtgctgagcttcgagctgctgcacgcccccgccaccgtgtgcggccccaagaagagcaccaacctggtgaagaacaagtgcgtgaacttcaacttcaacggcctgaccggcaccggcgtgctgaccgagagcaacaagaagttcctgcccttccagcagttcggcagagacatcgccgacaccaccgacgccgtgagagacccccagaccctggagatcctggacatcaccccctgcagcttcggcggcgtgagcgtgatcacccccggcaccaacaccagcaaccaggtggccgtgctgtaccagggcgtgaactgcaccgaggtgcccgtggccatccacgccgaccagctgacccccacctggagagtgtacagcaccggcagcaacgtgttccagaccagagccggctgcctgatcggcgccgagtacgtgaacaacagctacgagtgcgacatccccatcggcgccggcatctgcgccagctaccagacccagaccaagagccacagaagagccagaagcgtggccagccagagcatcatcgcctacaccatgagcctgggcgccgagaacagcgtggcctacagcaacaacagcatcgccatccccaccaacttcaccatcagcgtgaccaccgagatcctgcccgtgagcatgaccaagaccagcgtggactgcaccatgtacatctgcggcgacagcaccgagtgcagcaacctgctgctgcagtacggcagcttctgcacccagctgaagagagccctgaccggcatcgccgtggagcaggacaagaacacccaggaggtgttcgcccaggtgaagcagatctacaagaccccccccatcaagtacttcggcggcttcaacttcagccagatcctgcccgaccccagcaagcccagcaagagaagcttcatcgaggacctgctgttcaacaaggtgaccctggccgacgccggcttcatcaagcagtacggcgactgcctgggcgacatcgccgccagagacctgatctgcgcccagaagttcaacggcctgaccgtgctgccccccctgctgaccgacgagatgatcgcccagtacaccagcgccctgctggccggcaccatcaccagcggctggaccttcggcgccggcgccgccctgcagatccccttcgccatgcagatggcctacagattcaacggcatcggcgtgacccagaacgtgctgtacgagaaccagaagctgatcgccaaccagttcaacagcgccatcggcaagatccaggacagcctgagcagcaccgccagcgccctgggcaagctgcaggacgtggtgaaccacaacgcccaggccctgaacaccctggtgaagcagctgagcagcaagttcggcgccatcagcagcgtgctgaacgacatcctgagcagactggacaaggtggaggccgaggtgcagatcgacagactgatcaccggcagactgcagagcctgcagacctacgtgacccagcagctgatcagagccgccgagatcagagccagcgccaacctggccgccaccaagatgagcgagtgcgtgctgggccagagcaagagagtggacttctgcggcaagggctaccacctgatgagcttcccccagagcgccccccacggcgtggtgttcctgcacgtgacctacgtgcccgcccaggagaagaacttcaccaccgcccccgccatctgccacgacggcaaggcccacttccccagagagggcgtgttcgtgagcaacggcacccactggttcgtgacccagagaaacttctacgagccccagatcatcaccaccgacaacaccttcgtgagcggcaactgcgacgtggtgatcggcatcgtgaacaacaccgtgtacgaccccctgcagcccgagctggacagcttcaaggaggagctggacaagtacttcaagaaccacaccagccccgacgtggacctgggcgacatcagcggcatcaacgccagcgtggtgaacatccagaaggagatcgacagactgaacgaggtggccaagaacctgaacgagagcctgatcgacctgcaggagctgggcaagtacgagcagtacatcaagtggccctag

SEQ ID NO: 75 - DNA, 3627 bp, synthetic construct
  source 1..3627: mol_type = other DNA
atgttcgtgttcctggtgctgctgcccctggtgtcctcccagtgcgtgaacctgatcacccgtacccagtcctacaccaactccttcacccgtggtgtgtactaccccgacaaggtgttccgttcctccgtgctgcactccacccaggacctgttcctgcccttcttctccaacgtgacctggttccacgctatctccggtaccaacggtaccaagcgtttcgacaaccccgtgctgcccttcaacgacggtgtgtacttcgcttccaccgagaagtccaacatcatccgtggttggatcttcggtaccaccctggactccaagacccagtccctgctgatcgtgaacaacgctaccaacgtggtgatcaaggtgtgcgagttccagttctgcaacgaccccttcctggacgtgtactaccacaagaacaacaagtcctggatggagtccgagttccgtgtgtactcctccgctaacaactgcaccttcgagtacgtgtcccagcccttcctgatggacctggagggtaagcagggtaacttcaagaacctgcgtgagttcgtgttcaagaacatcgacggttacttcaagatctactccaagcacacccccatcaacctgggtcgtgacctgccccagggtttctccgctctggagcccctggtggacctgcccatcggtatcaacatcacccgtttccagaccctgctggctctgcaccgttcctacctgacccccggtgactcctcctccggttggaccgctggtgctgctgcttactacgtgggttacctgcagccccgtaccttcctgctgaagtacaacgagaacggtaccatcaccgacgctgtggactgcgctctggaccccctgtccgagaccaagtgcaccctgaagtccttcaccgtggagaagggtatctaccagacctccaacttccgtgtgcagcccaccgagtccatcgtgcgtttccccaacatcaccaacctgtgccccttcgacgaggtgttcaacgctacccgtttcgcttccgtgtacgcttggaaccgtaagcgtatctccaactgcgtggctgactactccgtgctgtacaacttcgctcccttcttcgctttcaagtgctacggtgtgtcccccaccaagctgaacgacctgtgcttcaccaacgtgtacgctgactccttcgtgatccgtggtaacgaggtgtcccagatcgctcccggtcagaccggtaacatcgctgactacaactacaagctgcccgacgacttcaccggttgcgtgatcgcttggaactccaacaagctggactccaaggtgggtggtaactacaactaccgttaccgtctgttccgtaagtccaacctgaagcccttcgagcgtgacatctccaccgagatctaccaggctggtaacaagccctgcaacggtgtggctggtgtgaactgctacttccccctgcagtcctacggtttccgtcccacctacggtgtgggtcaccagccctaccgtgtggtggtgctgtccttcgagctgctgcacgctcccgctaccgtgtgcggtcccaagaagtccaccaacctggtgaagaacaagtgcgtgaacttcaacttcaacggtctgaccggtaccggtgtgctgaccgagtccaacaagaagttcctgcccttccagcagttcggtcgtgacatcgctgacaccaccgacgctgtgcgtgacccccagaccctggagatcctggacatcaccccctgctccttcggtggtgtgtccgtgatcacccccggtaccaacacctccaaccaggtggctgtgctgtaccagggtgtgaactgcaccgaggtgcccgtggctatccacgctgaccagctgacccccacctggcgtgtgtactccaccggttccaacgtgttccagacccgtgctggttgcctgatcggtgctgagtacgtgaacaactcctacgagtgcgacatccccatcggtgctggtatctgcgcttcctaccagacccagaccaagtcccaccgtcgtgctcgttccgtggcttcccagtccatcatcgcttacaccatgtccctgggtgctgagaactccgtggcttactccaacaactccatcgctatccccaccaacttcaccatctccgtgaccaccgagatcctgcccgtgtccatgaccaagacctccgtggactgcaccatgtacatctgcggtgactccaccgagtgctccaacctgctgctgcagtacggttccttctgcacccagctgaagcgtgctctgaccggtatcgctgtggagcaggacaagaacacccaggaggtgttcgctcaggtgaagcagatctacaagaccccccccatcaagtacttcggtggtttcaacttctcccagatcctgcccgacccctccaagccctccaagcgttccttcatcgaggacctgctgttcaacaaggtgaccctggctgacgctggtttcatcaagcagtacggtgactgcctgggtgacatcgctgctcgtgacctgatctgcgctcagaagttcaacggtctgaccgtgctgccccccctgctgaccgacgagatgatcgctcagtacacctccgctctgctggctggtaccatcacctccggttggaccttcggtgctggtgctgctctgcagatccccttcgctatgcagatggcttaccgtttcaacggtatcggtgtgacccagaacgtgctgtacgagaaccagaagctgatcgctaaccagttcaactccgctatcggtaagatccaggactccctgtcctccaccgcttccgctctgggtaagctgcaggacgtggtgaaccacaacgctcaggctctgaacaccctggtgaagcagctgtcctccaagttcggtgctatctcctccgtgctgaacgacatcctgtcccgtctggacaaggtggaggctgaggtgcagatcgaccgtctgatcaccggtcgtctgcagtccctgcagacctacgtgacccagcagctgatccgtgctgctgagatccgtgcttccgctaacctggctgctaccaagatgtccgagtgcgtgctgggtcagtccaagcgtgtggacttctgcggtaagggttaccacctgatgtccttcccccagtccgctccccacggtgtggtgttcctgcacgtgacctacgtgcccgctcaggagaagaacttcaccaccgctcccgctatctgccacgacggtaaggctcacttcccccgtgagggtgtgttcgtgtccaacggtacccactggttcgtgacccagcgtaacttctacgagccccagatcatcaccaccgacaacaccttcgtgtccggtaactgcgacgtggtgatcggtatcgtgaacaacaccgtgtacgaccccctgcagcccgagctggactccttcaaggaggagctggacaagtacttcaagaaccacacctcccccgacgtggacctgggtgacatctccggtatcaacgcttccgtggtgaacatccagaaggagatcgaccgtctgaacgaggtggctaagaacctgaacgagtccctgatcgacctgcaggagctgggtaagtacgagcagtacatcaagtggccctag

SEQ ID NO: 76 - DNA, 3807 bp, synthetic construct
  source 1..3807: mol_type = other DNA
atgttcgtgttcctggtgctgctgcccctggtgagcagccaatgcgtgaacctgatcacaagaacacagagctacaccaacagcttcacaagaggcgtgtactaccccgacaaggtgttcagaagcagcgtgctgcacagcacccaagacctgtttctccccttcttcagcaacgtgacctggttccacgccatcagcggcaccaacggcaccaagagattcgacaaccccgtgctgcccttcaacgacggcgtgtacttcgctagcaccgagaagagcaacatcatcagaggctggatcttcggcaccaccctggacagcaagacacagagcctgctgatcgtgaataacgccaccaacgtggtgatcaaggtgtgcgagtttcagttctgcaacgaccccttcctggacgtgtactaccacaagaacaacaagagctggatggagagcgagttcagagtgtacagcagcgctaacaactgcaccttcgagtacgtgagccaacccttcctgatggacctggagggcaagcaaggcaacttcaagaacctgagagagttcgtgttcaagaacatcgacggctacttcaagatctacagcaagcacacccccatcaacctgggcagagacctgccccaaggcttcagcgccctggagcccctggtggacctgcccatcggcatcaacatcacaagatttcagaccctgctggccctgcacagaagctacctcacccctggggacagcagcagcggctggaccgctggcgccgctgcctactacgtgggctacctgcagcctagaaccttcctgctgaagtacaacgagaacggcaccattacagacgccgtggactgcgccctggaccccctgagcgagaccaagtgcaccctgaagagcttcaccgtggagaagggcatctatcagacaagcaacttcagagtgcagcccaccgagagcatcgtgagattccccaacatcaccaacctgtgccccttcgacgaggtgttcaacgccaccaccttcgctagcgtgtacgcctggaatagaaagagaatcagcaactgcgtggccgactacagcgtgctgtacaacttcgcccccttcttcgccttcaaatgctatggcgtgagccccaccaagctgaacgacctgtgcttcaccaacgtgtacgccgacagcttcgtgatcagaggcaacgaggtgagccaaatcgcccctgggcagaccggcaacatcgccgattacaactacaaactgcccgacgacttcaccggctgcgtgatcgcctggaacagcaacaagctggacagcaccgtgggcggcaactacaactaccggtacagactgttcagaaagagcaagctgaagcccttcgagagagacatcagcaccgagatctaccaagccggcaacaagccctgcaacggcgtggccggcgtgaactgctacttccccctgcagagctacggcttcagacccacctacggcgtgggccatcagccctacagagtggtcgtgctgagcttcgagctgctgcacgcccccgccaccgtgtgcggccccaagaagagcaccaacctggtgaagaacaagtgcgtgaacttcaacttcaacggcctgaccggcaccggcgtgctgaccgagagcaacaagaagttcctgccctttcagcagttcggcagagacatcgccgacaccaccgacgccgtgcgggaccctcagaccctggagatcctggacatcaccccctgcagctttggcggcgtgagcgtgatcacccccggcaccaacacaagcaaccaagtggccgtgctgtaccaaggcgtcaattgcaccgaggtgcccgtggccatccacgccgatcagctgacccccacctggagagtctacagcaccggcagcaacgtgtttcagacaagagccggctgcctgatcggcgccgagtacgtgaacaacagctacgagtgcgacatccccatcggcgccggcatctgcgctagctatcagacacagaccaagagccacggcagcgctagcagcgtggctagccaaagcatcatcgcctacaccatgagcctgggcgccgagaacagcgtggcctacagcaacaacagcatcgccatccccaccaacttcaccatcagcgtgaccaccgagatcctgcccgtcagcatgaccaagacaagcgtggactgcaccatgtacatctgcggcgacagcaccgagtgcagcaacctgctcctgcagtacggcagcttctgcacacagctgaagagagccctgaccggcatcgccgtggagcaagacaagaacacccaagaggtgttcgcccaagtgaagcagatctacaagaccccccccatcaagtacttcggcggcttcaacttcagccaaatcctgcccgatcctagcaagcctagcaagagaagcttcatcgaggacctgctgttcaacaaggtgaccctggccgacgccggcttcatcaagcagtacggcgactgcctgggcgatatcgccgctagagacctgatctgcgctcagaagttcaatggcctgaccgtgctgccccccctgctgaccgacgagatgatcgctcagtacacaagcgccctgctggccggcaccatcacaagcggctggacattcggcgccggcgctgctctgcagatccccttcgccatgcagatggcctacagattcaacggcatcggcgtgacacagaacgtgctgtacgagaatcagaagctgatcgccaatcagttcaacagcgccatcggcaagatccaagacagcctgagcagcaccgctagcgccctgggcaagctgcaagacgtggtgaaccacaacgcccaagccctgaacaccctggtgaagcagctgagcagcaagttcggcgccatcagcagcgtgctgaacgatatcctgagcagactggacccccccgaggccgaggtgcagatcgacagactgattaccggcagactgcagagcctgcagacctacgtgacacagcagctgatcagagccgccgagatcagagctagcgccaacctggccgccaccaagatgagcgagtgcgtgctggggcagagcaagagagtggacttctgcggcaagggctaccacctgatgagcttccctcagagcgccccccacggcgtggtgttcctgcacgtgacctacgtgcccgcccaagagaagaacttcaccaccgctcccgctatctgccacgacggcaaggcccacttccctagagagggcgtgttcgtgagcaacggcacccactggttcgtgacacagagaaacttctacgagcctcagatcatcaccaccgacaacaccttcgtgagcggcaactgcgacgtggtgatcggcatcgtgaacaacaccgtgtacgaccccctgcaacccgagctggacagcttcaaggaggagctggacaagtactttaagaaccacacaagccccgacgtggacctgggcgacattagcggcatcaacgctagcgtggtgaacattcagaaggagattgacagactgaacgaggtggccaagaacctgaacgagagcctgatcgacctgcaagagctgggcaagtacgagcagtacatcaagtggccctggtacatctggctgggcttcatcgccggcctgatcgccatcgtgatggtgaccatcatgctgtgctgcatgacaagctgttgcagctgcctcaagggctgctgcagctgcggcagctgctgcaagttcgacgaggacgacagcgagcccgtgctgaagggcgtgaagctgcactacacctga

SEQ ID NO: 77 - protein, 1268 aa, synthetic construct
MFVFLVLLPLVSSQCVNLITRTQSYTNSFTRGVYYPDKVFRSSVLHSTQDLFLPFFSNVTWFHAISGTNGTKRFDNPVLPFNDGVYFASTEKSNIIRGWIFGTTLDSKTQSLLIVNNATNVVIKVCEFQFCNDPFLDVYYHKNNKSWMESEFRVYSSANNCTFEYVSQPFLMDLEGKQGNFKNLREFVFKNIDGYFKIYSKHTPINLGRDLPQGFSALEPLVDLPIGINITRFQTLLALHRSYLTPGDSSSGWTAGAAAYYVGYLQPRTFLLKYNENGTITDAVDCALDPLSETKCTLKSFTVEKGIYQTSNFRVQPTESIVRFPNITNLCPFDEVFNATTFASVYAWNRKRISNCVADYSVLYNFAPFFAFKCYGVSPTKLNDLCFTNVYADSFVIRGNEVSQIAPGQTGNIADYNYKLPDDFTGCVIAWNSNKLDSTVGGNYNYRYRLFRKSKLKPFERDISTEIYQAGNKPCNGVAGVNCYFPLQSYGFRPTYGVGHQPYRVVVLSFELLHAPATVCGPKKSTNLVKNKCVNFNFNGLTGTGVLTESNKKFLPFQQFGRDIADTTDAVRDPQTLEILDITPCSFGGVSVITPGTNTSNQVAVLYQGVNCTEVPVAIHADQLTPTWRVYSTGSNVFQTRAGCLIGAEYVNNSYECDIPIGAGICASYQTQTKSHGSASSVASQSIIAYTMSLGAENSVAYSNNSIAIPTNFTISVTTEILPVSMTKTSVDCTMYICGDSTECSNLLLQYGSFCTQLKRALTGIAVEQDKNTQEVFAQVKQIYKTPPIKYFGGFNFSQILPDPSKPSKRSFIEDLLFNKVTLADAGFIKQYGDCLGDIAARDLICAQKFNGLTVLPPLLTDEMIAQYTSALLAGTITSGWTFGAGAALQIPFAMQMAYRFNGIGVTQNVLYENQKLIANQFNSAIGKIQDSLSSTASALGKLQDVVNHNAQALNTLVKQLSSKFGAISSVLNDILSRLDPPEAEVQIDRLITGRLQSLQTYVTQQLIRAAEIRASANLAATKMSECVLGQSKRVDFCGKGYHLMSFPQSAPHGVVFLHVTYVPAQEKNFTTAPAICHDGKAHFPREGVFVSNGTHWFVTQRNFYEPQIITTDNTFVSGNCDVVIGIVNNTVYDPLQPELDSFKEELDKYFKNHTSPDVDLGDISGINASVVNIQKEIDRLNEVAKNLNESLIDLQELGKYEQYIKWPWYIWLGFIAGLIAIVMVTIMLCCMTSCCSCLKGCCSCGSCCKFDEDDSEPVLKGVKLHYT

SEQ ID NO: 78 - DNA, 21 bp, synthetic construct
  source 1..21: mol_type = other DNA
acacgtcaatgggaagtgaaa

SEQ ID NO: 79 - DNA, 21 bp, synthetic construct
  source 1..21: mol_type = other DNA
gctagacgatccagacatgat